European Patent Specification EP 3 705 490 B1, published March 6, 2024. Title: ENGINEERING AND OPTIMIZATION OF IMPROVED SYSTEMS, METHODS AND ENZYME COMPOSITIONS FOR SEQUENCE MANIPULATION. Applicant: THE BROAD INSTITUTE, INC. MASSACHUSETTS INSTITUTE OF TECHNOLOGY PRESIDENT AND FELLOWS OF HARVARD COLLEGE. Application EP DIVISIONAL DERIVED FROM EP APPLICATION NO. EP16151694.3. The sequence listing filed with the application follows.

SEQUENCE LISTING (228 sequences)

SEQ ID NO: 1 - DNA, 20 bp, Homo sapiens
gagtccgagcagaagaagaa

SEQ ID NO: 2 - DNA, 20 bp, Homo sapiens
gagtcctagcaggagaagaa

SEQ ID NO: 3 - DNA, 20 bp, Homo sapiens
gagtctaagcagaagaagaa

SEQ ID NO: 4 - RNA, 60 nt, Artificial Sequence
  source: /note="Description of Artificial Sequence: Synthetic oligonucleotide"
  modified_base (1)..(20): a, c, u, g, unknown or other
  modified_base (23)..(44): a, c, u, g, unknown or other
  modified_base (47)..(60): a, c, u, g, unknown or other
nnnnnnnnnnnnnnnnnnnnccnnnnnnnnnnnnnnnnnnnnnnggnnnnnnnnnnnnnn

SEQ ID NO: 5 - RNA, 60 nt, Artificial Sequence
  source: /note="Description of Artificial Sequence: Synthetic oligonucleotide"
  modified_base (1)..(14): a, c, u, g, unknown or other
  modified_base (17)..(38): a, c, u, g, unknown or other
  modified_base (41)..(60): a, c, u, g, unknown or other
nnnnnnnnnnnnnnccnnnnnnnnnnnnnnnnnnnnnnggnnnnnnnnnnnnnnnnnnnn

SEQ ID NO: 6 - RNA, 60 nt, Artificial Sequence
  source: /note="Description of Artificial Sequence: Synthetic oligonucleotide"
  modified_base (1)..(20): a, c, u, g, unknown or other
  modified_base (23)..(43): a, c, u, g, unknown or other
  modified_base (46)..(60): a, c, u, g, unknown or other
nnnnnnnnnnnnnnnnnnnnccnnnnnnnnnnnnnnnnnnnnnggnnnnnnnnnnnnnnn

SEQ ID NO: 7 - RNA, 60 nt, Artificial Sequence
  source: /note="Description of Artificial Sequence: Synthetic oligonucleotide"
  modified_base (1)..(15): a, c, u, g, unknown or other
  modified_base (18)..(38): a, c, u, g, unknown or other
  modified_base (41)..(60): a, c, u, g, unknown or other
nnnnnnnnnnnnnnnccnnnnnnnnnnnnnnnnnnnnnggnnnnnnnnnnnnnnnnnnnn

SEQ ID NO: 8 - RNA, 60 nt, Artificial Sequence
  source: /note="Description of Artificial Sequence: Synthetic oligonucleotide"
  modified_base (1)..(20): a, c, u, g, unknown or other
  modified_base (23)..(42): a, c, u, g, unknown or other
  modified_base (45)..(60): a, c, u, g, unknown or other
nnnnnnnnnnnnnnnnnnnnccnnnnnnnnnnnnnnnnnnnnggnnnnnnnnnnnnnnnn

SEQ ID NO: 9 - RNA, 60 nt, Artificial Sequence; identical to SEQ ID NO: 7
  source: /note="Description of Artificial Sequence: Synthetic oligonucleotide"
  modified_base (1)..(15): a, c, u, g, unknown or other
  modified_base (18)..(38): a, c, u, g, unknown or other
  modified_base (41)..(60): a, c, u, g, unknown or other

SEQ ID NO: 10 - RNA, 60 nt, Artificial Sequence
  source: /note="Description of Artificial Sequence: Synthetic oligonucleotide"
  modified_base (1)..(20): a, c, u, g, unknown or other
  modified_base (23)..(41): a, c, u, g, unknown or other
  modified_base (44)..(60): a, c, u, g, unknown or other
nnnnnnnnnnnnnnnnnnnnccnnnnnnnnnnnnnnnnnnnggnnnnnnnnnnnnnnnnn

SEQ ID NO: 11 - RNA, 60 nt, Artificial Sequence
  source: /note="Description of Artificial Sequence: Synthetic oligonucleotide"
  modified_base (1)..(17): a, c, u, g, unknown or other
  modified_base (20)..(38): a, c, u, g, unknown or other
  modified_base (41)..(60): a, c, u, g, unknown or other
nnnnnnnnnnnnnnnnnccnnnnnnnnnnnnnnnnnnnggnnnnnnnnnnnnnnnnnnnn

SEQ ID NO: 12 - RNA, 60 nt, Artificial Sequence
  source: /note="Description of Artificial Sequence: Synthetic oligonucleotide"
  modified_base (1)..(20): a, c, u, g, unknown or other
  modified_base (23)..(40): a, c, u, g, unknown or other
  modified_base (43)..(60): a, c, u, g, unknown or other
nnnnnnnnnnnnnnnnnnnnccnnnnnnnnnnnnnnnnnnggnnnnnnnnnnnnnnnnnn

SEQ ID NO: 13 - RNA, 60 nt, Artificial Sequence
  source: /note="Description of Artificial Sequence: Synthetic oligonucleotide"
  modified_base (1)..(18): a, c, u, g, unknown or other
  modified_base (21)..(38): a, c, u, g, unknown or other
  modified_base (41)..(60): a, c, u, g, unknown or other
nnnnnnnnnnnnnnnnnnccnnnnnnnnnnnnnnnnnnggnnnnnnnnnnnnnnnnnnnn

SEQ ID NO: 14 - RNA, 60 nt, Artificial Sequence
  source: /note="Description of Artificial Sequence: Synthetic oligonucleotide"
  modified_base (1)..(20): a, c, u, g, unknown or other
  modified_base (23)..(39): a, c, u, g, unknown or other
  modified_base (42)..(60): a, c, u, g, unknown or other
nnnnnnnnnnnnnnnnnnnnccnnnnnnnnnnnnnnnnnggnnnnnnnnnnnnnnnnnnn

SEQ ID NO: 15 - RNA, 60 nt, Artificial Sequence
  source: /note="Description of Artificial Sequence: Synthetic oligonucleotide"
  modified_base (1)..(19): a, c, u, g, unknown or other
  modified_base (22)..(38): a, c, u, g, unknown or other
  modified_base (41)..(60): a, c, u, g, unknown or other
nnnnnnnnnnnnnnnnnnnccnnnnnnnnnnnnnnnnnggnnnnnnnnnnnnnnnnnnnn

SEQ ID NO: 16 - RNA, 60 nt, Artificial Sequence
  source: /note="Description of Artificial Sequence: Synthetic oligonucleotide"
  modified_base (1)..(20): a, c, u, g, unknown or other
  modified_base (23)..(38): a, c, u, g, unknown or other
  modified_base (41)..(60): a, c, u, g, unknown or other
nnnnnnnnnnnnnnnnnnnnccnnnnnnnnnnnnnnnnggnnnnnnnnnnnnnnnnnnnn

SEQ ID NO: 17 - RNA, 60 nt, Artificial Sequence; identical to SEQ ID NO: 16
  source: /note="Description of Artificial Sequence: Synthetic oligonucleotide"
  modified_base (1)..(20): a, c, u, g, unknown or other
  modified_base (23)..(38): a, c, u, g, unknown or other
  modified_base (41)..(60): a, c, u, g, unknown or other

SEQ ID NO: 18 - RNA, 60 nt, Artificial Sequence
  source: /note="Description of Artificial Sequence: Synthetic oligonucleotide"
  modified_base (1)..(20): a, c, u, g, unknown or other
  modified_base (23)..(37): a, c, u, g, unknown or other
  modified_base (40)..(60): a, c, u, g, unknown or other
nnnnnnnnnnnnnnnnnnnnccnnnnnnnnnnnnnnnggnnnnnnnnnnnnnnnnnnnnn

SEQ ID NO: 19 - RNA, 60 nt, Artificial Sequence
  source: /note="Description of Artificial Sequence: Synthetic oligonucleotide"
  modified_base (1)..(21): a, c, u, g, unknown or other
  modified_base (24)..(38): a, c, u, g, unknown or other
  modified_base (41)..(60): a, c, u, g, unknown or other
nnnnnnnnnnnnnnnnnnnnnccnnnnnnnnnnnnnnnggnnnnnnnnnnnnnnnnnnnn

SEQ ID NO: 20 - RNA, 60 nt, Artificial Sequence
  source: /note="Description of Artificial Sequence: Synthetic oligonucleotide"
  modified_base (1)..(20): a, c, u, g, unknown or other
  modified_base (23)..(36): a, c, u, g, unknown or other
  modified_base (39)..(60): a, c, u, g, unknown or other
nnnnnnnnnnnnnnnnnnnnccnnnnnnnnnnnnnnggnnnnnnnnnnnnnnnnnnnnnn

SEQ ID NO: 21 - RNA, 60 nt, Artificial Sequence
  source: /note="Description of Artificial Sequence: Synthetic oligonucleotide"
  modified_base (1)..(22): a, c, u, g, unknown or other
  modified_base (25)..(38): a, c, u, g, unknown or other
  modified_base (41)..(60): a, c, u, g, unknown or other
nnnnnnnnnnnnnnnnnnnnnnccnnnnnnnnnnnnnnggnnnnnnnnnnnnnnnnnnnn

SEQ ID NO: 22 - RNA, 60 nt, Artificial Sequence
  source: /note="Description of Artificial Sequence: Synthetic oligonucleotide"
  modified_base (1)..(20): a, c, u, g, unknown or other
  modified_base (23)..(35): a, c, u, g, unknown or other
  modified_base (38)..(60): a, c, u, g, unknown or other
nnnnnnnnnnnnnnnnnnnnccnnnnnnnnnnnnnggnnnnnnnnnnnnnnnnnnnnnnn

SEQ ID NO: 23 - RNA, 60 nt, Artificial Sequence
  source: /note="Description of Artificial Sequence: Synthetic oligonucleotide"
  modified_base (1)..(23): a, c, u, g, unknown or other
  modified_base (26)..(38): a, c, u, g, unknown or other
  modified_base (41)..(60): a, c, u, g, unknown or other
nnnnnnnnnnnnnnnnnnnnnnnccnnnnnnnnnnnnnggnnnnnnnnnnnnnnnnnnnn

SEQ ID NO: 24 - RNA, 60 nt, Artificial Sequence
  source: /note="Description of Artificial Sequence: Synthetic oligonucleotide"
  modified_base (1)..(20): a, c, u, g, unknown or other
  modified_base (23)..(34): a, c, u, g, unknown or other
  modified_base (37)..(60): a, c, u, g, unknown or other
nnnnnnnnnnnnnnnnnnnnccnnnnnnnnnnnnggnnnnnnnnnnnnnnnnnnnnnnnn

SEQ ID NO: 25 - RNA, 60 nt, Artificial Sequence
  source: /note="Description of Artificial Sequence: Synthetic oligonucleotide"
  modified_base (1)..(24): a, c, u, g, unknown or other
  modified_base (27)..(38): a, c, u, g, unknown or other
  modified_base (41)..(60): a, c, u, g, unknown or other
nnnnnnnnnnnnnnnnnnnnnnnnccnnnnnnnnnnnnggnnnnnnnnnnnnnnnnnnnn

SEQ ID NO: 26 - RNA, 60 nt, Artificial Sequence
  source: /note="Description of Artificial Sequence: Synthetic oligonucleotide"
  modified_base (1)..(20): a, c, u, g, unknown or other
  modified_base (23)..(33): a, c, u, g, unknown or other
  modified_base (36)..(60): a, c, u, g, unknown or other
nnnnnnnnnnnnnnnnnnnnccnnnnnnnnnnnggnnnnnnnnnnnnnnnnnnnnnnnnn

SEQ ID NO: 27 - RNA, 60 nt, Artificial Sequence
  source: /note="Description of Artificial Sequence: Synthetic oligonucleotide"
  modified_base (1)..(25): a, c, u, g, unknown or other
  modified_base (28)..(38): a, c, u, g, unknown or other
  modified_base (41)..(60): a, c, u, g, unknown or other
nnnnnnnnnnnnnnnnnnnnnnnnnccnnnnnnnnnnnggnnnnnnnnnnnnnnnnnnnn

SEQ ID NO: 28 - RNA, 60 nt, Artificial Sequence
  source: /note="Description of Artificial Sequence: Synthetic oligonucleotide"
  modified_base (1)..(20): a, c, u, g, unknown or other
  modified_base (23)..(32): a, c, u, g, unknown or other
  modified_base (35)..(60): a, c, u, g, unknown or other
nnnnnnnnnnnnnnnnnnnnccnnnnnnnnnnggnnnnnnnnnnnnnnnnnnnnnnnnnn

SEQ ID NO: 29 - RNA, 60 nt, Artificial Sequence
  source: /note="Description of Artificial Sequence: Synthetic oligonucleotide"
  modified_base (1)..(26): a, c, u, g, unknown or other
  modified_base (29)..(38): a, c, u, g, unknown or other
  modified_base (41)..(60): a, c, u, g, unknown or other
nnnnnnnnnnnnnnnnnnnnnnnnnnccnnnnnnnnnnggnnnnnnnnnnnnnnnnnnnn

SEQ ID NO: 30 - RNA, 60 nt, Artificial Sequence
  source: /note="Description of Artificial Sequence: Synthetic oligonucleotide"
  modified_base (1)..(20): a, c, u, g, unknown or other
  modified_base (23)..(31): a, c, u, g, unknown or other
  modified_base (34)..(60): a, c, u, g, unknown or other
nnnnnnnnnnnnnnnnnnnnccnnnnnnnnnggnnnnnnnnnnnnnnnnnnnnnnnnnnn

SEQ ID NO: 31 - RNA, 60 nt, Artificial Sequence
  source: /note="Description of Artificial Sequence: Synthetic oligonucleotide"
  modified_base (1)..(27): a, c, u, g, unknown or other
  modified_base (30)..(38): a, c, u, g, unknown or other
  modified_base (41)..(60): a, c, u, g, unknown or other
nnnnnnnnnnnnnnnnnnnnnnnnnnnccnnnnnnnnnggnnnnnnnnnnnnnnnnnnnn

SEQ ID NO: 32 - RNA, 60 nt, Artificial Sequence
  source: /note="Description of Artificial Sequence: Synthetic oligonucleotide"
  modified_base (1)..(20): a, c, u, g, unknown or other
  modified_base (23)..(30): a, c, u, g, unknown or other
  modified_base (33)..(60): a, c, u, g, unknown or other
nnnnnnnnnnnnnnnnnnnnccnnnnnnnnggnnnnnnnnnnnnnnnnnnnnnnnnnnnn

SEQ ID NO: 33 - RNA, 60 nt, Artificial Sequence
  source: /note="Description of Artificial Sequence: Synthetic oligonucleotide"
  modified_base (1)..(28): a, c, u, g, unknown or other
  modified_base (31)..(38): a, c, u, g, unknown or other
  modified_base (41)..(60): a, c, u, g, unknown or other
nnnnnnnnnnnnnnnnnnnnnnnnnnnnccnnnnnnnnggnnnnnnnnnnnnnnnnnnnn

SEQ ID NO: 34 - RNA, 60 nt, Artificial Sequence
  source: /note="Description of Artificial Sequence: Synthetic oligonucleotide"
  modified_base (1)..(20): a, c, u, g, unknown or other
  modified_base (23)..(29): a, c, u, g, unknown or other
  modified_base (32)..(60): a, c, u, g, unknown or other
nnnnnnnnnnnnnnnnnnnnccnnnnnnnggnnnnnnnnnnnnnnnnnnnnnnnnnnnnn

SEQ ID NO: 35 - RNA, 60 nt, Artificial Sequence
  source: /note="Description of Artificial Sequence: Synthetic oligonucleotide"
  modified_base (1)..(29): a, c, u, g, unknown or other
  modified_base (32)..(38): a, c, u, g, unknown or other
  modified_base (41)..(60): a, c, u, g, unknown or other
nnnnnnnnnnnnnnnnnnnnnnnnnnnnnccnnnnnnnggnnnnnnnnnnnnnnnnnnnn

SEQ ID NO: 36 - RNA, 60 nt, Artificial Sequence
  source: /note="Description of Artificial Sequence: Synthetic oligonucleotide"
  modified_base (1)..(20): a, c, u, g, unknown or other
  modified_base (23)..(28): a, c, u, g, unknown or other
  modified_base (31)..(60): a, c, u, g, unknown or other
nnnnnnnnnnnnnnnnnnnnccnnnnnnggnnnnnnnnnnnnnnnnnnnnnnnnnnnnnn

SEQ ID NO: 37 - RNA, 60 nt, Artificial Sequence
  source: /note="Description of Artificial Sequence: Synthetic oligonucleotide"
  modified_base (1)..(30): a, c, u, g, unknown or other
  modified_base (33)..(38): a, c, u, g, unknown or other
  modified_base (41)..(60): a, c, u, g, unknown or other
nnnnnnnnnnnnnnnnnnnnnnnnnnnnnnccnnnnnnggnnnnnnnnnnnnnnnnnnnn

SEQ ID NO: 38 - RNA, 60 nt, Artificial Sequence
  source: /note="Description of Artificial Sequence: Synthetic oligonucleotide"
  modified_base (1)..(20): a, c, u, g, unknown or other
  modified_base (23)..(27): a, c, u, g, unknown or other
  modified_base (30)..(60): a, c, u, g, unknown or other
nnnnnnnnnnnnnnnnnnnnccnnnnnggnnnnnnnnnnnnnnnnnnnnnnnnnnnnnnn

SEQ ID NO: 39 - RNA, 60 nt, Artificial Sequence
  source: /note="Description of Artificial Sequence: Synthetic oligonucleotide"
  modified_base (1)..(31): a, c, u, g, unknown or other
  modified_base (34)..(38): a, c, u, g, unknown or other
  modified_base (41)..(60): a, c, u, g, unknown or other
nnnnnnnnnnnnnnnnnnnnnnnnnnnnnnnccnnnnnggnnnnnnnnnnnnnnnnnnnn

SEQ ID NO: 40 - RNA, 60 nt, Artificial Sequence
  source: /note="Description of Artificial Sequence: Synthetic oligonucleotide"
  modified_base (1)..(20): a, c, u, g, unknown or other
  modified_base (23)..(26): a, c, u, g, unknown or other
  modified_base (29)..(60): a, c, u, g, unknown or other
nnnnnnnnnnnnnnnnnnnnccnnnnggnnnnnnnnnnnnnnnnnnnnnnnnnnnnnnnn

SEQ ID NO: 41 - RNA, 60 nt, Artificial Sequence
  source: /note="Description of Artificial Sequence: Synthetic oligonucleotide"
  modified_base (1)..(32): a, c, u, g, unknown or other
  modified_base (35)..(38): a, c, u, g, unknown or other
  modified_base (41)..(60): a, c, u, g, unknown or other
nnnnnnnnnnnnnnnnnnnnnnnnnnnnnnnnccnnnnggnnnnnnnnnnnnnnnnnnnn

SEQ ID NO: 42 - RNA, 60 nt, Artificial Sequence
  source: /note="Description of Artificial Sequence: Synthetic oligonucleotide"
  modified_base (1)..(20): a, c, u, g, unknown or other
  modified_base (23)..(25): a, c, u, g, unknown or other
  modified_base (28)..(60): a, c, u, g, unknown or other
nnnnnnnnnnnnnnnnnnnnccnnnggnnnnnnnnnnnnnnnnnnnnnnnnnnnnnnnnn

SEQ ID NO: 43 - RNA, 60 nt, Artificial Sequence
  source: /note="Description of Artificial Sequence: Synthetic oligonucleotide"
  modified_base (1)..(33): a, c, u, g, unknown or other
  modified_base (36)..(38): a, c, u, g, unknown or other
  modified_base (41)..(60): a, c, u, g, unknown or other
nnnnnnnnnnnnnnnnnnnnnnnnnnnnnnnnnccnnnggnnnnnnnnnnnnnnnnnnnn

SEQ ID NO: 44 - RNA, 60 nt, Artificial Sequence
  source: /note="Description of Artificial Sequence: Synthetic oligonucleotide"
  modified_base (1)..(20): a, c, u, g, unknown or other
  modified_base (23)..(24): a, c, u, g, unknown or other
  modified_base (27)..(60): a, c, u, g, unknown or other
nnnnnnnnnnnnnnnnnnnnccnnggnnnnnnnnnnnnnnnnnnnnnnnnnnnnnnnnnn

SEQ ID NO: 45 - RNA, 60 nt, Artificial Sequence
  source: /note="Description of Artificial Sequence: Synthetic oligonucleotide"
  modified_base (1)..(34): a, c, u, g, unknown or other
  modified_base (37)..(38): a, c, u, g, unknown or other
  modified_base (41)..(60): a, c, u, g, unknown or other
nnnnnnnnnnnnnnnnnnnnnnnnnnnnnnnnnnccnnggnnnnnnnnnnnnnnnnnnnn

SEQ ID NO: 46 - RNA, 60 nt, Artificial Sequence
  source: /note="Description of Artificial Sequence: Synthetic oligonucleotide"
  modified_base (1)..(20): a, c, u, g, unknown or other
  modified_base (23)..(23): a, c, u, g, unknown or other
  modified_base (26)..(60): a, c, u, g, unknown or other
nnnnnnnnnnnnnnnnnnnnccnggnnnnnnnnnnnnnnnnnnnnnnnnnnnnnnnnnnn

SEQ ID NO: 47 - RNA, 60 nt, Artificial Sequence
  source: /note="Description of Artificial Sequence: Synthetic oligonucleotide"
  modified_base (1)..(35): a, c, u, g, unknown or other
  modified_base (38)..(38): a, c, u, g, unknown or other
  modified_base (41)..(60): a, c, u, g, unknown or other
nnnnnnnnnnnnnnnnnnnnnnnnnnnnnnnnnnnccnggnnnnnnnnnnnnnnnnnnnn

SEQ ID NO: 48 - RNA, 60 nt, Artificial Sequence
  source: /note="Description of Artificial Sequence: Synthetic oligonucleotide"
  modified_base (1)..(21): a, c, u, g, unknown or other
  modified_base (26)..(60): a, c, u, g, unknown or other
nnnnnnnnnnnnnnnnnnnnnccggnnnnnnnnnnnnnnnnnnnnnnnnnnnnnnnnnnn

SEQ ID NO: 49 - RNA, 60 nt, Artificial Sequence
  source: /note="Description of Artificial Sequence: Synthetic oligonucleotide"
  modified_base (1)..(35): a, c, u, g, unknown or other
  modified_base (40)..(60): a, c, u, g, unknown or other
nnnnnnnnnnnnnnnnnnnnnnnnnnnnnnnnnnnccggnnnnnnnnnnnnnnnnnnnnn

SEQ ID NO: 50 - RNA, 60 nt, Artificial Sequence
  source: /note="Description of Artificial Sequence: Synthetic oligonucleotide"
  modified_base (1)..(23): a, c, u, g, unknown or other
  modified_base (26)..(60): a, c, u, g, unknown or other
nnnnnnnnnnnnnnnnnnnnnnnggnnnnnnnnnnnnnnnnnnnnnnnnnnnnnnnnnnn

SEQ ID NO: 51 - RNA, 60 nt, Artificial Sequence
  source: /note="Description of Artificial Sequence: Synthetic oligonucleotide"
  modified_base (1)..(33): a, c, u, g, unknown or other
  modified_base (38)..(60): a, c, u, g, unknown or other
nnnnnnnnnnnnnnnnnnnnnnnnnnnnnnnnnggccnnnnnnnnnnnnnnnnnnnnnnn

SEQ ID NO: 52 - RNA, 60 nt, Artificial Sequence
  source: /note="Description of Artificial Sequence: Synthetic oligonucleotide"
  modified_base (1)..(22): a, c, u, g, unknown or other
  modified_base (26)..(60): a, c, u, g, unknown or other
nnnnnnnnnnnnnnnnnnnnnncggnnnnnnnnnnnnnnnnnnnnnnnnnnnnnnnnnnn

SEQ ID NO: 53 - RNA, 60 nt, Artificial Sequence
  source: /note="Description of Artificial Sequence: Synthetic oligonucleotide"
  modified_base (1)..(32): a, c, u, g, unknown or other
  modified_base (35)..(35): a, c, u, g, unknown or other
  modified_base (38)..(60): a, c, u, g, unknown or other
nnnnnnnnnnnnnnnnnnnnnnnnnnnnnnnnggnccnnnnnnnnnnnnnnnnnnnnnnn

SEQ ID NO: 54 - RNA, 60 nt, Artificial Sequence
  source: /note="Description of Artificial Sequence: Synthetic oligonucleotide"
  modified_base (1)..(31): a, c, u, g, unknown or other
  modified_base (34)..(35): a, c, u, g, unknown or other
  modified_base (38)..(60): a, c, u, g, unknown or other
nnnnnnnnnnnnnnnnnnnnnnnnnnnnnnnggnnccnnnnnnnnnnnnnnnnnnnnnnn

SEQ ID NO: 55 - RNA, 60 nt, Artificial Sequence
  source: /note="Description of Artificial Sequence: Synthetic oligonucleotide"
  modified_base (1)..(30): a, c, u, g, unknown or other
  modified_base (33)..(35): a, c, u, g, unknown or other
  modified_base (38)..(60): a, c, u, g, unknown or other
nnnnnnnnnnnnnnnnnnnnnnnnnnnnnnggnnnccnnnnnnnnnnnnnnnnnnnnnnn

SEQ ID NO: 56 - RNA, 60 nt, Artificial Sequence
  source: /note="Description of Artificial Sequence: Synthetic oligonucleotide"
  modified_base (1)..(29): a, c, u, g, unknown or other
  modified_base (32)..(35): a, c, u, g, unknown or other
  modified_base (38)..(60): a, c, u, g, unknown or other
nnnnnnnnnnnnnnnnnnnnnnnnnnnnnggnnnnccnnnnnnnnnnnnnnnnnnnnnnn

SEQ ID NO: 57 - RNA, 60 nt, Artificial Sequence
  source: /note="Description of Artificial Sequence: Synthetic oligonucleotide"
  modified_base (1)..(28): a, c, u, g, unknown or other
  modified_base (31)..(35): a, c, u, g, unknown or other
  modified_base (38)..(60): a, c, u, g, unknown or other
nnnnnnnnnnnnnnnnnnnnnnnnnnnnggnnnnnccnnnnnnnnnnnnnnnnnnnnnnn

SEQ ID NO: 58 - RNA, 12 nt, Artificial Sequence
  source: /note="Description of Artificial Sequence: Synthetic oligonucleotide"
guuuuagagcua

SEQ ID NO: 59 - protein, 7 aa, Simian virus 40
PKKKRKV

SEQ ID NO: 60 - protein, 16 aa, Unknown
  source: /note="Description of Unknown: Nucleoplasmin bipartite NLS sequence"
KRPAATKKAGQAKKKK

SEQ ID NO: 61 - protein, 9 aa, Unknown
  source: /note="Description of Unknown: C-myc NLS sequence"
PAAKRVKLD

SEQ ID NO: 62 - protein, 11 aa, Unknown
  source: /note="Description of Unknown: C-myc NLS sequence"
RQRRNELKRSP

SEQ ID NO: 63 - protein, 38 aa, Homo sapiens
NQSSNFGPMKGGNFGGRSSGPYGGGGQYFAKPRNQGGY

SEQ ID NO: 64 - protein, 42 aa, Unknown
  source: /note="Description of Unknown: IBB domain from importin-alpha sequence"
RMRIZFKNKGKDTAELRRRRVEVSVELRKAKKDEQILKRRNV

SEQ ID NO: 65 - protein, 8 aa, Unknown
  source: /note="Description of Unknown: Myoma T protein sequence"
VSRKRPRP

SEQ ID NO: 66 - protein, 8 aa, Unknown
  source: /note="Description of Unknown: Myoma T protein sequence"
PPKKARED

SEQ ID NO: 67 - protein, 8 aa, Homo sapiens
PQPKKKPL

SEQ ID NO: 68 - protein, 12 aa, Mus musculus
SALIKKKKKMAP

SEQ ID NO: 69 - protein, 5 aa, Influenza virus
DRLRR

SEQ ID NO: 70 - protein, 7 aa, Influenza virus
PKQKKRK

SEQ ID NO: 71 - protein, 10 aa, Hepatitus delta virus
RKLKKKIKKL

SEQ ID NO: 72 - protein, 10 aa, Mus musculus
REKKKFLKRR

SEQ ID NO: 73 - protein, 20 aa, Homo sapiens
KRKGDEVDGVDEVAKKKSKK

SEQ ID NO: 74 - protein, 17 aa, Homo sapiens
RKCLQAGMNLEARKTKK

SEQ ID NO: 75 - DNA, 137 bp, Artificial Sequence
  source: /note="Description of Artificial Sequence: Synthetic polynucleotide"
  modified_base (1)..(20): a, c, t, g, unknown or other
nnnnnnnnnnnnnnnnnnnngtttttgtactctcaagatttagaaataaatcttgcagaagctacaaagataaggcttcatgccgaaatcaacaccctgtcattttatggcagggtgttttcgttatttaatttttt

SEQ ID NO: 76 - DNA, 123 bp, Artificial Sequence
  source: /note="Description of Artificial Sequence: Synthetic polynucleotide"
  modified_base (1)..(20): a, c, t, g, unknown or other
nnnnnnnnnnnnnnnnnnnngtttttgtactctcagaaatgcagaagctacaaagataaggcttcatgccgaaatcaacaccctgtcattttatggcagggtgttttcgttatttaatttttt

SEQ ID NO: 77 - DNA, 110 bp, Artificial Sequence
  source: /note="Description of Artificial Sequence: Synthetic polynucleotide"
  modified_base (1)..(20): a, c, t, g, unknown or other
nnnnnnnnnnnnnnnnnnnngtttttgtactctcagaaatgcagaagctacaaagataaggcttcatgccgaaatcaacaccctgtcattttatggcagggtgttttttt

SEQ ID NO: 78 - DNA, 102 bp, Artificial Sequence
  source: /note="Description of Artificial Sequence: Synthetic polynucleotide"
  modified_base (1)..(20): a, c, t, g, unknown or other
nnnnnnnnnnnnnnnnnnnngttttagagctagaaatagcaagttaaaataaggctagtccgttatcaacttgaaaaagtggcaccgagtcggtgctttttt

SEQ ID NO: 79 - DNA, 88 bp, Artificial Sequence
  source: /note="Description of Artificial Sequence: Synthetic oligonucleotide"
  modified_base (1)..(20): a, c, t, g, unknown or other
nnnnnnnnnnnnnnnnnnnngttttagagctagaaatagcaagttaaaataaggctagtccgttatcaacttgaaaaagtgttttttt

SEQ ID NO: 80 - DNA, 76 bp, Artificial Sequence
  source: /note="Description of Artificial Sequence: Synthetic oligonucleotide"
  modified_base (1)..(20): a, c, t, g, unknown or other
nnnnnnnnnnnnnnnnnnnngttttagagctagaaatagcaagttaaaataaggctagtccgttatcatttttttt

SEQ ID NO: 81 - protein, 984 aa, Campylobacter jejuni
MARILAFDIGISSIGWAFSENDELKDCGVRIFTKVENPKTGESLALPRRLARSARKRLARRKARLNHLKHLIANEFKLNYEDYQSFDESLAKAYKGSLISPYELRFRALNELLSKQDFARVILHIAKRRGYDDIKNSDDKEKGAILKAIKQNEEKLANYQSVGEYLYKEYFQKFKENSKEFTNVRNKKESYERCIAQSFLKDELKLIFKKQREFGFSFSKKFEEEVLSVAFYKRALKDFSHLVGNCSFFTDEKRAPKNSPLAFMFVALTRIINLLNNLKNTEGILYTKDDLNALLNEVLKNGTLTYKQTKKLLGLSDDYEFKGEKGTYFIEFKKYKEFIKALGEHNLSQDDLNEIAKDITLIKDEIKLKKALAKYDLNQNQIDSLSKLEFKDHLNISFKALKLVTPLMLEGKKYDEACNELNLKVAINEDKKDFLPAFNETYYKDEVTNPVVLRAIKEYRKVLNALLKKYGKVHKINIELAREVGKNHSQRAKIEKEQNENYKAKKDAELECEKLGLKINSKNILKLRLFKEQKEFCAYSGEKIKISDLQDEKMLEIDHIYPYSRSFDDSYMNKVLVFTKQNQEKLNQTPFEAFGNDSAKWQKIEVLAKNLPTKKQKRILDKNYKDKEQKNFKDRNLNDTRYIARLVLNYTKDYLDFLPLSDDENTKLNDTQKGSKVHVEAKSGMLTSALRHTWGFSAKDRNNHLHHAIDAVIIAYANNSIVKAFSDFKKEQESNSAELYAKKISELDYKNKRKFFEPFSGFRQKVLDKIDEIFVSKPERKKPSGALHEETFRKEEEFYQSYGGKEGVLKALELGKIRKVNGKIVKNGDMFRVDIFKHKKTNKFYAVPIYTMDFALKVLPNKAVARSKKGEIKDWILMDENYEFCFSLYKDSLILIQTKDMQEPEFVYYNAFTSSTVSLIVSKHDNKFETLSKNQKILFKNANEKEVIAKSIGIQNLKVFEKYIVSALGEVTKAEFRQREDFKK

SEQ ID NO: 82 - DNA, 91 bp, Artificial Sequence
  source: /note="Description of Artificial Sequence: Synthetic oligonucleotide"
tataatctcataagaaatttaaaaagggactaaaataaagagtttgcgggactctgcggggttacaatcccctaaaaccgcttttaaaatt

SEQ ID NO: 83 - DNA, 36 bp, Artificial Sequence
  source: /note="Description of Artificial Sequence: Synthetic oligonucleotide"
gttttagtccctttttaaatttctttatggtaaaat

SEQ ID NO: 84 - RNA, 95 nt, Artificial Sequence
  source: /note="Description of Artificial Sequence: Synthetic oligonucleotide"
  modified_base (1)..(20): a, c, u, g, unknown or other
nnnnnnnnnnnnnnnnnnnnguuuuagucccgaaagggacuaaaauaaagaguuugcgggacucugcgggguuacaauccccuaaaaccgcuuuu

SEQ ID NO: 85 - DNA, 3243 bp, Artificial Sequence
  source: /note="Description of Artificial Sequence: Synthetic polynucleotide"
accggtgccaccatgtacccatacgatgttccagattacgcttcgccgaagaaaaagcgcaaggtcgaagcgtccatgaaaaggaactacattctggggctggacatcgggattacaagcgtggggtatgggattattgactatgaaacaagggacgtgatcgacgcaggcgtcagactgttcaaggaggccaacgtggaaaacaatgagggacggagaagcaagaggggagccaggcgcctgaaacgacggagaaggcacagaatccagagggtgaagaaactgctgttcgattacaacctgctgaccgaccattctgagctgagtggaattaatccttatgaagccagggtgaaaggcctgagtcagaagctgtcagaggaagagttttccgcagctctgctgcacctggctaagcgccgaggagtgcataacgtcaatgaggtggaagaggacaccggcaacgagctgtctacaaaggaacagatctcacgcaatagcaaagctctggaagagaagtatgtcgcagagctgcagctggaacggctgaagaaagatggcgaggtgagagggtcaattaataggttcaagacaagcgactacgtcaaagaagccaagcagctgctgaaagtgcagaaggcttaccaccagctggatcagagcttcatcgatacttatatcgacctgctggagactcggagaacctactatgagggaccaggagaagggagccccttcggatggaaagacatcaaggaatggtacgagatgctgatgggacattgcacctattttccagaagagctgagaagcgtcaagtacgcttataacgcagatctgtacaacgccctgaatgacctgaacaacctggtcatcaccagggatgaaaacgagaaactggaatactatgagaagttccagatcatcgaaaacgtgtttaagcagaagaaaaagcctacactgaaacagattgctaaggagatcctggtcaacgaagaggacatcaagggctaccgggtgacaagcactggaaaaccagagttcaccaatctgaaagtgtatcacgatattaaggacatcacagcacggaaagaaatcattgagaacgccgaactgctggatcagattgctaagatcctgactatctaccagagctccgaggacatccaggaagagctgactaacctgaacagcgagctgacccaggaagagatcgaacagattagtaatctgaaggggtacaccggaacacacaacctgtccctgaaagctatcaatctgattctggatgagctgtggcatacaaacgacaatcagattgcaatctttaaccggctgaagctggtcccaaaaaaggtggacctgagtcagcagaaagagatcccaaccacactggtggacgatttcattctgtcacccgtggtcaagcggagcttcatccagagcatcaaagtgatcaacgccatcatcaagaagtacggcctgcccaatgatatcattatcgagctggctagggagaagaacagcaaggacgcacagaagatgatcaatgagatgcagaaacgaaaccggcagaccaatgaacgcattgaagagattatccgaactaccgggaaagagaacgcaaagtacctgattgaaaaaatcaagctgcacgatatgcaggagggaaagtgtctgtattctctggaggccatccccctggaggacctgctgaacaatccattcaactacgaggtcgatcatattatccccagaagcgtgtccttcgacaattcctttaacaacaaggtgctggtcaagcaggaagagaactctaaaaagggcaataggactcctttccagtacctgtctagttcagattccaagatctcttacgaaacctttaaaaagcacattctgaatctggccaaaggaaagggccgcatcagcaagaccaaaaaggagtacctgctggaagagcgggacatcaacagattctccgtccagaaggattttattaaccggaatctggtggacacaagatacgctactcgcggcctgatgaatctgctgcgatcctatttccgggtgaacaatctggatgtgaaagtcaagtccatcaacggcgggttcacatcttttctgaggcgcaaatggaagtttaaaaaggagcgcaacaaagggtacaagcaccatgccgaagatgctctgattatcgcaaatgccgacttcatctttaaggagtggaaaaagctggacaaagccaagaaagtgatggagaaccagatgttcgaagagaagcaggccgaatctatgcccgaaatcgagacagaacaggagtacaaggagattttcatcactcctcaccagatcaagcatatcaaggatttcaaggactacaagtactctcaccgggtggataaaaagcccaacagagagctgatcaatgacaccctgtatagtacaagaaaagacgataaggggaataccctgattgtgaacaatctgaacggactgtacgacaaagataatgacaagctgaaaaagctgatcaacaaaagtcccgagaagctgctgatgtaccaccatgatcctcagacatatcagaaactgaagctgattatggagcagtacggcgacgagaagaacccactgtataagtactatgaagagactgggaactacctgaccaagtatagcaaaaaggataatggccccgtgatcaagaagatcaagtactatgggaacaagctgaatgcccatctggacatcacagacgattaccctaacagtcgcaacaaggtggtcaagctgtcactgaagccatacagattcgatgtctatctggacaacggcgtgtataaatttgtgactgtcaagaatctggatgtcatcaaaaaggagaactactatgaagtgaatagcaagtgctacgaagaggctaaaaagctgaaaaagattagcaaccaggcagagttcatcgcctccttttacaacaacgacctgattaagatcaatggcgaactgtatagggtcatcggggtgaacaatgatctgctgaaccgcattgaagtgaatatgattgacatcacttaccgagagtatctggaaaacatgaatgataagcgcccccctcgaattatcaaaacaattgcctctaagactcagagtatcaaaaagtactcaaccgacattctgggaaacctgtatgaggtgaagagcaaaaagcaccctcagattatcaaaaagggctaagaattc

SEQ ID NO: 86 - protein, 1115 aa, Artificial Sequence
  source: /note="Description of Artificial Sequence: Synthetic polypeptide"
MSDLVLGLDIGIGSVGVGILNKVTGEIIHKNSRIFPAAQAENNLVRRTNRQGRRLARRKKHRRVRLNRLFEESGLITDFTKISINLNPYQLRVKGLTDELSNEELFIALKNMVKHRGISYLDDASDDGNSSVGDYAQIVKENSKQLETKTPGQIQLERYQTYGQLRGDFTVEKDGKKHRLINVFPTSAYRSEALRILQTQQEFNPQITDEFINRYLEILTGKRKYYHGPGNEKSRTDYGRYRTSGETLDNIFGILIGKCTFYPDEFRAAKASYTAQEFNLLNDLNNLTVPTETKKLSKEQKNQIINYVKNEKAMGPAKLFKYIAKLLSCDVADIKGYRIDKSGKAEIHTFEAYRKMKTLETLDIEQMDRETLDKLAYVLTLNTEREGIQEALEHEFADGSFSQKQVDELVQFRKANSSIFGKGWHNFSVKLMMELIPELYETSEEQMTILTRLGKQKTTSSSNKTKYIDEKLLTEEIYNPVVAKSVRQAIKIVNAAIKEYGDFDNIVIEMARENQTTQKGQKNSRERMKRIEEGIKELGSQILKEHPVENTQLQNEKLYLYYLQNGRDMYVDQELDINRLSDYDVDHIVPQSFLKDDSIDNKVLTRSDKNRGKSDNVPSEEVVKKMKNYWRQLLNAKLITQRKFDNLTKAERGGLSELDKAGFIKRQLVETRQITKHVAQILDSRMNTKYDENDKLIREVKVITLKSKLVSDFRKDFQFYKVREINNYHHAHDAYLNAVVGTALIKKYPKLESEFVYGDYKVYDVRKMIAKSEQEIGKATAKYFFYSNIMNFFKTEITLANGEIRKRPLIETNGETGEIVWDKGRDFATVRKVLSMPQVNIVKKTEVQTGGFSKESILPKRNSDKLIARKKDWDPKKYGGFDSPTVAYSVLVVAKVEKGKSKKLKSVKELLGITIMERSSFEKNPIDFLEAKGYKEVKKDLIIKLPKYSLFELENGRKRMLASAGELQKGNELALPSKYVNFLYLASHYEKLKGSPEDNEQKQLFVEQHKHYLDEIIEQISEFSKRVILADANLDKVLSAYNKHRDKPIREQAENIIHLFTLTNLGAPAAFKYFDTTIDRKRYTSTKEVLDATLIHQSITGLYETRIDLSQLGGD

SEQ ID NO: 87 - protein, 1374 aa, Artificial Sequence
  source: /note="Description of Artificial Sequence: Synthetic polypeptide"
MDKKYSIGLDIGTNSVGWAVITDEYKVPSKKFKVLGNTDRHSIKKNLIGALLFDSGETAEATRLKRTARRRYTRRKNRICYLQEIFSNEMAKVDDSFFHRLEESFLVEEDKKHERHPIFGNIVDEVAYHEKYPTIYHLRKKLVDSTDKADLRLIYLALAHMIKFRGHFLIEGDLNPDNSDVDKLFIQLVQTYNQLFEENPINASGVDAKAILSARLSKSRRLENLIAQLPGEKKNGLFGNLIALSLGLTPNFKSNFDLAEDAKLQLSKDTYDDDLDNLLAQIGDQYADLFLAAKNLSDAILLSDILRVNTEITKAPLSASMIKRYDEHHQDLTLLKALVRQQLPEKYKEIFFDQSKNGYAGYIDGGASQEEFYKFIKPILEKMDGTEELLVKLNREDLLRKQRTFDNGSIPHQIHLGELHAILRRQEDFYPFLKDNREKIEKILTFRIPYYVGPLARGNSRFAWMTRKSEETITPWNFEEVVDKGASAQSFIERMTNFDKNLPNEKVLPKHSLLYEYFTVYNELTKVKYVTEGMRKPAFLSGEQKKAIVDLLFKTNRKVTVKQLKEDYFKKIECFDSVEISGVEDRFNASLGTYHDLLKIIKDKDFLDNEENEDILEDIVLTLTLFEDREMIEERLKTYAHLFDDKVMKQLKRRRYTGWGRLSRKLINGIRDKQSGKTILDFLKSDGFANRNFMQLIHDDSLTFKEDIQKAQVSGQGDSLHEHIANLAGSPAIKKGILQTVKVVDELVKVMGRHKPENIVIEMARETNEDDEKKAIQKIQKANKDEKDAAMLKAANQYNGKAELPHSVFHGHKQLATKIRLWHQQGERCLYTGKTISIHDLINNSNQFEVDHILPLSITFDDSLANKVLVYATANQEKGQRTPYQALDSMDDAWSFRELKAFVRESKTLSNKKKEYLLTEEDISKFDVRKKFIERNLVDTRYASRVVLNALQEHFRAHKIDTKVSVVRGQFTSQLRRHWGIEKTRDTYHHHAVDALIIAASSQLNLWKKQKNTLVSYSEDQLLDIETGELISDDEYKESVFKAPYQHFVDTLKSKEFEDSILFSYQVDSKFNRKISDATIYATRQAKVGKDKADETYVLGKIKDIYTQDGYDAFMKIYKKDKSKFLMYRHDPQTFEKVIEPILENYPNKQINEKGKEVPCNPFLKYKEEHGYIRKYSKKGNGPEIKSLKYYDSKLGNHIDITPKDSNNKVVLQSVSPWRADVYFNKTTGKYEILGLKYADLQFEKGTGTYKISQEKYNDIKKKEGVDSDSEFKFTLYKNDLLLVKDTETKEQQLFRFLSRTMPKQKHYVELKPYDKQKFEGGEALIKVLGNVANSGQCKKGLGKSNISIYKVRTDVLGNQHIIKNEGDKPKLDF

SEQ ID NO: 88 - DNA, 4677 bp, Artificial Sequence
  source: /note="Description of Artificial Sequence: Synthetic polynucleotide"
tctttcttgcgctatgacacttccagcaaaaggtagggcgggctgcgagacggcttcccggcgctgcatgcaacaccgatgatgcttcgaccccccgaagctccttcggggctgcatgggcgctccgatgccgctccagggcgagcgctgtttaaatagccaggcccccgattgcaaagacattatagcgagctaccaaagccatattcaaacacctagatcactaccacttctacacaggccactcgagcttgtgatcgcactccgctaagggggcgcctcttcctcttcgtttcagtcacaacccgcaaacatgtacccatacgatgttccagattacgcttcgccgaagaaaaagcgcaaggtcgaagcgtccgacaagaagtacagcatcggcctggacatcggcaccaactctgtgggctgggccgtgatcaccgacgagtacaaggtgcccagcaagaaattcaaggtgctgggcaacaccgaccggcacagcatcaagaagaacctgatcggagccctgctgttcgacagcggcgaaacagccgaggccacccggctgaagagaaccgccagaagaagatacaccagacggaagaaccggatctgctatctgcaagagatcttcagcaacgagatggccaaggtggacgacagcttcttccacagactggaagagtccttcctggtggaagaggataagaagcacgagcggcaccccatcttcggcaacatcgtggacgaggtggcctaccacgagaagtaccccaccatctaccacctgagaaagaaactggtggacagcaccgacaaggccgacctgcggctgatctatctggccctggcccacatgatcaagttccggggccacttcctgatcgagggcgacctgaaccccgacaacagcgacgtggacaagctgttcatccagctggtgcagacctacaaccagctgttcgaggaaaaccccatcaacgccagcggcgtggacgccaaggccatcctgtctgccagactgagcaagagcagacggctggaaaatctgatcgcccagctgcccggcgagaagaagaatggcctgttcggcaacctgattgccctgagcctgggcctgacccccaacttcaagagcaacttcgacctggccgaggatgccaaactgcagctgagcaaggacacctacgacgacgacctggacaacctgctggcccagatcggcgaccagtacgccgacctgtttctggccgccaagaacctgtccgacgccatcctgctgagcgacatcctgagagtgaacaccgagatcaccaaggcccccctgagcgcctctatgatcaagagatacgacgagcaccaccaggacctgaccctgctgaaagctctcgtgcggcagcagctgcctgagaagtacaaagagattttcttcgaccagagcaagaacggctacgccggctacattgacggcggagccagccaggaagagttctacaagttcatcaagcccatcctggaaaagatggacggcaccgaggaactgctcgtgaagctgaacagagaggacctgctgcggaagcagcggaccttcgacaacggcagcatcccccaccagatccacctgggagagctgcacgccattctgcggcggcaggaagatttttacccattcctgaaggacaaccgggaaaagatcgagaagatcctgaccttccgcatcccctactacgtgggccctctggccaggggaaacagcagattcgcctggatgaccagaaagagcgaggaaaccatcaccccctggaacttcgaggaagtggtggacaagggcgcttccgcccagagcttcatcgagcggatgaccaacttcgataagaacctgcccaacgagaaggtgctgcccaagcacagcctgctgtacgagtacttcaccgtgtataacgagctgaccaaagtgaaatacgtgaccgagggaatgagaaagcccgccttcctgagcggcgagcagaaaaaggccatcgtggacctgctgttcaagaccaaccggaaagtgaccgtgaagcagctgaaagaggactacttcaagaaaatcgagtgcttcgactccgtggaaatctccggcgtggaagatcggttcaacgcctccctgggcacataccacgatctgctgaaaattatcaaggacaaggacttcctggacaatgaggaaaacgaggacattctggaagatatcgtgctgaccctgacactgtttgaggacagagagatgatcgaggaacggctgaaaacctatgcccacctgttcgacgacaaagtgatgaagcagctgaagcggcggagatacaccggctggggcaggctgagccggaagctgatcaacggcatccgggacaagcagtccggcaagacaatcctggatttcctgaagtccgacggcttcgccaacagaaacttcatgcagctgatccacgacgacagcctgacctttaaagaggacatccagaaagcccaggtgtccggccagggcgatagcctgcacgagcacattgccaatctggccggcagccccgccattaagaagggcatcctgcagacagtgaaggtggtggacgagctcgtgaaagtgatgggccggcacaagcccgagaacatcgtgatcgaaatggccagagagaaccagaccacccagaagggacagaagaacagccgcgagagaatgaagcggatcgaagagggcatcaaagagctgggcagccagatcctgaaagaacaccccgtggaaaacacccagctgcagaacgagaagctgtacctgtactacctgcagaatgggcgggatatgtacgtggaccaggaactggacatcaaccggctgtccgactacgatgtggaccatatcgtgcctcagagctttctgaaggacgactccatcgacaacaaggtgctgaccagaagcgacaagaaccggggcaagagcgacaacgtgccctccgaagaggtcgtgaagaagatgaagaactactggcggcagctgctgaacgccaagctgattacccagagaaagttcgacaatctgaccaaggccgagagaggcggcctgagcgaactggataaggccggcttcatcaagagacagctggtggaaacccggcagatcacaaagcacgtggcacagatcctggactcccggatgaacactaagtacgacgagaatgacaagctgatccgggaagtgaaagtgatcaccctgaagtccaagctggtgtccgatttccggaaggatttccagttttacaaagtgcgcgagatcaacaactaccaccacgcccacgacgcctacctgaacgccgtcgtgggaaccgccctgatcaaaaagtaccctaagctggaaagcgagttcgtgtacggcgactacaaggtgtacgacgtgcggaagatgatcgccaagagcgagcaggaaatcggcaaggctaccgccaagtacttcttctacagcaacatcatgaactttttcaagaccgagattaccctggccaacggcgagatccggaagcggcctctgatcgagacaaacggcgaaaccggggagatcgtgtgggataagggccgggattttgccaccgtgcggaaagtgctgagcatgccccaagtgaatatcgtgaaaaagaccgaggtgcagacaggcggcttcagcaaagagtctatcctgcccaagaggaacagcgataagctgatcgccagaaagaaggactgggaccctaagaagtacggcggcttcgacagccccaccgtggcctattctgtgctggtggtggccaaagtggaaaagggcaagtccaagaaactgaagagtgtgaaagagctgctggggatcaccatcatggaaagaagcagcttcgagaagaatcccatcgactttctggaagccaagggctacaaagaagtgaaaaaggacctgatcatcaagctgcctaagtactccctgttcgagctggaaaacggccggaagagaatgctggcctctgccggcgaactgcagaagggaaacgaactggccctgccctccaaatatgtgaacttcctgtacctggccagccactatgagaagctgaagggctcccccgaggataatgagcagaaacagctgtttgtggaacagcacaagcactacctggacgagatcatcgagcagatcagcgagttctccaagagagtgatcctggccgacgctaatctggacaaagtgctgtccgcctacaacaagcaccgggataagcccatcagagagcaggccgagaatatcatccacctgtttaccctgaccaatctgggagcccctgccgccttcaagtactttgacaccaccatcgaccggaagaggtacaccagcaccaaagaggtgctggacgccaccctgatccaccagagcatcaccggcctgtacgagacacggatcgacctgtctcagctgggaggcgacagccccaagaagaagagaaaggtggaggccagctaaggatccggcaagactggccccgcttggcaacgcaacagtgagcccctccctagtgtgtttggggatgtgactatgtattcgtgtgttggccaacgggtcaacccgaacagattgatacccgccttggcatttcctgtcagaatgtaacgtcagttgatggtact

SEQ ID NO: 89 - DNA, 3150 bp, Artificial Sequence
  source: /note="Description of Artificial Sequence: Synthetic polynucleotide"
tctttcttgcgctatgacacttccagcaaaaggtagggcgggctgcgagacggcttcccggcgctgcatgcaacaccgatgatgcttcgaccccccgaagctccttcggggctgcatgggcgctccgatgccgctccagggcgagcgctgtttaaatagccaggcccccgattgcaaagacattatagcgagctaccaaagccatattcaaacacctagatcactaccacttctacacaggccactcgagcttgtgatcgcactccgctaagggggcgcctcttcctcttcgtttcagtcacaacccgcaaacatgcctaagaagaagaggaaggttaacacgattaacatcgctaagaacgacttctctgacatcgaactggctgctatcccgttcaacactctggctgaccattacggtgagcgtttagctcgcgaacagttggcccttgagcatgagtcttacgagatgggtgaagcacgcttccgcaagatgtttgagcgtcaacttaaagctggtgaggttgcggataacgctgccgccaagcctctcatcactaccctactccctaagatgattgcacgcatcaacgactggtttgaggaagtgaaagctaagcgcggcaagcgcccgacagccttccagttcctgcaagaaatcaagccggaagccgtagcgtacatcaccattaagaccactctggcttgcctaaccagtgctgacaatacaaccgttcaggctgtagcaagcgcaatcggtcgggccattgaggacgaggctcgcttcggtcgtatccgtgaccttgaagctaagcacttcaagaaaaacgttgaggaacaactcaacaagcgcgtagggcacgtctacaagaaagcatttatgcaagttgtcgaggctgacatgctctctaagggtctactcggtggcgaggcgtggtcttcgtggcataaggaagactctattcatgtaggagtacgctgcatcgagatgctcattgagtcaaccggaatggttagcttacaccgccaaaatgctggcgtagtaggtcaagactctgagactatcgaactcgcacctgaatacgctgaggctatcgcaacccgtgcaggtgcgctggctggcatctctccgatgttccaaccttgcgtagttcctcctaagccgtggactggcattactggtggtggctattgggctaacggtcgtcgtcctctggcgctggtgcgtactcacagtaagaaagcactgatgcgctacgaagacgtttacatgcctgaggtgtacaaagcgattaacattgcgcaaaacaccgcatggaaaatcaacaagaaagtcctagcggtcgccaacgtaatcaccaagtggaagcattgtccggtcgaggacatccctgcgattgagcgtgaagaactcccgatgaaaccggaagacatcgacatgaatcctgaggctctcaccgcgtggaaacgtgctgccgctgctgtgtaccgcaaggacaaggctcgcaagtctcgccgtatcagccttgagttcatgcttgagcaagccaataagtttgctaaccataaggccatctggttcccttacaacatggactggcgcggtcgtgtttacgctgtgtcaatgttcaacccgcaaggtaacgatatgaccaaaggactgcttacgctggcgaaaggtaaaccaatcggtaaggaaggttactactggctgaaaatccacggtgcaaactgtgcgggtgtcgacaaggttccgttccctgagcgcatcaagttcattgaggaaaaccacgagaacatcatggcttgcgctaagtctccactggagaacacttggtgggctgagcaagattctccgttctgcttccttgcgttctgctttgagtacgctggggtacagcaccacggcctgagctataactgctcccttccgctggcgtttgacgggtcttgctctggcatccagcacttctccgcgatgctccgagatgaggtaggtggtcgcgcggttaacttgcttcctagtgaaaccgttcaggacatctacgggattgttgctaagaaagtcaacgagattctacaagcagacgcaatcaatgggaccgataacgaagtagttaccgtgaccgatgagaacactggtgaaatctctgagaaagtcaagctgggcactaaggcactggctggtcaatggctggcttacggtgttactcgcagtgtgactaagcgttcagtcatgacgctggcttacgggtccaaagagttcggcttccgtcaacaagtgctggaagataccattcagccagctattgattccggcaagggtctgatgttcactcagccgaatcaggctgctggatacatggctaagctgatttgggaatctgtgagcgtgacggtggtagctgcggttgaagcaatgaactggcttaagtctgctgctaagctgctggctgctgaggtcaaagataagaagactggagagattcttcgcaagcgttgcgctgtgcattgggtaactcctgatggtttccctgtgtggcaggaatacaagaagcctattcagacgcgcttgaacctgatgttcctcggtcagttccgcttacagcctaccattaacaccaacaaagatagcgagattgatgcacacaaacaggagtctggtatcgctcctaactttgtacacagccaagacggtagccaccttcgtaagactgtagtgtgggcacacgagaagtacggaatcgaatcttttgcactgattcacgactccttcggtacgattccggctgacgctgcgaacctgttcaaagcagtgcgcgaaactatggttgacacatatgagtcttgtgatgtactggctgatttctacgaccagttcgctgaccagttgcacgagtctcaattggacaaaatgccagcacttccggctaaaggtaacttgaacctccgtgacatcttagagtcggacttcgcgttcgcgtaaggatccggcaagactggccccgcttggcaacgcaacagtgagcccctccctagtgtgtttggggatgtgactatgtattcgtgtgttggccaacgggtcaacccgaacagattgatacccgccttggcatttcctgtcagaatgtaacgtcagttgatggtact

SEQ ID NO: 90 - DNA, 125 bp, Artificial Sequence
  source: /note="Description of Artificial Sequence: Synthetic polynucleotide"
  modified_base (23)..(42): a, c, t, g, unknown or other
gaaattaatacgactcactatannnnnnnnnnnnnnnnnnnngttttagagctagaaatagcaagttaaaataaggctagtccgttatcaacttgaaaaagtggcaccgagtcggtgcttttttt

SEQ ID NO: 91 - DNA, 8452 bp, Artificial Sequence
  source: /note="Description of Artificial Sequence: Synthetic polynucleotide"
tgcggtatttcacaccgcatcaggtggcacttttcggggaaatgtgcgcggaacccctatttgtttatttttctaaatacattcaaatatgtatccgctcatgagattatcaaaaaggatcttcacctagatccttttaaattaaaaatgaagttttaaatcaatctaaagtatatatgagtaaacttggtctgacagttaccaatgcttaatcagtgaggcacctatctcagcgatctgtctatttcgttcatccatagttgcctgactccccgtcgtgtagataactacgatacgggagggcttaccatctggccccagtgctgcaatgataccgcgagacccacgctcaccggctccagatttatcagcaataaaccagccagccggaagggccgagcgcagaagtggtcctgcaactttatccgcctccatccagtctattaattgttgccgggaagctagagtaagtagttcgccagttaatagtttgcgcaacgttgttgccattgctacaggcatcgtggtgtcacgctcgtcgtttggtatggcttcattcagctccggttcccaacgatcaaggcgagttacatgatcccccatgttgtgcaaaaaagcggttagctccttcggtcctccgatcgttgtcagaagtaagttggccgcagtgttatcactcatggttatggcagcactgcataattctcttactgtcatgccatccgtaagatgcttttctgtgactggtgagtactcaaccaagtcattctgagaatagtgtatgcggcgaccgagttgctcttgcccggcgtcaatacgggataataccgcgccacatagcagaactttaaaagtgctcatcattggaaaacgttcttcggggcgaaaactctcaaggatcttaccgctgttgagatccagttcgatgtaacccactcgtgcacccaactgatcttcagcatcttttactttcaccagcgtttctgggtgagcaaaaacaggaaggcaaaatgccgcaaaaaagggaataagggcgacacggaaatgttgaatactcatactcttcctttttcaatattattgaagcatttatcagggttattgtctcatgaccaaaatcccttaacgtgagttttcgttccactgagcgtcagaccccgtagaaaagatcaaaggatcttcttgagatcctttttttctgcgcgtaatctgctgcttgcaaacaaaaaaaccaccgctaccagcggtggtttgtttgccggatcaagagctaccaactctttttccgaaggtaactggcttcagcagagcgcagataccaaatactgttcttctagtgtagccgtagttaggccaccacttcaagaactctgtagcaccgcctacatacctcgctctgctaatcctgttaccagtggctgttgccagtggcgataagtcgtgtcttaccgggttggactcaagacgatagttaccggataaggcgcagcggtcgggctgaacggggggttcgtgcacacagcccagcttggagcgaacgacctacaccgaactgagatacctacagcgtgagctatgagaaagcgccacgcttcccgaagggagaaaggcggacaggtatccggtaagcggcagggtcggaacaggagagcgcacgagggagcttccagggggaaacgcctggtatctttatagtcctgtcgggtttcgccacctctgacttgagcgtcgatttttgtgatgctcgtcaggggggcggagcctatggaaaaacgccagcaacgcggcctttttacggttcctggccttttgctggccttttgctcacatgttctttcctgcgttatcccctgattctgtggataaccgtattaccgcctttgagtgagctgataccgctcgccgcagccgaacgaccgagcgcagcgagtcagtgagcgaggaagcggtcgctgaggcttgacatgattggtgcgtatgtttgtatgaagctacaggactgatttggcgggctatgagggcgggggaagctctggaagggccgcgatggggcgcgcggcgtccagaaggcgccatacggcccgctggcggcacccatccggtataaaagcccgcgaccccgaacggtgacctccactttcagcgacaaacgagcacttatacatacgcgactattctgccgctatacataaccactcagctagcttaagatcccatcaagcttgcatgccgggcgcgccagaaggagcgcagccaaaccaggatgatgtttgatggggtatttgagcacttgcaacccttatccggaagccccctggcccacaaaggctaggcgccaatgcaagcagttcgcatgcagcccctggagcggtgccctcctgataaaccggccagggggcctatgttctttacttttttacaagagaagtcactcaacatcttaaaatggccaggtgagtcgacgagcaagcccggcggatcaggcagcgtgcttgcagatttgacttgcaacgcccgcattgtgtcgacgaaggcttttggctcctctgtcgctgtctcaagcagcatctaaccctgcgtcgccgtttccatttgcaggagattcgaggtaccatgtacccatacgatgttccagattacgcttcgccgaagaaaaagcgcaaggtcgaagcgtccgacaagaagtacagcatcggcctggacatcggcaccaactctgtgggctgggccgtgatcaccgacgagtacaaggtgcccagcaagaaattcaaggtgctgggcaacaccgaccggcacagcatcaagaagaacctgatcggagccctgctgttcgacagcggcgaaacagccgaggccacccggctgaagagaaccgccagaagaagatacaccagacggaagaaccggatctgctatctgcaagagatcttcagcaacgagatggccaaggtggacgacagcttcttccacagactggaagagtccttcctggtggaagaggataagaagcacgagcggcaccccatcttcggcaacatcgtggacgaggtggcctaccacgagaagtaccccaccatctaccacctgagaaagaaactggtggacagcaccgacaaggccgacctgcggctgatctatctggccctggcccacatgatcaagttccggggccacttcctgatcgagggcgacctgaaccccgacaacagcgacgtggacaagctgttcatccagctggtgcagacctacaaccagctgttcgaggaaaaccccatcaacgccagcggcgtggacgccaaggccatcctgtctgccagactgagcaagagcagacggctggaaaatctgatcgcccagctgcccggcgagaagaagaatggcctgttcggcaacctgattgccctgagcctgggcctgacccccaacttcaagagcaacttcgacctggccgaggatgccaaactgcagctgagcaaggacacctacgacgacgacctggacaacctgctggcccagatcggcgaccagtacgccgacctgtttctggccgccaagaacctgtccgacgccatcctgctgagcgacatcctgagagtgaacaccgagatcaccaaggcccccctgagcgcctctatgatcaagagatacgacgagcaccaccaggacctgaccctgctgaaagctctcgtgcggcagcagctgcctgagaagtacaaagagattttcttcgaccagagcaagaacggctacgccggctacattgacggcggagccagccaggaagagttctacaagttcatcaagcccatcctggaaaagatggacggcaccgaggaactgctcgtgaagctgaacagagaggacctgctgcggaagcagcggaccttcgacaacggcagcatcccccaccagatccacctgggagagctgcacgccattctgcggcggcaggaagatttttacccattcctgaaggacaaccgggaaaagatcgagaagatcctgaccttccgcatcccctactacgtgggccctctggccaggggaaacagcagattcgcctggatgaccagaaagagcgaggaaaccatcaccccctggaacttcgaggaagtggtggacaagggcgcttccgcccagagcttcatcgagcggatgaccaacttcgataagaacctgcccaacgagaaggtgctgcccaagcacagcctgctgtacgagtacttcaccgtgtataacgagctgaccaaagtgaaatacgtgaccgagggaatgagaaagcccgccttcctgagcggcgagcagaaaaaggccatcgtggacctgctgttcaagaccaaccggaaagtgaccgtgaagcagctgaaagaggactacttcaagaaaatcgagtgcttcgactccgtggaaatctccggcgtggaagatcggttcaacgcctccctgggcacataccacgatctgctgaaaattatcaaggacaaggacttcctggacaatgaggaaaacgaggacattctggaagatatcgtgctgaccctgacactgtttgaggacagagagatgatcgaggaacggctgaaaacctatgcccacctgttcgacgacaaagtgatgaagcagctgaagcggcggagatacaccggctggggcaggctgagccggaagctgatcaacggcatccgggacaagcagtccggcaagacaatcctggatttcctgaagtccgacggcttcgccaacagaaacttcatgcagctgatccacgacgacagcctgacctttaaagaggacatccagaaagcccaggtgtccggccagggcgatagcctgcacgagcacattgccaatctggccggcagccccgccattaagaagggcatcctgcagacagtgaaggtggtggacgagctcgtgaaagtgatgggccggcacaagcccgagaacatcgtgatcgaaatggccagagagaaccagaccacccagaagggacagaagaacagccgcgagagaatgaagcggatcgaagagggcatcaaagagctgggcagccagatcctgaaagaacaccccgtggaaaacacccagctgcagaacgagaagctgtacctgtactacctgcagaatgggcgggatatgtacgtggaccaggaactggacatcaaccggctgtccgactacgatgtggaccatatcgtgcctcagagctttctgaaggacgactccatcgacaacaaggtgctgaccagaagcgacaagaaccggggcaagagcgacaacgtgccctccgaagaggtcgtgaagaagatgaagaactactggcggcagctgctgaacgccaagctgattacccagagaaagttcgacaatctgaccaaggccgagagaggcggcctgagcgaactggataaggccggcttcatcaagagacagctggtggaaacccggcagatcacaaagcacgtggcacagatcctggactcccggatgaacactaagtacgacgagaatgacaagctgatccgggaagtgaaagtgatcaccctgaagtccaagctggtgtccgatttccggaaggatttccagttttacaaagtgcgcgagatcaacaactaccaccacgcccacgacgcctacctgaacgccgtcgtgggaaccgccctgatcaaaaagtaccctaagctggaaagcgagttcgtgtacggcgactacaaggtgtacgacgtgcggaagatgatcgccaagagcgagcaggaaatcggcaaggctaccgccaagtacttcttctacagcaacatcatgaactttttcaagaccgagattaccctggccaacggcgagatccggaagcggcctctgatcgagacaaacggcgaaaccggggagatcgtgtgggataagggccgggattttgccaccgtgcggaaagtgctgagcatgccccaagtgaatatcgtgaaaaagaccgaggtgcagacaggcggcttcagcaaagagtctatcctgcccaagaggaacagcgataagctgatcgccagaaagaaggactgggaccctaagaagtacggcggcttcgacagccccaccgtggcctattctgtgctggtggtggccaaagtggaaaagggcaagtccaagaaactgaagagtgtgaaagagctgctggggatcaccatcatggaaagaagcagcttcgagaagaatcccatcgactttctggaagccaagggctacaaagaagtgaaaaaggacctgatcatcaagctgcctaagtactccctgttcgagctggaaaacggccggaagagaatgctggcctctgccggcgaactgcagaagggaaacgaactggccctgccctccaaatatgtgaacttcctgtacctggccagccactatgagaagctgaagggctcccccgaggataatgagcagaaacagctgtttgtggaacagcacaagcactacctggacgagatcatcgagcagatcagcgagttctccaagagagtgatcctggccgacgctaatctggacaaagtgctgtccgcctacaacaagcaccgggataagcccatcagagagcaggccgagaatatcatccacctgtttaccctgaccaatctgggagcccctgccgccttcaagtactttgacaccaccatcgaccggaagaggtacaccagcaccaaagaggtgctggacgccaccctgatccaccagagcatcaccggcctgtacgagacacggatcgacctgtctcagctgggaggcgacagccccaagaagaagagaaaggtggaggccagctaacatatgattcgaatgtctttcttgcgctatgacacttccagcaaaaggtagggcgggctgcgagacggcttcccggcgctgcatgcaacaccgatgatgcttcgaccccccgaagctccttcggggctgcatgggcgctccgatgccgctccagggcgagcgctgtttaaatagccaggcccccgattgcaaagacattatagcgagctaccaaagccatattcaaacacctagatcactaccacttctacacaggccactcgagcttgtgatcgcactccgctaagggggcgcctcttcctcttcgtttcagtcacaacccgcaaacatgacacaagaatccctgttacttctcgaccgtattgattcggatgattcctacgcgagcctgcggaacgaccaggaattctgggaggtgagtcgacgagcaagcccggcggatcaggcagcgtgcttgcagatttgacttgcaacgcccgcattgtgtcgacgaaggcttttggctcctctgtcgctgtctcaagcagcatctaaccctgcgtcgccgtttccatttgcagccgctggcccgccgagccctggaggagctcgggctgccggtgccgccggtgctgcgggtgcccggcgagagcaccaaccccgtactggtcggcgagcccggcccggtgatcaagctgttcggcgagcactggtgcggtccggagagcctcgcgtcggagtcggaggcgtacgcggtcctggcggacgccccggtgccggtgccccgcctcctcggccgcggcgagctgcggcccggcaccggagcctggccgtggccctacctggtgatgagccggatgaccggcaccacctggcggtccgcgatggacggcacgaccgaccggaacgcgctgctcgccctggcccgcgaactcggccgggtgctcggccggctgcacagggtgccgctgaccgggaacaccgtgctcaccccccattccgaggtcttcccggaactgctgcgggaacgccgcgcggcgaccgtcgaggaccaccgcgggtggggctacctctcgccccggctgctggaccgcctggaggactggctgccggacgtggacacgctgctggccggccgcgaaccccggttcgtccacggcgacctgcacgggaccaacatcttcgtggacctggccgcgaccgaggtcaccgggatcgtcgacttcaccgacgtctatgcgggagactcccgctacagcctggtgcaactgcatctcaacgccttccggggcgaccgcgagatcctggccgcgctgctcgacggggcgcagtggaagcggaccgaggacttcgcccgcgaactgctcgccttcaccttcctgcacgacttcgaggtgttcgaggagaccccgctggatctctccggcttcaccgatccggaggaactggcgcagttcctctgggggccgccggacaccgcccccggcgcctgataaggatccggcaagactggccccgcttggcaacgcaacagtgagcccctccctagtgtgtttggggatgtgactatgtattcgtgtgttggccaacgggtcaacccgaacagattgatacccgccttggcatttcctgtcagaatgtaacgtcagttgatggtact

SEQ ID NO: 92 - DNA, 102 bp, Artificial Sequence
  source: /note="Description of Artificial Sequence: Synthetic polynucleotide"
gttttagagctatgctgttttgaatggtcccaaaacggaagggcctgagtccgagcagaagaagaagttttagagctatgctgttttgaatggtcccaaaac

SEQ ID NO: 93 - DNA, 100 bp, Homo sapiens
cggaggacaaagtacaaacggcagaagctggaggaggaagggcctgagtccgagcagaagaagaagggctcccatcacatcaaccggtggcgcattgcca

SEQ ID NO: 94 - DNA, 50 bp, Homo sapiens
agctggaggaggaagggcctgagtccgagcagaagaagaagggctcccac

SEQ ID NO: 95 - RNA, 30 nt, Artificial Sequence
  source: /note="Description of Artificial Sequence: Synthetic oligonucleotide"
gaguccgagcagaagaagaaguuuuagagc

SEQ ID NO: 96 - DNA, 49 bp, Artificial Sequence
  source: /note="Description of Artificial Sequence: Synthetic oligonucleotide"
agctggaggaggaagggcctgagtccgagcagaagagaagggctcccat

SEQ ID NO: 97 - DNA, 53 bp, Homo sapiens
ctggaggaggaagggcctgagtccgagcagaagaagaagggctcccatcacat

SEQ ID NO: 98 - DNA, 52 bp, Homo sapiens
ctggaggaggaagggcctgagtccgagcagaagagaagggctcccatcacat

SEQ ID NO: 99 - DNA, 54 bp, Homo sapiens
ctggaggaggaagggcctgagtccgagcagaagaaagaagggctcccatcacat

SEQ ID NO: 100 - DNA, 50 bp, Homo sapiens
ctggaggaggaagggcctgagtccgagcagaagaagggctcccatcacat

SEQ ID NO: 101 - DNA, 47 bp, Homo sapiens
ctggaggaggaagggcctgagcccgagcagaagggctcccatcacat

SEQ ID NO: 102 - RNA, 155 nt, Artificial Sequence
  source: /note="Description of Artificial Sequence: Synthetic polynucleotide"
guuucagugcuauaggaaacuauaggaaaucaccuucgggugagcugaaauccccuaaagcuaagauugaauccggccacuaucuauuaguagauauccggauauucugauauaaaaccucauucuuugauuagaccaaaggaugagguuuuuuu

SEQ ID NO: 103 - RNA, 107 nt, Artificial Sequence
  source: /note="Description of Artificial Sequence: Synthetic polynucleotide"
guuugagaguuggaaacaacgaguucaaauaagaauucaucaaaaucgucccuuuugggaccgcucauuguggagcaucaaggcuuaacaugguuaagccuuuuuuu

SEQ ID NO: 104 - RNA, 99 nt, Artificial Sequence
  source: /note="Description of Artificial Sequence: Synthetic oligonucleotide"
guuugagaguaggaaacuacacgguucaaauaaagaauuuuucuaaucgcccaaugggcccauauugauauggaugaaacucgcuuagcgaguuuuuuu

SEQ ID NO: 105 - RNA, 91 nt, Artificial Sequence
  source: /note="Description of Artificial Sequence: Synthetic oligonucleotide"
guuuuagcacuagaaauaguuaaguuaaaacaagcuuaaagcgucaauguaauauuuuauuaacacccuacugugucagugggguuuuuuu

SEQ ID NO: 106 - RNA, 94 nt, Artificial Sequence
  source: /note="Description of Artificial Sequence: Synthetic oligonucleotide"
guuuuagauggugaaaaccagauuuaaaaucaagcaaugcaucuuuugaugcaaaguuucaauauuugucccacguuaucgagggacuuuuuuu

SEQ ID NO: 107 - RNA, 78 nt, Artificial Sequence
  source: /note="Description of Artificial Sequence: Synthetic oligonucleotide"
auuuuaguaccuggaaacagaucuacuaaaacaaggcuuuaugccgaaaucaagagcaccgacgggugcucuuuuuuu

SEQ ID NO: 108 - RNA, 84 nt, Artificial Sequence
  source: /note="Description of Artificial Sequence: Synthetic oligonucleotide"
guuuuuguacucgaaagagccuacaaagauaaggcuuuaugccgaauucaagcaccccauguuuugacaugaggugcuuuuuuu

SEQ ID NO: 109 - RNA, 85 nt, Artificial Sequence
  source: /note="Description of Artificial Sequence: Synthetic oligonucleotide"
guuuuuguaccuuagaaauaagaucuacaaaaauaaggauuuauuccgaauuuaccaccuauuuuaauuaauaggugguuuuuuu

SEQ ID NO: 110 - RNA, 100 nt, Artificial Sequence
  source: /note="Description of Artificial Sequence: Synthetic polynucleotide"
guugugauuugcuuucauuugaaaaauugaagcaaaucacaauaaggauuauuccguugugaaaacaauuaaagcggucuugcaaaaggucgcuuuuuuu

SEQ ID NO: 111 - RNA, 102 nt, Artificial Sequence
  source: /note="Description of Artificial Sequence: Synthetic polynucleotide"
guugugauucgcuuucaaugaaaauugaagcgaaucacaauaaggauuauuccguugugaaaacauuuacuacggggcaucgaaagacugccucguuuuuuu

SEQ ID NO: 112 - RNA, 90 nt, Artificial Sequence
  source: /note="Description of Artificial Sequence: Synthetic oligonucleotide"
guugugguuugauuagaaauaaucuuaucacaauaaggcuauaugccguagacgaaagucuuuagucccgcuucggugggacuuuuuuuu

SEQ ID NO: 113 - RNA, 78 nt, Artificial Sequence
  source: /note="Description of Artificial Sequence: Synthetic oligonucleotide"
guuggggaugaccgcgaaagcgauuaucucuaauaagacuuaagucgcaaaaugcucccuauuuugggagcuuuuuuu

SEQ ID NO: 114 - RNA, 85 nt, Artificial Sequence
  source: /note="Description of Artificial Sequence: Synthetic oligonucleotide"
guugcggcuggagaaauccagccguuaacauguucccuucggggagcacgaaaugcggggcgggccacgguccgccccuuuuuuu

SEQ ID NO: 115 - RNA, 126 nt, Artificial Sequence
  source: /note="Description of Artificial Sequence: Synthetic polynucleotide"
gccgugguuuccgaaaggaaaccacgguaacagaauuaccguaagguuuuuucugugaaggaucaucccucgcuugggcaaccaggcgggggaaauuccucguucgggccaaucagcccuuuuuuu

SEQ ID NO: 116 - RNA, 82 nt, Artificial Sequence
  source: /note="Description of Artificial Sequence: Synthetic oligonucleotide"
guuguaauucccugaaaagguuauuacaauaagguaagaaaccuaaaagcucuaaucccauucuucggaaugggauuuuuuu

SEQ ID NO: 117 - RNA, 83 nt, Artificial Sequence
  source: /note="Description of Artificial Sequence: Synthetic oligonucleotide"
guuuuaguacucuggaaacagaaucuacuaaaacaaggcaaaaugccguguuuaucucgucaacuuguuggcgagauuuuuuu

SEQ ID NO: 118 - RNA, 94 nt, Artificial Sequence
  source: /note="Description of Artificial Sequence: Synthetic oligonucleotide"
guuuuagcacuguacaagaaauugucgugcuaaaauaaggcgcuguuaaugcagcugccgcauccgccagagcauuuaugcucuggcuuuuuuu

SEQ ID NO: 119 - DNA, 4350 bp, Artificial Sequence
  source: /note="Description of Artificial Sequence: Synthetic polynucleotide"
accggtgccaccatgtacccatacgatgttccagattacgcttcgccgaagaaaaagcgcaaggtcgaagcgtccatgactcagagcgagcgacgattttcttgcagcattggcattgacatgggggctaagtacactggggtgttctacgcactgttcgaccgggaggaactgcccacaaacctgaacagcaaggccatgaccctggtcatgcctgagacagggccaagatacgtgcaggcacagagaactgccgtcagacacaggctgcgcggacagaagagatataccctggctaggaaactggcatttctggtggtcgacgatatgatcaagaaacaggaaaagaggctgactgatgaggaatggaaacgaggacgggaggccctgtccggcctgctgaagcggagagggtactctcggcccaacgctgacggcgaagatctgacccctctggagaatgtgagagcagacgtgttcgccgctcatcctgccttcagcacatatttttccgaagtgcgctctctggctgagcagtgggaggagttcaccgcaaacatcagcaatgtcgagaagtttctgggcgacccaaacatccccgccgataaagagttcattgaatttgccgtggctgaagggctgattgacaagaccgagaagaaagcctaccagtcagctctgagcaccctgagggcaaacgccaatgtgctgacaggactgcggcagatgggccacaagcctagatcagaatattttaaagcaatcgaggccgacctgaagaaagatagccgcctggccaagattaacgaagcattcggaggagcagagcgcctggctcgactgctgggaaacctgtccaatctgcagctgcgggcagaaagatggtacttcaatgcccccgacatcatgaaggataggggctgggagcctgatcgcttcaagaaaacactggtgcgggcttttaagttctttcacccagcaaaggaccagaacaaacagcatctggaactgatcaaacagattgagaacagcgaagatatcattgagactctgtgcaccctggacccaaacagaaccatccccccttacgaggatcagaacaataggcgcccacccctggaccagactctgctgctgagtcccgaaaagctgacccggcagtatggcgagatctggaaaacatggagcgccagactgacctccgctgaacccacactggcacctgcagccgagattctggaaagatctaccgacaggaagagtcgcgtggcagtcaacggacacgagccactgcctacactggcttaccagctgagttatgcactgcagagagccttcgacaggtcaaaagccctggatccatatgctctgagggcactggctgcaggctcaaaaagcaataagctgacatccgcccgcactgctctggagaactgcatcggaggccagaatgtgaaaaccttcctggactgtgcccgacggtactatcgggaagcagacgatgccaaagtcgggctgtggttcgacaacgccgatggactgctggagagatctgacctgcatcctccaatgaagaaaaagatcctgcccctgctggtggccaatattctgcagacagatgaaaccacaggccagaagtttctggacgagatctggcgaaaacagattaaggggcgggaaactgtggctagccgatgtgcacggatcgagacagtgcggaaatccttcgggggaggctttaacattgcctacaataccgctcagtatagggaggtgaacaagctgccccgcaatgcccaggataaagaactgctgacaatcagagatagggtggctgagactgcagacttcattgccgctaacctggggctgtctgacgagcagaaaagaaagttcgccaatccttttagtctggctcagttctacaccctgatcgagacagaagtgtccggattttctgcaactaccctggccgtccacctggagaacgcctggaggatgacaatcaaggatgctgtgattaatggggaaactgtcagagcagcacagtgcagcaggctgcctgcagagacagctcgcccattcgatggactggtgagaaggctggtcgacagacaggcttgggagatcgcaaagagggtgtcaactgacattcagagcaaagtcgatttctccaacggcatcgtggacgtcagcatttttgtggaggaaaataagttcgagttttccgcatctgtggccgatctgaaaaagaacaaacgggtcaaagacaagatgctgtccgaggccgaaaagctggaaaccagatggctgatcaaaaatgagcggatcaagaaggccagccggggaacttgtccctacaccggcgataggctggctgaggggggagaaatcgaccacattctgccccgaagcctgatcaaggatgcccggggaattgtgtttaacgctgagcctaatctgatctatgcaagctcccgcggcaaccagctgaaaaagaatcagcgatacagtctgtcagatctgaaggccaactatcggaatgagatcttcaaaactagcaacatcgctgcaattaccgccgagattgaggacgtggtcactaagctgcagcagacccatagactgaaattctttgatctgctgaatgagcacgaacaggactgcgtgcggcacgccctgttcctggacgatggcagcgaagctcgcgacgcagtgctggagctgctggcaacacagcgccgaactcgcgtcaacgggacacagatctggatgattaagaacctggccaacaagatccgagaggaactgcagaattggtgtaagacaactaacaatagactgcactttcaggccgctgcaactaacgtgtccgatgcaaagaatctgaggctgaaactggcccagaaccagcccgacttcgagaagccagatatccagcccattgccagccattccatcgacgccctgtgctctttcgctgtggggagtgctgacgcagaacgcgatcagaatggatttgactacctggatggcaagaccgtgctgggactgtatccacagagctgtgaggtcattcacctgcaggccaagccccaggaggaaaaaagtcatttcgattcagtggctatctttaaggaaggcatctacgcagagcagttcctgcctatctttaccctgaacgaaaagatctggattggatatgagacactgaatgccaaaggcgaaagatgcggggctattgaggtgagtggcaaacagccaaaggagctgctggaaatgctggcccccttctttaacaagcctgtgggcgacctgtcagcccacgctacttaccggatcctgaaaaagcctgcatatgagtttctggcaaaggcagctctgcagccactgagcgcagaggaaaaaagactggcagccctgctggatgctctgcgctactgtaccagtcgaaagtcactgatgagcctgttcatggctgcaaacgggaaatccctgaaaaagcgggaggacgtgctgaaacccaagctgttccagctgaaggtcgagctgaaaggcgaaaagagcttcaagctgaacgggagcctgaccctgcctgtgaagcaggactggctgagaatctgcgatagcccagaactggcagacgcctttggcaaaccctgttccgccgatgagctgacatctaagctggctcgcatttggaaacgacctgtgatgcgggatctggctcatgcaccagtccggagagagttcagcctgcccgcaatcgacaacccaagtggagggttcaggattaggcgcaccaacctgtttggcaatgagctgtaccaggtgcacgccatcaacgctaaaaagtatcgcggcttcgcctccgctgggtctaatgtcgactggtccaaggggatcctgtttaacgagctgcagcatgaaaatctgaccgagtgcggaggcaggttcattacaagcgccgatgtgactcctatgtccgaatggcgcaaggtggtcgcagaggacaacctgtctatctggattgctccagggacagaaggacgacggtacgtgagggtcgagacaacattcatccaggccagtcactggtttgaacagtcagtggagaattgggccattactagtcctctgtcactgccagcttccttcaaggtggacaaaccagctgagtttcagaaggcagtcggaaccgagctgtcagaactgctgggccagcccaggagcgaaatcttcattgagaacgtgggcaatgccaagcatatccgcttttggtacattgtggtgagcagcaacaaaaagatgaacgagtcttacaacaatgtgtctaagagttaagaattc

SEQ ID NO: 120 - DNA, 4269 bp, Artificial Sequence
  source: /note="Description of Artificial Sequence: Synthetic polynucleotide"
accggtgccaccatgtacccatacgatgttccagattacgcttcgccgaagaaaaagcgcaaggtcgaagcgtccatgaaaaaagaaatcaaagactacttcctggggctggatgtggggactgggagcgtggggtgggctgtgaccgatactgactacaaactgctgaaggctaaccgaaaagacctgtggggcatgagatgcttcgagacagccgaaactgctgaggtgcggagactgcacaggggagccaggcgccgaatcgagcggagaaagaaacgcattaagctgctgcaggagctgttctctcaggaaatcgccaaaaccgatgagggcttctttcagagaatgaaggaaagccccttttacgctgaggacaaaacaatcctgcaggaaaacactctgttcaatgacaaggattttgctgataagacttaccacaaagcatatcctaccattaatcatctgatcaaggcttggattgagaacaaggtgaaaccagacccccgactgctgtacctggcatgtcacaacatcattaagaaaaggggacatttcctgtttgaaggcgacttcgattcagagaatcagtttgataccagcatccaggcactgttcgagtatctgcgcgaggacatggaggtggacatcgatgccgacagccagaaggtcaaagagattctgaaggatagctccctgaagaactctgaaaaacagagtcggctgaataagatcctggggctgaagccttccgacaaacagaagaaagccatcacaaacctgatttctggaaacaagatcaatttcgccgatctgtacgacaatccagatctgaaggacgctgagaaaaactcaatcagcttctccaaggacgattttgatgcactgagtgacgatctggcctcaattctgggcgacagctttgaactgctgctgaaggccaaagctgtctataactgctctgtgctgagtaaggtcatcggggacgagcagtacctgagcttcgccaaggtgaaaatctacgaaaagcacaaaaccgatctgacaaagctgaaaaacgtgatcaagaaacatttccccaaggactacaagaaggtctttggatacaacaagaacgagaaaaacaacaacaattactccggctatgtgggagtctgtaagaccaagagtaagaaactgatcattaacaactcagtcaaccaggaagatttctacaagtttctgaaaactatcctgtcagccaagagcgagatcaaggaagtgaatgacatcctgaccgagattgaaactggcacctttctgccaaagcagatctctaaaagtaacgcagagattccctatcagctgaggaaaatggagctggaaaagatcctgtccaatgccgaaaagcacttctcttttctgaagcagaaagacgaaaaaggactgtcacatagcgagaagatcattatgctgctgaccttcaagatcccttactatattggcccaatcaacgataatcacaagaaattctttcccgacagatgctgggtggtcaagaaagagaaatccccttctggcaagaccacaccatggaacttctttgatcatatcgacaaggaaaaaacagcagaggccttcattacttctaggaccaatttttgcacttacctggtgggagagagcgtcctgcctaagtctagtctgctgtactccgaatataccgtgctgaacgagatcaacaatctgcagatcattatcgatggcaagaatatttgtgacatcaagctgaaacagaagatctacgaggacctgttcaagaagtacaagaaaattacccagaagcagatcagcaccttcatcaagcacgaaggcatctgcaacaaaaccgatgaagtgatcatcctggggattgacaaggaatgtacatcaagcctgaaaagctacatcgagctgaaaaacattttcggcaagcaggtggatgagatctccactaagaatatgctggaggaaattatcagatgggctaccatctacgacgagggggaaggaaagaccatcctgaaaacaaagatcaaggcagaatacggaaagtattgctccgacgagcagattaagaaaatcctgaacctgaagttctccggctgggggcgactgtctcggaaatttctggagacagtgactagtgaaatgcccggcttctcagaacctgtcaatattatcaccgccatgagggagacacagaacaatctgatggagctgctgtcctctgagttcaccttcaccgagaacattaagaaaatcaattctggattcgaagatgccgagaagcagtttagttacgacggcctggtgaaaccactgtttctgagtccctcagtcaagaaaatgctgtggcagaccctgaagctggtgaaagagattagccatatcacacaggccccccctaagaaaattttcatcgaaatggcaaagggggccgagctggaacctgctcggactaagaccagactgaaaatcctgcaggatctgtataacaattgtaagaacgatgctgacgccttcagctcagagatcaaagacctgagcggaaagattgagaacgaagataatctgaggctgcgctccgacaagctgtacctgtactatactcagctggggaaatgcatgtattgtggaaagccaattgagatcggccacgtgttcgatacctcaaactacgatattgaccatatctatccccagagcaagatcaaagacgatagcatttccaatcgggtgctggtctgcagctcctgtaacaagaacaaggaggacaagtacccactgaaatcagagatccagagcaagcagcgcggcttctggaactttctgcagcgaaacaatttcatttctctggagaagctgaatagactgacaagggccactccaatcagtgacgatgagacagccaagtttattgctaggcagctggtggaaactcgccaggctaccaaggtggccgctaaagtcctggaaaagatgttccccgagacaaaaatcgtgtacagcaaggccgagactgtctccatgttccggaacaagtttgatatcgtgaagtgcagagaaattaacgattttcaccatgctcacgacgcatacctgaatatcgtggtcggcaacgtgtataataccaagttcacaaacaatccttggaactttatcaaggagaaaagagataatccaaagattgctgacacctacaactactataaggtgttcgattatgacgtcaaaaggaacaatatcacagcatgggagaaggggaaaactattatcaccgtgaaagacatgctgaagagaaacacaccaatctacactaggcaggcagcctgtaagaaaggggagctgttcaatcagaccattatgaagaaaggactgggccagcaccccctgaagaaagaaggacctttttccaatatctctaaatacggcgggtataacaaggtgagcgctgcatactatacactgattgagtatgaggaaaagggcaacaaaatccgctccctggaaactattcccctgtacctggtgaaagatatccagaaggatcaggacgtcctgaagtcttatctgacagacctgctggggaagaaagagttcaagatcctggtgcccaagatcaagatcaacagcctgctgaagatcaatgggtttccttgccatattacaggaaaaactaacgatagtttcctgctgcgccctgccgtgcagttttgctgttcaaacaatgaggtcctgtacttcaagaaaattatccggttttccgaaatccgctctcagcgagagaagatcgggaaaacaattagcccatacgaggacctgagcttccggtcatatatcaaggagaacctgtggaagaaaactaagaacgatgaaatcggagagaaggaattttacgacctgctgcagaagaaaaacctggagatctatgatatgctgctgactaagcacaaagacaccatctacaagaaacgccctaattctgccaccattgatatcctggtgaaggggaaagagaagttcaaaagcctgattatcgaaaaccagtttgaagtgatcctggagatcctgaagctgttttctgcaacacggaatgtcagtgacctgcagcatatcggaggcagcaagtactccggcgtggccaaaatcgggaacaagatctctagtctggataactgtatcctgatctatcagtccatcaccggcatcttcgagaaacggatcgacctgctgaaggtgtaagaattc

SEQ ID NO: 121 - DNA, 4179 bp, Artificial Sequence
  source: /note="Description of Artificial Sequence: Synthetic polynucleotide"
accggtgccaccatgtacccatacgatgttccagattacgcttcgccgaagaaaaagcgcaaggtcgaagcgtccatgaccaaggagtattacctggggctggatgtggggaccaattccgtgggatgggcagtgaccgattctcagtacaacctgtgcaagtttaagaaaaaggatatgtggggcatccggctgttcgaaagcgccaacacagcaaaggaccggagactgcagagagggaataggcgccgactggagcggaaaaagcagagaattgatctgctgcaggaaatcttctccccagagatctgcaagattgaccccactttctttatccgactgaacgaatcccggctgcacctggaggacaagtctaacgatttcaaatacccactgtttattgagaaggactattctgatatcgagtactataaagagttccccaccatttttcacctgaggaagcatctgatcgagagtgaggaaaaacaggatatccggctgatctacctggccctgcacaacatcattaagacccgaggacattttctgattgacggcgatctgcagagcgccaagcagctgaggcccatcctggatacattcctgctgtccctgcaggaggaacagaacctgtcagtgagcctgtccgaaaatcagaaggacgagtatgaggaaattctgaaaaaccgcagcatcgccaagtccgaaaaagtgaaaaagctgaagaatctgtttgagatctcagacgagctggaaaaagaggagaagaaggcccagagcgccgtgatcgagaacttctgcaagtttatcgtgggaaataagggcgatgtctgtaaattcctgcgggtgtctaaggaggaactggagattgactctttcagtttttcagagggcaagtacgaggacgacatcgtgaaaaacctggaggaaaaagtgcctgaaaaggtctacctgtttgagcagatgaaggcaatgtatgattggaatattctggtcgacatcctggaaaccgaggaatacatcagcttcgccaaagtgaagcagtatgagaaacacaagactaacctgcggctgctgagagacatcattctgaaatactgcaccaaggatgagtataatcggatgtttaacgacgagaaggaagctggcagctacaccgcatatgtggggaaactgaaaaagaacaacaagaagtactggatcgagaaaaagagaaatcccgaggagttctacaaatccctgggcaagctgctggataaaattgagcctctgaaggaggacctggaagtgctgactatgatgatcgaggagtgtaagaaccacaccctgctgccaattcagaaaaataaggacaacggcgtgatcccccaccaggtgcatgaggtcgaactgaaaaagatcctggaaaatgccaaaaagtactattccttcctgaccgagacagacaaggatgggtactcagtggtccagaaaatcgagagcattttcaggtttcgcatcccctactatgtggggcctctgagtacccggcaccaggaaaagggatcaaacgtgtggatggtcagaaaacctggcagggaggatcgcatctacccatggaatatggaggaaatcattgactttgagaagagcaacgaaaatttcattacacggatgactaacaaatgtacatatctgatcggggaagatgtcctgcccaagcattctctgctgtacagtaaatatatggtgctgaatgagctgaacaatgtgaaggtcagaggaaaaaagctgcctacatctctgaaacagaaggtgttcgaggacctgtttgaaaacaaatccaaagtgactggaaagaatctgctggagtacctgcagatccaggacaaagatatccagattgacgatctgtctggcttcgacaaggacttcaagaccagcctgaagagctatctggacttcaaaaagcagatttttggggaggaaatcgagaaggaaagcattcagaacatgatcgaagatatcattaagtggatcaccatctacggcaatgacaaggagatgctgaaacgagtgattcgggctaattatagcaaccagctgacagaggaacagatgaaaaagatcactggatttcagtacagtggctgggggaacttctcaaagatgtttctgaaagggatcagcggatccgacgtgagcaccggcgaaacattcgacatcattaccgcaatgtgggagacagacaacaatctgatgcagatcctgtcaaaaaagttcacctttatggacaacgtcgaggacttcaacagcggcaaggtcgggaaaatcgacaagattacttacgatagcaccgtgaaggaaatgttcctgtcccctgagaacaaaagggccgtctggcagaccattcaggtggctgaggagatcaagaaagtgatgggctgcgagccaaaaaagatctttattgaaatggcacggggcggggagaaggtgaaaaagaggacaaaatctcgcaaggcccagctgctggagctgtacgccgcttgcgaggaagattgtagagaactgatcaaggagattgaggaccgggacgagagggacttcaatagcatgaagctgtttctgtactatacccagttcgggaaatgtatgtattccggcgacgacatcgatattaacgagctgattcgcggcaattctaagtgggaccgagatcacatctacccccagagcaaaattaaggacgattccatcgataacctggtgctggtcaataagacatataatgccaaaaagtccaatgagctgctgtctgaggacatccagaaaaagatgcattcattctggctgagcctgctgaacaaaaagctgatcactaaaagcaagtacgaccgcctgactcgaaagggcgactttaccgatgaggaactgagtgggttcatcgctagacagctggtggaaacaaggcagtcaactaaggcaatcgccgatatcttcaagcagatctacagctccgaggtggtctatgtgaagagcagcctggtgagcgacttcaggaaaaagccactgaactacctgaagtctcggagagtcaatgattaccaccatgcaaaagacgcctatctgaacattgtggtcgggaacgtgtacaacaaaaagtttaccagtaatcccatccagtggatgaaaaagaatcgcgatacaaactatagcctgaacaaggtgttcgaacacgacgtggtcattaacggagaagtgatctgggaaaagtgcacataccatgaggacactaatacctatgatggaggcactctggaccgaatccggaagattgtggaacgcgataacattctgtacaccgagtacgcttattgtgagaagggcgaactgtttaatgcaaccatccagaacaaaaatggaaactccacagtctctctgaaaaagggcctggacgtgaaaaagtacgggggatacttcagcgccaacacaagttacttctcactgatcgagtttgaggacaagaagggggatagagcaaggcacatcattggagtgcctatctatattgcaaacatgctggagcattctccaagtgccttcctggagtactgcgaacagaaggggtatcagaatgtgcggattctggtcgagaaaatcaaaaagaacagcctgctgatcattaatggataccctctgcgcattcgaggcgagaacgaagtggatacttcctttaagagggccatccagctgaagctggaccagaaaaactatgagctggtccgcaatatcgagaagttcctggaaaaatacgtggagaaaaagggaaactatccaattgacgagaatagagatcacatcacacatgaaaagatgaaccagctgtacgaggtgctgctgtccaaaatgaaaaagttcaacaagaagggcatggccgacccctctgataggatcgaaaagagtaagcctaaattcatcaagctggaggacctgatcgataagattaatgtgatcaacaaaatgctgaacctgctgcgctgtgacaatgatactaaggccgacctgtctctgattgagctgcccaaaaacgctgggagtttcgtggtcaaaaagaataccatcggaaagtcaaaaatcatcctggtgaatcagagcgtgactggactgtacgagaatagacgggaactgtaagaattc

SEQ ID NO: 122 - DNA, 4086 bp, Artificial Sequence
  source: /note="Description of Artificial Sequence: Synthetic polynucleotide"
accggtgccaccatgtacccatacgatgttccagattacgcttcgccgaagaaaaagcgcaaggtcgaagcgtccatggggaggaaaccttacattctgtctctggatattggaactgggtccgtcggctacgcttgcatggataaaggattcaacgtgctgaagtaccacgacaaagatgccctgggagtgtatctgttcgacggcgctctgactgcacaggagcggagacagtttaggacctccaggcgccgaaagaaccggagaatcaaacgcctgggcctgctgcaggaactgctggcacccctggtgcagaaccctaatttctaccagtttcagcggcagttcgcctggaagaacgacaatatggattttaagaacaagagcctgtctgaggtgctgagcttcctgggatatgaatccaagaaataccctaccatctaccacctgcaggaggctctgctgctgaaagacgagaagtttgatccagaactgatctacatggcactgtatcatctggtgaaatacagaggccactttctgttcgatcatctgaagatcgagaacctgactaacaatgacaatatgcacgatttcgtggagctgattgaaacctatgagaacctgaacaatatcaagctgaatctggactacgagaaaaccaaagtgatctatgagattctgaaagacaacgaaatgactaagaatgatagagccaaaagggtcaagaacatggagaagaaactggaacagttctctatcatgctgctggggctgaagttcaatgagggaaaactgtttaaccacgccgataatgctgaggaactgaagggggctaaccagagccatacatttgcagacaactacgaggaaaatctgactcccttcctgaccgtggaacagtcagagtttattgaaagggccaacaaaatctatctgagcctgactctgcaggatatcctgaagggcaagaaatcaatggctatgagcaaagtggccgcttacgacaagttcagaaatgagctgaaacaggtgaaggacattgtctataaggctgattctaccaggacacagttcaagaaaatctttgtgagctccaagaaaagtctgaagcagtacgacgcaactcccaacgatcagaccttctctagtctgtgcctgtttgaccagtacctgattcgcccaaagaaacagtatagcctgctgatcaaggagctgaagaaaatcattccccaggactccgaactgtactttgaggcagaaaatgataccctgctgaaggtgctgaacaccacagacaatgctagcatccctatgcagattaacctgtacgaggcagaaaccatcctgcgaaatcagcagaaatatcacgccgagatcacagatgagatgattgaaaaggtgctgtctctgatccagttccgcattccatactatgtggggcccctggtcaacgaccatacagccagtaagtttggatggatggagcgcaaaagtaacgaatcaatcaagccttggaatttcgacgaggtggtcgatcgaagtaaatcagccactcagtttattaggcgcatgaccaacaagtgttcctacctgatcaatgaggatgtgctgccaaaaaactctctgctgtatcaggagatggaagtcctgaacgaactgaatgccacacagatcaggctgcagactgacccaaaaaaccgcaagtaccgaatgatgccccagattaagctgttcgctgtggagcacatctttaagaaatataaaaccgtcagccattccaagttcctggaaattatgctgaacagcaatcacagggagaactttatgaatcatggagaaaagctgagtatcttcggcacacaggacgataagaaatttgcatcaaagctgtcaagctaccaggacatgactaaaatcttcggggatattgagggaaagcgcgcccagattgaggaaatcattcagtggatcaccatttttgaggacaagaaaatcctggtgcagaagctgaaagagtgctatcctgaactgacatccaagcagatcaaccagctgaagaaactgaattactctggctgggggaggctgagtgagaagctgctgactcacgcctatcagggccatagcatcattgaactgctgcgccactccgatgagaatttcatggaaattctgaccaacgacgtgtacgggttccagaattttatcaaagaggaaaaccaggtccagagcaataagatccagcatcaggatattgccaacctgactacctctcccgctctgaagaaaggcatctggagtacaattaagctggtgcgggagctgacttccattttcggggagcctgaaaagatcattatggagtttgctaccgaggaccagcagaaaggcaagaaacagaaatcaagaaagcagctgtgggacgataacatcaagaaaaataagctgaaaagcgtggacgagtacaaatatatcattgatgtcgccaataagctgaacaatgagcagctgcagcaggaaaaactgtggctgtacctgagccagaacggcaagtgtatgtatagcgggcagtccatcgacctggatgccctgctgtcccccaatgctaccaagcactacgaggtggatcatattttccctcggagcttcatcaaggacgatagcattgacaacaaggtgctggtcatcaagaaaatgaatcagacaaagggcgatcaggtgcccctgcagttcattcagcagccttacgagagaatcgcatattggaagagcctgaacaaagccgggctgatctctgatagtaaactgcacaagctgatgaaaccagagttcacagctatggacaaggaaggcttcatccagcggcagctggtggagactagacagatcagcgtgcatgtccgggattttctgaaagaggaataccctaataccaaagtgatcccaatgaaggccaaaatggtgagcgagttccggaagaaatttgacatcccaaagattagacagatgaacgacgcacaccatgccatcgatgcttacctgaatggcgtggtctatcacggggcacagctggcctaccccaacgtggacctgtttgatttcaattttaagtgggagaaagtccgagaaaagtggaaagccctgggagagttcaacacaaagcagaaatctcgggaactgttctttttcaagaaactggagaagatggaagtgtcccagggcgagcggctgatctctaagatcaagctggacatgaaccacttcaagatcaactactccagaaagctggccaacatccctcagcagttttataatcagaccgcagtgtctccaaagacagccgagctgaaatacgaatctaacaagagtaatgaggtggtctataagggactgacaccataccagacttatgtggtcgccatcaagagcgtgaacaagaaaggcaaggagaaaatggaataccagatgatcgaccactacgtgttcgatttttataaattccagaacggcaatgagaaggaactggctctgtacctggcacagagggagaacaaggacgaagtgctggatgctcagattgtctatagtctgaataagggggatctgctgtacatcaacaatcatccctgctatttcgtgtcacgcaaagaggtcatcaacgcaaagcagtttgagctgaccgtggaacagcagctgtctctgtacaacgtgatgaacaacaaggagacaaatgtcgaaaagctgctgatcgagtatgacttcattgccgagaaagtgatcaacgaataccaccattatctgaatagcaagctgaaagaaaagcgagtccggacctttttctcagagagcaaccagacacacgaggacttcatcaaggccctggacgagctgtttaaggtggtcaccgcatccgccacaaggtctgataaaatcgggagtcgcaagaacagcatgactcatcgagccttcctgggaaaaggcaaggacgtgaagattgcttacacctccatctctggactgaaaacaactaaacctaagagtctgtttaagctggccgagtcaagaaacgaactgtaagaattc

SEQ ID NO: 123 - DNA, 4209 bp, Artificial Sequence
  source: /note="Description of Artificial Sequence: Synthetic polynucleotide"
accggtgccaccatgtacccatacgatgttccagattacgcttcgccgaagaaaaagcgcaaggtcgaagcgtccatgacaaaaatcaaagacgactacatcgtgggactggacatcggcacagactcctgcgggtgggtggctatgaacagcaataatgacattctgaaactgcagggcaagaccgcaatcgggtcacgcctgttcgagggagggaagagcgcagctgaacggagactgtttcgcaccacacacaggcgcatcaaacgacggagatggcgactgaagctgctggaggagttcttcgacccctacatggcagaggtggatccttatttctttgcccggctgaaggaatctggcctgagtccactggacaaaagaaagaccgtgagctccattgtgttccccacatccgccgaggataagaagttctacgacgattaccctacaatctaccatctgaggtataaactgatgactgaggacgaaaagttcgatctgcgcgaagtgtacctggctatccaccatatcattaagtaccgaggaaacttcctgtataataccagtgtgaaagacttcaaggcatcaaagatcgatgtcaaatctagtatcgagaagctgaacgagctgtatgaaaatctgggcctggacctgaacgtggagttcaacattagcaatactgccgagatcgaaaaggtgctgaaagacaagcagatcttcaagcgggataaagtcaagaaaattgccgagctgtttgctatcaaaaccgacaacaaggaacagagcaagagaatcaaagatatttccaaacaggtggccaatgctgtcctggggtacaagaccaggttcgacacaatcgctctgaaagagatttccaaggacgaactgtctgattggaacttcaaactgtcagacatcgatgcagacagcaagtttgaggccctgatgggaaacctggatgagaatgaacaggccatcctgctgactattaaggagctgtttaacgaagtgaccctgaatggaattgtcgaggacggcaacaccctgagcgaatccatgatcaacaagtacaatgatcaccgggacgatctgaagctgctgaaagaagtgatcgaaaatcatattgacagaaagaaagccaaggagctggcactggcctacgatctgtatgtcaacaataggcacggacagctgctgcaggctaagaaaaagctgggcaaaatcaagccccgctctaaggaggacttctacaaagtggtcaacaagaatctggacgattcacgggcaagcaaggagatcaaaaagaaaattgaactggacagctttatgcctaagcagagaaccaacgccaatggcgtgatcccataccagctgcagcagctggagctggataagatcatcgaaaaccagtctaagtactatccattcctgaaggagattaatcccgtgtcaagccacctgaaagaggccccctataagctggacgaactgatccgatttcgggtgccttactatgtcggccccctgatttctcctaacgagagtaccaaggatatccagacaaagaaaaaccagaatttcgcctggatgattcgcaaagaggaagggcgaatcacaccttggaactttgaccagaaggtggatcgaattgagagcgccaataagttcatcaaacggatgactaccaaggacacttacctgtttggggaggatgtgctgccagctaacagcctgctgtatcagaagttcaccgtcctgaacgaactgaacaacatccggattaatggaaaaagaatctccgtggacctgaagcaggagatctacgaaaacctgtttaagaaacacacaactgtgaccgtcaagaaactggagaattatctgaaggaaaaccataatctggtgaaagtcgagatcaaggggctggccgatgaaaagaaattcaacagcggactgaccacatacaatagattcaagaacctgaacatctttgacaaccagattgacgatctgaagtacaggaacgatttcgagaagatcatcgaatggtctacaatttttgaggacaagagtatctacaaagaaaagctgaggagcatcgattggctgaacgagaagcagattaacgctctgtctaatatcagactgcaggggtggggaaggctgagtaagaaactgctggcacagctgcacgaccataatggccagaccatcattgagcagctgtgggattcccagaacaatttcatgcagattgtgacacaggccgactttaaagatgctatcgcaaaggccaaccagaatctgctggtggctacctcagtcgaggacattctgaacaatgcatacacaagccccgcaaacaagaaagccatcagacaggtcatcaaggtggtcgacgatatcgtgaaggcagcctccggaaaggtcccaaaacagatcgccattgagttcactagggatgctgacgaaaatcccaagagaagtcagaccaggggctcaaagctgcagaaagtgtacaaggacctgagcactgagctggcctccaagaccattgctgaggaactgaacgaagcaatcaaagacaagaaactggtgcaggataagtactatctgtactttatgcagctggggcgggacgcctatacaggagagcctatcaatatcgatgaaatccagaagtacgatatcgaccacattctgccacagtctttcatcaaggacgatgccctggacaacagggtgctggtgagccgggctgtgaacaatggcaaatctgataatgtgcctgtcaagctgtttggcaacgagatggctgcaaatctggggatgactatcaggaaaatgtgggaggaatggaagaacatcggcctgattagcaaaacaaagtacaacaatctgctgactgatcccgaccacattaacaagtataagagtgccgggttcatcaggcgccagctggtggagacatcacagatcatcaagctggtgagcactatcctgcagagtcgctaccctaacactgaaatcattaccgtgaaggctaagtacaatcattatctgcgggagaaatttgacctgtataagagcagagaagtcaacgactaccaccatgctattgatgcatatctgtccgccatctgcggaaatctgctgtaccagaactatccaaatctgcggcccttctttgtgtacggccagtataagaaattctcctctgatcctgacaaagagaaggccatttttaacaaaacccgcaagttctcctttatctctcagctgctgaaaaacaagagtgagaacagcaaggaaatcgctaagaaactgaaacgggcataccagttcaagtatatgctggtgtctcgagagactgaaacccgggaccaggagatgttcaaaatgaccgtgtacccccggttcagccacgatacagtcaaggctcctaggaacctgattccaaagaaaatgggcatgtcccctgacatctacggaggctatacaaacaattctgacgcatacatggtcatcgtccgcattgataagaaaaagggaactgagtataagatcctgggcattccaacccgggaactggtgaatctgaaaaaggccgagaaggaggaccattacaaaagctatctgaaggagatcctgacaccaaggattctgtacaacaaaaatgggaagcgcgataaaaagatcacttccttcgaaattgtgaaatctaagatcccctataagcaggtcatccaggatggggacaaaaagtttatgctgggaagttcaacatacgtgtataacgcaaagcagctgacactgagcactgagtccatgaaagccatcactaacaatttcgataaggacagcgatgagaacgacgctctgattaaggcatacgatgaaatcctggacaaagtggataagtatctgccactgttcgacatcaacaagttccgggagaagctgcacagtgggcgagaaaagttcatcaagctgagcctggaggacaaaaaggataccatcctgaaagtgctggaaggactgcatgataacgctgtcatgacaaagatccctactattggcctgtccacaccactggggttcatgcagtttcccaacggcgtgattctgagcgagaatgccaaactgatctaccagtcccccaccgggctgttcaaaaagtcagtgaagatcagcgacctgtaagaattc

SEQ ID NO: 124 - DNA, 3405 bp, Artificial Sequence
  source: /note="Description of Artificial Sequence: Synthetic polynucleotide"
accggtgccaccatgtacccatacgatgttccagattacgcttcgccgaagaaaaagcgcaaggtcgaagcgtccatgggctacactgtgggactggatattggggtggcttccgtcggggtggctgtgctggatgagaatgacaacatcgtggaggctgtgtcaaacatctttgatgaagccgacacaagcaacaataaggtgcggagaactctgagggagggcaggcgcacaaagcggcggcagaaaacccgcattgaggacttcaagcagctgtgggagacttcaggctacatcattcctcacaagctgcatctgaatatcattgagctgcgcaacaaagggctgaccgaactgctgagcctggatgagctgtattgcgtgctgctgtccatgctgaagcaccgggggatctcctacctggaggacgccgacgatggcgagaaggggaatgcctataagaaaggactggcttttaacgaaaaacagctgaaggagaaaatgccatgtgagatccagctggaacgcatgaagaaatacgggaagtaccatggagagttcatcatcgaaattaatgatgagaaggaataccagagcaacgtgttcaccacaaaggcttataagaaggagctggaaaagatcttcgagacacagcggtgcaacggcaacaagatcaacacaaagttcattaagaaatacatggagatctacgaacgaaagcgggaatactatatcggaccaggcaatgagaaaagcagaacagactacggcatctatactaccaggactgatgaggaagggaatttcatcgacgagaagaacatttttggcaaactgatcgggaagtgtagtgtgtaccccgaggaatatagagcaagctccgcctcatacaccgcccaggagttcaatctgctgaacgatctgaacaatctgaaaatcaacaatgagaagctgacagaatttcagaagaaagagattgtcgaaatcattaaggacgcttctagtgtgaacatgaggaaaatcattaagaaagtcatcgatgaggacattgaacagtacagcggagcacgaatcgataagaaaggcaaggaaatctaccacaccttcgagatctatcggaagctgaagaaagagctgaaaacaatcaatgtggatatcgactcttttactagagaggaactggataagaccatggacatcctgaccctgaacacagagagggaaagtattgtgaaggccttcgacgaacagaaatttgtctacgaggaaaatctgatcaagaaactgattgagtttcggaagaacaatcagagactgttcagcggctggcatagtttttcatacaaggctatgctgcagctgatcccagtgatgtacaaggagcccaaagaacagatgcagctgctgaccgaaatgaacgtgttcaaaagtaagaaagagaagtacgtcaactacaagtacatcccagagaacgaagtggtcaaggagatctataaccccgtggtcgtgaagagcattagaacaactgtgaaaattctgaatgcactgatcaagaaatacgggtatcctgaatccgtcgtgatcgagatgccaagggataagaactctgacgatgagaaggaaaagatcgacatgaaccagaagaaaaaccaggaggaatacgagaaaatcctgaacaagatctacgatgagaagggaatcgaaattaccaacaaggactacaagaaacagaagaaactggtgctgaagctgaaactgtggaacgagcaggaaggactgtgcctgtattccggcaagaaaatcgctattgaggatctgctgaatcaccccgagttctttgaaattgaccatatcattcctaagagcatctccctggacgattctcgcagtaacaaggtcctggtgtacaaaacagaaaattctatcaaggagaacgataccccctaccactatctgacacggattaacggaaagtggggctttgacgaatataaagctaatgtgctggagctgagaaggcgcggcaagatcgacgataagaaagtgaacaatctgctgtgcatggaggatatcactaagattgacgtcgtgaaagggttcattaaccgcaatctgaacgacaccagatacgcatccagggtggtgctgaacgaaatgcagtccttctttgagtctcgaaagtactgtaatactaaggtcaaagtgatccgaggctctctgacctatcagatgcggcaggatctgcacctgaagaaaaacagagaggaatcatacagccaccatgctgtggacgcaatgctgatcgcattctcccagaaggggtacgaggcctataggaagatccagaaagattgctacgactttgagacaggcgaaattctggacaaggaaaaatggaataagtacattgacgatgacgagtttgatgacatcctgtataaagagaggatgaacgaaatccgcaagaaaatcattgaggccgaggaaaaggtgaagtacaactacaagatcgataagaagtgcaatcgcgggctgtgtaaccagactatctacgggacccgagaaaaggacggaaaaatccacaagatttcaagctacaacatctatgatgacaaggagtgtaattccctgaagaaaatgattaacagtgggaaaggatcagatctgctgatgtacaacaatgatcctaagacatatcgcgacatgctgaaaatcctggaaacttactcctctgagaagaatccattcgtggcatataacaaagagacaggagactactttcggaaatattctaagaatcacaacggacccaaggtcgagaaggtgaaatactatagcggccagatcaactcctgcatcgatatttctcacaagtacggccatgccaaaaatagtaagaaagtcgtgctggtgtcactgaacccttatagaaccgacgtctactatgataatgacacaggcaagtactatctggtcggggtgaagtacaatcatatcaaatgtgtcggaaacaagtacgtgattgatagcgagacatataacgaactgctgaggaaggagggcgtgctgaacagcgatgagaacctggaggacctgaacagcaaaaacatcacttacaagttcagtctgtacaagaacgacatcatccagtacgagaagggcggggaatactatacagagcgctttctgagccgaatcaaagaacagaagaacctgattgagactaaacccatcaataagcctaacttccagcggaagaataagaaaggcgagtgggaaaataccagaaaccagatcgccctggctaagactaaatacgtggggaagctggtcaccgatgtgctgggaaactgttacatcgtgaacatggagaagttctccctggtcgtggacaaataagaattc

SEQ ID NO: 125 - DNA, 3474 bp, Artificial Sequence
  source: /note="Description of Artificial Sequence: Synthetic polynucleotide"
accggtgccaccatgtacccatacgatgttccagattacgcttcgccgaagaaaaagcgcaaggtcgaagcgtccatgactaacggcaagattctggggctggacattggcatcgcaagcgtgggggtggggattattgaggcaaaaactggaaaggtggtgcatgccaattcccggctgttctctgccgctaacgctgagaacaatgcagaacggagagggtttaggggatctaggcgcctgaatcgacggaagaaacaccgcgtgaagcgagtccgggatctgttcgagaaatacggaatcgtcaccgactttcgcaacctgaatctgaacccttatgagctgcgagtgaagggcctgaccgaacagctgaaaaacgaggaactgttcgcagccctgagaacaatctctaagagaagggggattagttacctggacgatgccgaggacgatagtaccggatcaacagactatgctaagagcatcgatgagaatcgccgactgctgaaaaacaagacaccaggccagattcagctggagaggctggaaaagtacggccagctgcgcgggaatttcaccgtctatgacgagaacggggaagcccatcgcctgatcaatgtgtttagtacatcagattacgagaaagaagcacggaagatcctggagacacaggccgactacaacaagaaaatcacagctgagttcattgacgattatgtggaaatcctgacccagaaacgaaagtactatcacggccccgggaacgaaaagagccggactgactacggacggttccggaccgatgggaccacactggagaatattttcggaatcctgattggcaagtgcaacttttaccctgatgaatatcgagcaagcaaggccagctacaccgcacaggagtataatttcctgaacgacctgaacaatctgaaggtgagcaccgaaacagggaagctgtcaacagagcagaaagaaagcctggtggagtttgccaagaatactgctaccctgggacccgctaaactgctgaaggagatcgcaaaaattctggactgtaaggtggatgagatcaaaggatacagagaggacgataaaggcaagccagatctgcataccttcgagccctataggaaactgaagtttaatctggaaagcatcaacattgacgatctgtcccgcgaagtgatcgacaagctggctgatattctgactctgaacaccgagagagaaggaatcgaggacgcaattaagaggaatctgccaaaccagttcacagaggaacagatcagcgagatcatcaaggtgcggaagagccagtccactgctttcaataagggctggcactcttttagtgcaaaactgatgaacgagctgatccccgaactgtacgccacctccgacgagcagatgacaattctgactcggctggaaaaattcaaggtcaataagaaaagctccaaaaacacaaagactatcgacgagaaggaagtcactgatgagatctacaatcctgtggtcgccaagagcgtgagacagaccatcaaaatcattaacgctgcagtcaagaaatatggcgacttcgataagatcgtgattgaaatgccacgggataaaaatgctgacgatgagaagaagttcatcgacaagagaaataaggagaacaagaaggaaaaggacgatgccctgaaaagggccgcttacctgtataattctagtgacaagctgcccgatgaggtgttccacggcaacaagcagctggaaaccaaaatccgactgtggtatcagcagggggagcggtgcctgtatagtggaaagcccatctcaattcaggagctggtgcataactctaacaatttcgaaatcgatcacattctgcctctgtcactgagctttgacgatagtctggccaataaggtgctggtctacgcttggacaaaccaggagaaaggccagaaaaccccttatcaggtcatcgactccatggatgcagcctggtctttcagggagatgaaggactacgtgctgaaacagaagggactgggcaagaaaaagcgcgactatctgctgactaccgagaacatcgataagattgaagtgaagaagaagttcatcgagaggaatctggtggatactcgctacgcatctcgagtggtcctgaactctctgcagagtgccctgagagagctggggaaagacactaaggtgtctgtggtcaggggacagttcaccagtcagctgcggagaaaatggaagatcgataagagccgcgagacataccaccatcacgcagtggacgccctgatcattgctgcatcaagccagctgaaactgtgggagaagcaggacaatcccatgtttgtggattatggcaagaaccaggtggtcgacaaacagactggggagatcctgtccgtgtctgacgatgagtacaaggaactggtgttccagcccccttatcagggctttgtgaataccatctcctctaaagggttcgaggacgaaattctgtttagctaccaggtggattccaaatataaccggaaggtcagtgacgcaaccatctactcaacaagaaaagccaagattggcaaggataagaaagaggaaacctacgtgctgggaaaaatcaaggacatctactcccagaatggcttcgataccttcatcaagaagtacaacaaagataagactcagttcctgatgtatcagaaggactctctgacatgggagaacgtgatcgaagtcattctgagggactacccaacaactaagaaaagcgaggacggcaaaaatgatgtgaagtgcaacccctttgaggaatacaggcgcgagaatgggctgatctgtaagtattccaagaaagggaaaggaactcccatcaagagcctgaagtactatgacaagaaactggggaactgcatcgatattaccccagaggaatcacgcaataaggtcatcctgcagagcattaacccttggcgagccgacgtgtacttcaatccagagacactgaagtacgaactgatgggcctgaaatattcagatctgagctttgaaaagggcactgggaactaccatatcagccaggagaaatatgacgctatcaaagagaaggaaggaattggcaagaaatccgagttcaagtttacactgtaccgcaacgacctgatcctgatcaaggatatcgccagtggcgagcaggaaatctacagattcctgtcaagaactatgcccaatgtgaaccactacgtcgagctgaagccttacgacaaggaaaagttcgataacgtgcaggagctggtcgaagcactgggagaggcagataaagtgggacgatgtatcaaaggactgaataagccaaacatcagcatctacaaggtgagaaccgacgtcctgggaaacaaatatttcgtgaagaaaaagggcgacaaacccaagctggattttaagaacaacaagaagtaagaattc

SEQ ID NO: 126 - DNA, 3462 bp, Artificial Sequence
  source: /note="Description of Artificial Sequence: Synthetic polynucleotide"
accggtgccaccatgtacccatacgatgttccagattacgcttcgccgaagaaaaagcgcaaggtcgaagcgtccatggccgaccgaatctctctggggctggacattggggtggcaagcgtggggttctcagtgctggacattgataagggaaaagtcattgagctgggcgccaggctgttctctgctactgtggccgctggcaaccaggatcgaagagacatgcgaggagccaggcgcctgctgaaccggaacaagcagcgacggcaggataccggaaagctgttcaagaaatttggcctgatcgacgattttgataagggcagcttctacgacaactttaatcagaacctgaatccttatgagctgagagtgaaaggcctgacagaacagctgactaaggaggaactggccgagtctctgtaccagatcgtgaaacatagggggattagttatgcactgaaggacgccgatgtggacgaaggcgggacagactactcagtcagcctgaaaatcaacagccaggagctggcagaaaagactccagcccagattcagctgcagagactgaatgattatggaaaggtgaggggccaggtggtcatcggcgacgatccagacaaccagaaggtgctgctgaatgtgttccccacatcagcttacgagaaagaagcaaagcagatcattgccactcagcagcagttctatcctgagagcctgaccgacaagttcaccgaggaatactgccagatcctgactcgcaagcgagattattttgtggggccaggaaacgagaaaagccggaccgactacgggatctacaagactgatggaagaaccctggacaatctgttcgaggaactgatcggccacgataagatctaccccgaggaactgcgggcatctgcagccagttataccgcccagctgtttaacgtgctgaatgacctgaacaatctgagaatcctgaactacgaggatgggaaactgacaaaggaggacaaggaaaagatcatcgctgaaattaagaacaacaccacaactatcaacatgctgaatgtgattaagaaagtcgccgggtgttccaaggacgatatcaaaggattccgagtgaatgagaaggataaacccgaaatcagctccatgcctgtgtaccgcaaaattcataaggacctgctgaaggccggcgtggatatctcagactggcccgtcgagttcatcgacgaactgagctttattctgacactgaacactgagaatggggaaattcgcaaacagctgaacaatcgactggcccctaagttcgattttctgaacgctgacctgatccagctgatcattgataataaggactcctttgagattaagactaacaacaagtggcacagattcagcgtgaaaaccatgaacaaactgatcccagagatgatggaaagacccgtggagcagatgaccctgctgaatgaaatgggactggtcaagaaagataagaaacgctttgagaacaataagtacctgccttacaaggaaatcgcaaaggacattttcaacccagtggcctccaaatctgtccgcgaggccctgaagatcgtgaatgctgtcctgaagaaatacggccacattgattatctggtggtcgaaatgcctcgggataaaaacctgaaggaggaacaggacaatatcaaggagttccagaacaaaaataagaaagctaaggacgctgcattcgaagcatttgtgaaatcagtcgggagcgagcagagagtgaaggaagccctgtctaaaaaccggaagctgcagatgaagatgagactgtggtatcagcagcaggagatcgatccatataatggaaagacaatcgatgccactgacctgattaacaatcctgataagttcgagattgaccatatcattccacagagtatctcattttacgacagtattaacaataagaccctgtgcttcgcctcaatgaaccaggtgaaaggacagaaaaccccctacgagtttatgctggaaggccacgggcagtcctatgacaagttcaaagctacagtgatggcaaacaagaattttggcaaggctaaaagggcaaactacctgttcgaggaaaatgtgagcgatatcgagactcggaagagattcctgtcccgcaacctggtggacacccgatattctagtcgggtggtgctgaacagcctgcaggatttctttcgggagaaatctgccgacaccaaggtgacagtcattcgcggcaagtttacctccaacatgcgaaaacattggcacatcgataagactagggagacattccaccatcacgccattgacgcttctatcattgccgctacaccatttctgcgcatgtggaagaaaggaggcactatcttccccgtgaaggtcggagaagaaagtatcgatattgagacaggcgaaattctggacgataagaattttgacaaagcaatgtacgaggaaccctatagtggcttcgtgtcagagatcatgaacgccgacgatcggatcaagttcagccaccaggtggataagaaaatgaataggaaggtgagcgacgccaccatctacagtactcgcaccgggaaactggctaaggataagaaagacgctgagtacatcgtggcaaaggtcaaagatatctacagcgtggacggattcaagaagttcaagaaagtctacgataaggacaaaaccaagtttctgctgtacaaatatgatcctaggacattctcaaagctggagcgcatcattagcgattgcccagacaaagtggaaaaggtccagacaaacggcaaagtgaaggctgtcgatatcagtccattcgagatgtacagaagggaccatgggatgatcaagaaatactcaaagaaaggaaacggccccgccatcaagcagctgaagtacctggataagaaactgggcagccacatcgacattacccccgcaaacgccaatggaaaacacgtgatcctgcagagtctgaagccttggagaaccgacgtctatctgaaccacgagacaggcgagtacgaaatcatggggattaagtatagcgatctgaagttcaacaagaatgaggggtacggaatcaagaaagacaagtatctggaaattaagaaagtggaggaagtctccgagaagtctgagttcatgtttagcctgtacaggaaggatcgcgtgaaagtccaggacatgaaaaccggcgagtccgtggaactgctgttctggagcaggaacttttccaataagaaatacgctgagctgaagcccatctcccaggcagaaaacgacaagaaactgcctgtgtatggcaaagggagactgatcaagaggctgattcccaaaaactgtaagatctggaaagtgaataccacaattctgggcgatccctactatctggagaaagaaagcgactcccctaaggatatcctggactaagaattc

SEQ ID NO: 127 - DNA, 4611 bp, Artificial Sequence
  source: /note="Description of Artificial Sequence: Synthetic polynucleotide"
accggtgccaccatgtacccatacgatgttccagattacgcttcgccgaagaaaaagcgcaaggtcgaagcgtccatgaagaaaacactgggactggacctggggactaacagcattgggtgggccgtcatcaactcaaacatcgactcagaaggaaaagaaaagctggtggggatcagctcctgcggaagccggatcattcctatggacgctaccacactgggagatttcggaaagggcaacactaaaagtccagtggcagagcgaacccgactgcggggcattcggagactgctggaaaggtcactgctgaggcgcgagcgactgcaccgagtgctgtcagtcatggggttcctgccagagcattacgctagccagctggaccgctatggaaagtttctgccagaaaccgagcccaagctggcatggtacaaagacgatagcggcaggtatcagttcctgtttcagaagtccttccacgagatgctggaggactttcgacagcatcagccagaactggtggcaggagagaagaaaatcccttacgattggacaatctactatctgcggaagaaagcactgtctcaggagatcactaaggaggaactggcctggattctgctgaatttcaaccagaaacgcggctactatcagctgcgaggggaggaagagcaggaagagaacaataagagcgtggagtatcacgccctgaaagtggtgagcgtcgaggactctggagaaagaaagggcaaagatatctggtacaatgtgactctggagaacggatgggtctatcgacgggctagcaacattcccctggactggaccggcaaggtgaaagagttcgtggtcactaccgagctggacgatgccgggaacccaaagaaagataaggaaggaaatgtgaaaagatcctttagggcaccaaaggaggacgattgggggctgctgaaaactaggacccaggctcagatcgacgaatccggcaagaccgtgggaacttacatctacgagtctctgctgtgtatgcccaaccagaagatccggggaaaactggtgaggaccattgaacgcaagtactataaagacgagctgagacagatcctggtgaagcagagcgagttccacgccgctctgcaggatcataatctgctgctgtcctgtatcgaagagctgtaccctaacaatgaggcccacagaaggctgctgagcgccagcagcttcatctacttcctgatcgaggacattctgttttatcagcgcccactgaagtcccagaaagggctgatcgataactgcccctacgagtctcacatctacaaggataagaaagatggaagtctgcaccatgtgcctctgaagtgtgtcagcaaatcccatccactgttccaggaatttcgcctgtggcagttcctgtctaacctgcgaatctaccagagagagaggatgatggacggcagtctgaaactggacgtggatgtcacccgggagttcctgccctcagaagaggactacgtgaagctgtttgattggctgaatgagagaaaggaaatctctcagaaattcctgctggcttataaaccttttgggctgaagaaaaacgaacaggcaaattacagatggaactatgtggaggacaagagctacccctgcaacgagacacgggcagaaatcaagagcagactgtccaaagccggagtgcctgaagagtttctgactgaagagaaggaagaggccctgtggcacatcctgtattctattagtgataagaaagagctgactaaggctctgggcaccttcgcagccaaaaactgtctgaatgagtctttcgtggaagtctttgccaagatccccccttttgagtcaaactacgctgcatatagcctgaaggctattaggaaactgctggcactgatgcgcatggggaagtactggaatgaacaggccatcgacaggcagactcgcgatcgaatcgagaaaattctgaccggagagtatgacgaaacaatccggagcagagtgagggagaaggcaatgctgctgaccgatattagcagcttccggggcctgcctctgtggctggcctgttacatcgtgtatgaccgccactcagagagcaaggaactggtcaaatgggagacaccagccgacatcgatcatttcctgtccaagtttaaacagaacagcctgcggaaccccatcgtggaacaggtcattacagagtccctgcgcactgtgcgagacatttggaagcaggagggaaaaatcgatgagattcacgtggaactgggccgggagatgaagaaccctgcaaaagagcgcgcccgaattacagctcaggtgcaggaaaatgagaacactaatctgagaatcaaggctctgctggcagagttcatgaaccccgaatttgagattgaaaatgtgcatccatactcacccggccagcaggaaatcctgcggatctacgaggacggcgtgctgagcgggatcgctgagaaggatctgcctgacgatatcacagcaattctgaagaaattccgagaaaacgacgtgaagaaacggccaacaactagcgaagtcctgcggtacaaactgtggctggagcagcggtacagatccccatataccggaagagtgatccccctgggcaagctgttcacacctgcttacgagatcgaacacgtgattccccagagccggtattttgacgattccatctctaacaaagtgatctgcgaaagtgccgtcaataagctgaaagataactgtctgggctatgagttcatcaagaaacattccggggagatggtggaactggggaatggagagacagtgcccgtgttcagcgtggaagagtacgaacggttcgtcaaggagtcttacttcggcaacagtaagaaaatgaagaaactgctgctggaggacatcccagatagcttcattgagagacagctgaatgacagtcgatacatctcacgggtggtcacatctctgctgagtaacctggtgtgcgaagagggagagcaggatggcctgtccaagaatgtgatcgtctgtaccggcgggattacagacaggctgaagaaagattggggagtgcaggaagtctggaaccgcatcattctgcctcggttcctgagactgaatgagatcaccggacggacagactttacaagtacttcagtgaacggccacctgctgcctgccctgccactgtacctgcagaagggctttaataagaaaagaattgaccataggcaccatgccatggatgctatcgtgattgcctgcgctaaccggaatatcgtcaactacctgaacaattcctctgctagaaagaacagcgaaattagccgatatgacctgcagcggctgctgtgtgagaaggtgaaaaccgatgccaacggcaattacaagtggatcctgaggaaaccatgggagacattcacccaggatgtgtatgccgctctgacaaacatcgtggtcagctttaagcagaatctgcgcgtgattaatcgaaccacaaactactatcagcactacaacgaggcaggggaaaagcgcatgatccctcagaccaaaggcgacagatgggccattagaaagccaatgcataaagatactgtgtatggcgaagtcaatctgagaaaggagaaaaccctgccactgagggacgtggtcaagaaccccagtatcgtggtcgataaatcactgaagaacaagctgtacgagctgctgaagagccagtatgacctgaaggcaatcgccaaatacttcgagacacaccaggacgtgtgggcagatgtcaacctgaagaaaattaaggtgtactacttcactaaggagacaaacgaaagattctttgccactaggaagagcctggacccatcctttgatcagaagaaaatcgaagaggaagtgactgataccggcgtccagaagattctgctgcaccatctgcagcagaacaataacgaccctgatatggccttttccccagacggcatcgataggatgaaccagaatatgaccattctgaatgacgggaagtggcaccagcccatctacaaagtgcgcacatatgaaaaggcagataaattcgccgtcggcgagtctgggaacaaggccaagaaatttgtggaagcagccaaaggcaccaatctgttctttgccgtgtacgagagtgtccaggaggacgaagctatcgggaagcaggtctgcaaacggacattcgccactatccccctgaacgaagtgatcaagagaaagaaacagggcctgcccgctgcacctgaggacctgaacgggaatctgcccaagtttgtgctgagccctaacgatctggtctacctgcccaccgaggaagagaggaatagttcacgcatcattcagcctctggacagggagcgcatctataagatggtgagctcctctgggagtcagtgcttctttatcaaagtgttcgtcgccaattcaatttgggataagaacgaatacagcagcctgaacaagatggagagggctattacaaacgaaatgatcaaggagatttgtgtgcctatcaaaattgaccgcctgggcaatgtcagcctgatccagatttaagaattc

SEQ ID NO: 128 - DNA, 4458 bp, Artificial Sequence
  source: /note="Description of Artificial Sequence: Synthetic polynucleotide"
accggtgccaccatgtacccatacgatgttccagattacgcttcgccgaagaaaaagcgcaaggtcgaagcgtccatgacaaagactattctgggactggatctggggactaacagcattggatgggcactgattaaccaggacttcgataacaaaaagggggagatcctgggcatgggcagccggatcattcctatgacacaggatattaaggacgagttcggaaaaggcaactctatcagtcagacagctgagcgaactcgactgcggggagtccggagactgatccacagaactctgctgaggcgcgagcggctgcatagagtgctgaatatcattggcttcctgccagaacactatgccaaccagattgactttgagaagaggttcggcaagttcaagcctgaatctgagccaaaaatcagtttcgatggaaatgacgtgttcctgtttgagaagagctaccaggaaatgctggtcgactttaaaatccaccagccacagctggtgagcaacggcaagaaaattccccatgactggacaatctactatctgagaaagaaagctctgtctaagaaaattgagaaggaggaactggcatggatcctgctgaacttcaatcagaaacggggatactatcagctgagaggcgaggaagaggaagagacaccaaataagctggtggagtttcatagcctgaaaattgtggaggtcaacgccgatgaaccccagaaaggaaagcctgagatctggtactcactggtgctggaaaacggctgggtctatcgacgggctagcaagactcccctgttcgattggaaagacaagattagggagtttatcgtgaccacagaaatcaacaatgatggaactgtcaaaaccgacaaggagggcaccgaaaagaggagcttccgcgcaccaaaacccgaggactggactctgcagaagaaaaagaccgagttcgagctgtcaaagagcgggaatgaagtgggagccttcatctacgaaagtatcctgcagaaacccaaccagaagattagaggcaaactgatttcaaccatcgagaggaaattttataaggaagagctgaaaaccatcctgaaaacacagctgttctttcacaaagaactgaaggatgagaaactgtacaatgcctgcatcgaagagctgtataagaacaatgaagctcaccggagcctgctgtccaacaaggggttcgagcatctgtttattaacgacatcctgttctaccagcgacctctgcggtctaaaaagagtcagatctcaaactgcccactggagaagcgcacatataaaaaggaggggattgaaatcactgagggcatcaaagtgatctccaaatctaatccaatctaccaggagttccggctgtggcagtggattagcaacctgtccctgtattgtatcgaacccaccgagacaaatgtgacttcaacctttctgaacagcattgaagattacgagaatctgttcgaatttctgaacaatcgcaaggaaatcgagcagaagcacctgctgaaatatctgctggagaaccaggggtttaaaggaaagctgctgacaaacgaactggagaagttccgctggaattttgtcgctgacaaaaagtacccctgtaatgagacaggcagcctgctgcatactcggctgagcaaagtgaagaacatttcccctgatttcctgaccaaggaaatcgagcaccagctgtggcatatcatctacagcgtgaccgacaagattgaatatgagcaggccctgaaaacctttgctcggaaaaacaatctggatgtggactccttctttgagcacttcaaaaagatccccccttttgagtctacctacggagcatatagtgaaaaggccatcaagaagctgctgccactgatcagactgggcaaatactggaactgggaggccattgatagtatctcaaaggacaggattagtaaaatcctgtcaggggaatacgatgagaacattaagaacagagtgagggagaaagcagtccacctgacctccgaaaacaatttccagggactgcaggagtggctggccaagtacatcgtctatgatcgccattctgagggcaatgacctggggaagtggactagcgtgtccgacctggagacatacctgaaggagttcaagcagcatagcctgcggaaccctattgtggagcaggtcatcacagaaactctgagagtggtcaaggatatttggatcaagcacgggaaaggaaccgaaaatttctttgacgaaatccatgtggagctgggccgggaaatgaagaacaattccgaggatcgcaaacgactgaccaacacaattactgaaaacgagaatacaaacctgagaatcaaggccctgctgatggaaatgatgaatgataacgacgtggagaacgtcaggccttactctccaagtcagcaggagattctgaagatctatgaggacggagctctgaatagcaacatcgagctggacgatgaaattgtgaagatctccaaaaaggcagagcccaccaaatctgaactgcagcgctacaagctgtggctggagcagaaataccgatccccttatactggccaggtcatcccactgaacaagctgttcacctctgaatatgagatcgaacacgtggtccctcagagtcgcttctttgacgatagcttcagcaacaaagtgatctgcgagtcagccgtcaacaagcggaaggataaccagctggggctgcagttcatcaagaaccatagcggagaaaaagtggagctgggcttcgggaaggtggtccaggtctttacagaagagcagtacctggattttgtgaaggagcactatagcaaaaatcgctccaagcataacaaactgctgctggaagagattcccgagaagatgatcgaaaggcagctgaatgacactcgctacatcagtaagttcgtgagctccattctgtccaacatcgtcagatctgagaaggacgatgacggcctgaatagcaaaaacattctgcctggaaatggcaagatcactaccgaactgaaaagggactgggggctgaatgatgtgtggaacgacctgattctgccaagattcgagaggatgaataccatcacaaacagcgatctgtttacaacttacaacgacaagtatcagaaacacctgcccaccgtgcctttcgagtactccaagggctttcagaaaaagcgcattgatcaccgacaccatgctatggacgcactggtcatcgcatgtgccacacgggatcatctgaatctgatgaacaatcagtctgccaagagtgaactgaaacgatacgacctgcagaacaagctgcggaaaaaggagccttacttcaaccagaaggagaacaaacagaaggaagccttcaaggattttatcaaaccatggggcactttcaccgaggacagcaagaatgctctggaaaaaatcattatctcctttaagcagaacctgagagtgatcaacaaggcaacaaactcatacgagagctataaggatgaggacgggaatctgaggatcggcaaggatgggaaaccagagaagggcctgatcaagcagaaggggctgaactgggcaatcagaaagcccctgcacaaagacaccgtgtcaggccagattaacctgagcaggatcaagctgcccaatgggaaaatcctgacagccactcgcaagaatctggataccagtttcgacctgaaaacaattgagaactcaatcaccgacacaggcattcagaaaatcctgaagaattacctgctgtccaaggaatctccagagctggccttctctcccgagggcctggaagagatgaacaatgagatcgaaaagtacaacaatgggaaatttcaccatcctattaacaaggctaggatctatgaactggggagcaaattcaatgtcggacagacaggcaacagaagggataagtttgtggaggccgctaaaggaactaatctgttctttgctatctaccaggacgagaataagaaccgctcttatgaaactattcccctgaacgaagtgatcgagcaccagaagtggcgagcaagtctgcctaaggaagagcaggagaaaattccactggtgcccgtcaacaagctgaaggggaccttcatcttttccctgtctcccaacgatctggtgtacgtcccttccaatgacgagctggaacgaagtgcttcaattgacttctctaagctgaaaaaggaacagatcaaccggctgtataaaatggtgtctagttcaggatcccagtgcttctttgtgaagagtgaggtcgcaacctcagtggtcaacaaaatggaatacagcagcctgaacaagatggagaagtctatcgataacctgatggtgaaggagatttgtatcaaactgaagattgacaggctgggcaacatcagcaaggcctaagaattc

SEQ ID NO: 129 - DNA, 4689 bp, Artificial Sequence
  source: /note="Description of Artificial Sequence: Synthetic polynucleotide"
accggtgccaccatgtacccatacgatgttccagattacgcttcgccgaagaaaaagcgcaaggtcgaagcgtccatgaccaaaatcctggggctggacctggggactaatagcatcgggtgggcaatccgcgacacagaaaatgagggcatcaatcagatcctggacaagggcgcccgcattttcagcgagggagtgaagtccgagaatggcaaagaaatcagtagggcagctgaacgaaccgcttaccggagcgcaagaaagatcaaatatcggagaaaactgcggaagtacgagacactgaaggtgctgtcaattaacggaatgtgccccctgagcgtggaggaagtcgaacagtggaagaaatctggcttcaaggaatatcccctgaatcctgagtttctggattggctgcggaccaacgaggacaagaacatcaatccttacctgttcagagataaagctagcaagcagaaagtgacactgtttgaactgggaagagctctgtatcacatcgcacagaggcgcggcttcctgagtaacaggctggaccagtcagccgagggcgtctttgaggaacataatcctcagatccagaacctgattgaggacctggacagctccaacacaattctgaatgagctgaaggaatactatatcaatctggggatcattgacgagactgaaaagtccggcttcaagaaagacctggatgagggggaaaagaaactgaagtcactgtacaacagcctggtggccatcacaaagaaaaacgctaacgatatcgaaacttgcaagcaggagctgatcgctagactgaataagaaagaggacctgggcaaggtcaaagggaagatcaaagatatttctcaggcaatgctggacaggaactttaagactctgggacagtatttcttttcactgtacaacaaggagcgaatccggaaccagtataccagccgcgaggaacactacctggaggagttcatcattatctgtcagacccaggggatcgagggaattaacacaaatgagaagctgcctgagaagaagttcaccggcctggcaaaagatctgtatcgagccattttctttcagcggccactgaaatcccagaagggcctgatcgggaagtgctctttcgagaagaacaagtctcgctgtgccgtgagtcacccagactatgaggaatttcgaatgtggagctacctgaacacaatcaaaattggcactcagtccgagaaaaccctgcgcttcctgacactggaggaaaagctgaaactggtgcccaagttctaccgaaagagtgatttcaacttcgaggtgctggctaaggagctggtcgaaaaaggagcatcattcggctactacaagtctagtaagaaaaatgagttcttttactggttcaactataagcccaccgattcagtgagcgcctgcgtggtgagcgcttctctggagaacgcaatcggcaaggactggaagatcaagactttcgaatatcagactagaaacaccgagaagaatgaagtgaccaaatccgtcgattacaaggacctgtggcacctgctgtccgtggcaacatctgatacttacctgtatgactttgccatcgaaaagctgaaactggagcctaaaaacgcaaaggccttcagcaagacaaaactgaagaaagactttgccagtctgtcactggcagccatcgctaaaattctgccatatctgaagcagggcctgctgtactcccacgccgtgttcatggctaacatcgagaatattgtcgacgccgatatctggaaggatgaggaacagcagaagttcatccagtccaagattgtggagctggtcgacaattatatcgtggaaaagtctaaactggagctgatcaatgggctgctgaagatctacaacaccgaggataaggaaggacggaaagtgtactattcaaaggaggctgaaagcctgttcgaggcagacctgagaaagaaactggtccccttctacaaggctaacatcatcatcgaggaacacgagcaggaaatcattttccaggatctgtttcctatcctgatggaccagctgaagaaacaggagttcatcaaaattggcagactggataagcagattgaagccttcctggagggggaaaatgaggaaggacagatcttttgtaaccacacagataagctgaagaaactgtaccatccaagcgacatcgaggtgtttaagaaaaagactatcaaagatgagtgggggaatgaaaaggtggtcctgggatccccactgaccacatctatcaagaaccccatggcaatgagagccctgcaccagctgaggaaggtgctgaatacactgattgccaacgaccagatcgacgaggatactcggatccatattgagatggccagagaactgaacgatgctaataagcgaaaaggcatccaggacttccagaacgagaacaagaagtttcgggaggaagccatcaaggagatcaagaagctgtacctggaggaatgccacaaagacgtgaaccccaccgaggacgatatcctgaggtatcagctgtggctggaacagggaaagtgcgagatctacgaggaaggcaacaatatcagcatttgtgatatcattggcagcaatccctcctatgacatcgagcataccattcctcggagcatctcccaggataacagccagatgaacaagacactgtgtagcctgaagttcaacagatccatcaaaaagcagaagatgccagtggagctgtccaactacaatgacattctgcccaggatcgcacactggaaaaaggaggccgaggaactgactaggcagatcgaaaccatttctcgcagcatcaagagcgctgcaaccaaggtggccaaggataagaacatcagaaagaggcattacctgacactgaagcgagactatattctggggaaatacgagcggttcacttgggaggaacctaaagtgggctttaaaaactcccagatcccagacactgggatcattaccaagtacgctcaggcatatctgaaatcttacttcaaaagggtggagagtgtcaagggaggagcagtggctgagttccggaaactgtggggcatccaggaatcttttatcgatgagaactggtggaagcactataaggacaaagatagagacaaacatacccaccatacaatcgacgcaatcactattgcctgtatgcccaaggataaatacgacctgctggcacacgcctggaggctggaggatgaacaggacaaaaaggccgctaaggtgctgatcgagcaggccaaaccatggaaaaccttcaaggaggatatcgaaaagattgagactgaaatcctggtgagccattttacccccgacaacgtcaaaaagcagtcaaagagcatcatcaagaatcgcggcaaaaaggtgtacgtcctgaagaacgagctgcctgtgaacttcaagaacaagatcgaagggaaggattatttcaagctgaaatttgacagcaagattctgtacaaaatccccaaaaagaaagagaagcagaccgatacattctatgaggaactgcctaaaaactacctgaatggagtggaaggcaaggactacttcaaaatcaatactaccggcaagaccttctacaaaatcccaatttttaaccagggcgacacaatccgggggagcctgcaccaggagacaacttacggagccattaagctgccagatatcgacattgaaacaaagaaacccctgcatactgataagggaggcttcattctgaagaaagacatcaaaggcaatgagattgtgttctttgtggtccgcaaggaaatctctaaaattagtgagaacgatgtgcagaatatcgtcgacaacgtggtccggaagaaaattgagaatgctatcgcaaactccctgatcacttttaagatcgtgaagaaaaagaaagtggccgtcatcaaagagggggtcaccatttggatgagggagcccaacattgaaaaggggatcgagggaatccctattaagaaagtgcgcatcattaccaattctgtcaaaaaccctatcgagattaaggtgcacagtccactgtccaagtctcgccacaagcataaacagaaggtctacggccagaacgatgagaattatgccatggctctgtacgaactggacgggaagcgggagttcgaactgatcaacaattttaatctggccaagctgctgaaacagagtcagtcatactatccactgcataaagagaaggaaatcaagggaaagaaaattctggtgcccatcgagaagagaaacaacaaggatgtcatcctgaagaggggccagcaggtggtgttctacgacaaaaccgtggagaaccccaaggatatctctgaaatcattgactttcgcgagcgaatctacatcattgaagggctgaccatccagagacagaaagataagaaaacatccaaagtgaatgagtacggaatcattcagctgcgccacttcaaggaagctcgaaaaagtgaggaaatctcaaaggataacttcaaacctgacggcgagttcaagatcaacgagaataagccaactaggaaaatgaaccataatcagttcaccgcctttgtggaggggatcgacttcaaggtcctgcctagcggaaagtttcagaaaatttaagaattc

SEQ ID NO: 130 - DNA, 3621 bp, Artificial Sequence
  source: /note="Description of Artificial Sequence: Synthetic polynucleotide"
accggtgccaccatgtacccatacgatgttccagattacgcttcgccgaagaaaaagcgcaaggtcgaagcgtccatgagcaagaaagtcagtagacgctatgaagaacaggcacaggagatttgtcagaggctggggagtagaccttattccatcgggctggacctgggagtgggatctatcggagtggcagtcgccgcttacgacccaattaagaaacagccctccgatctggtgttcgtcagctccaggatttttatcccttctaccggcgcagccgagcggagacagaagagaggacagaggaacagcctgcgccaccgagcaaatcgcctgaaattcctgtggaagctgctggctgaacgaaacctgatgctgtcatatagcgagcaggacgtgccagatcctgcacggctgagatttgaggacgctgtggtccgagcaaacccatacgagctgcggctgaagggcctgaatgaacagctgaccctgagcgagctggggtatgcactgtaccacatcgccaatcataggggatctagttcagtgcgcacattcctggatgaggaaaagagctccgacgataagaaactggaggaacagcaggctatgacagaacagctggcaaaagagaagggaatttccactttcatcgaagtgctgacagcctttaacactaatggcctgatcgggtacaggaactccgagtctgtgaagagtaagggcgtgccagtccccactcgcgacatcatttcaaatgagattgatgtgctgctgcagacccagaagcagttctatcaggaaatcctgtcagacgagtactgcgatcggattgtcagcgcaatcctgtttgaaaacgagaagatcgtgccagaagccggctgctgtccctatttccctgacgagaagaaactgcccagatgtcactttctgaatgaggaaaggcgcctgtgggaagccattaacaatgctaggatcaagatgcccatgcaggagggcgctgcaaaacgctaccagagtgcttcattcagcgacgagcagagacacattctgtttcatatcgcaaggagcgggactgatatcacccctaaactggtgcagaaggagttcccagccctgaaaacctccatcattgtgctgcagggaaaagagaaggctattcagaagatcgcaggcttccgatttcgacggctggaggaaaaatctttttggaagagactgagtgaggaacagaaggacgatttctttagcgcctggacaaacactcctgacgataaaagactgtccaagtacctgatgaaacacctgctgctgacagaaaatgaggtggtcgacgccctgaaaaccgtgagcctgattggagattatggcccaatcggcaagaccgcaacacagctgctgatgaaacatctggaggatggcctgacttacaccgaagccctggagcggggaatggaaaccggcgagttccaggaactgtcagtgtgggagcagcagagcctgctgccctactatgggcagatcctgacaggatctactcaggccctgatggggaagtattggcactctgcttttaaagaaaagagagacagtgagggattctttaagcctaacacaaatagcgatgaggaaaaatacggcaggattgccaacccagtggtccatcagactctgaacgaactgcgcaagctgatgaatgagctgattaccatcctgggagctaaacctcaggagatcacagtggaactggcacgagagctgaaggtcggagctgagaaaagagaggacatcattaagcagcagaccaaacaggaaaaggaggctgtgctggcatatagcaagtactgcgagcccaacaatctggacaaaaggtatattgaaaggttccgcctgctggaggatcaggcctttgtgtgcccttactgtctggagcacattagcgtcgcagatatcgcagctggaagggcagacgtggatcatatcttcccacgcgacgatacagctgacaactcctacgggaataaggtggtcgcacaccgacagtgtaacgatatcaagggaaagcggaccccctatgcagccttcagtaatacatcagcctggggccccatcatgcattacctggacgaaacccctgggatgtggcgcaaaagaaggaagtttgagacaaacgaggaagagtatgctaagtacctgcagtcaaaaggcttcgtgagcaggtttgaaagcgataactcctatatcgcaaaagctgcaaaggagtacctgcgctgcctgttcaatccaaacaatgtgactgccgtcgggtccctgaagggaatggagacatctatcctgcggaaggcctggaatctgcagggaattgacgatctgctgggcagccggcactggagtaaggacgccgataccagccccacaatgcgcaaaaaccgggacgacaatcggcaccatggcctggacgccatcgtggctctgtattgttccagatctctggtccagatgattaacaccatgtccgagcagggcaagcgagcagtggaaatcgaggctatgattcctatcccagggtacgcatccgaaccaaatctgtctttcgaagcccagcgggagctgtttagaaagaaaatcctggagttcatggacctgcacgcctttgtgagtatgaaaaccgacaacgatgcaaatggcgccctgctgaaagatactgtgtattcaattctgggagcagacacccagggagaggatctggtgttcgtggtcaagaaaaagattaaggacatcggcgtgaaaatcggggattatgaagaggtcgcatctgccattcgaggccggatcaccgacaaacagccaaagtggtatcccatggaaatgaaagataagatcgagcagctgcagtctaagaacgaagccgctctgcagaaatacaaggagagtctggtgcaggcagccgctgtcctggaagagagtaataggaagctgattgagtcaggcaaaaagcccatccagctgagtgaaaaaacaatttcaaaaaaggccctggagctggtgggcgggtactattacctgattagcaacaacaagcgcacaaagactttcgtggtcaaggaaccttcaaacgaggtgaaagggttcgcatttgacactggaagcaatctgtgcctggacttttatcacgatgcccagggaaagctgtgtggcgagatcattagaaaaatccaggctatgaacccttcctataagccagcatacatgaaacaggggtattctctgtacgtgagactgtaccagggcgacgtgtgcgagctgagggcaagcgatctgactgaagcagagtccaacctggccaagaccacacatgtccgcctgcccaatgctaaacctgggcgaaccttcgtgatcattatcacctttacagagatggggtctggatatcagatctacttcagcaacctggccaagtccaaaaagggacaggacactagttttaccctgactaccatcaagaattatgatgtgcggaaagtccagctgtctagtgccgggctggtgagatacgtcagccctctgctggtggacaaaatcgagaaggatgaagtcgctctgtgtggagagtaagaattc

SEQ ID NO: 131 - DNA, 3588 bp, Artificial Sequence
  source: /note="Description of Artificial Sequence: Synthetic polynucleotide"
accggtgccaccatgtacccatacgatgttccagattacgcttcgccgaagaaaaagcgcaaggtcgaagcgtccatggcaagacctgcatttcgggcacctcggagagaacacgtcaacggctggacccctgacccacatcggattagcaaaccctttttcatcctggtgagctggcacctgctgtcccgggtggtcattgacagctcctctggatgcttcccaggcaccagccgggaccacaccgacaagtttgccgagtgggaatgtgctgtgcagccctacaggctgagtttcgacctggggaccaactcaatcggatggggcctgctgaatctggatcgccagggaaaaccaagggagatccgagcactggggtcccgcatcttcagcgacggacgggatccccaggacaaggcttctctggctgtggcacggagactggccagacagatgaggcgccgacgggacagatatctgactagaaggaccaggctgatgggagctctggtgcgcttcggcctgatgccagcagaccctgcagctaggaagcgcctggaagtggccgtcgatccatacctggcacgagagcgggccacaagagaaaggctggagcccttcgaaatcgggagggccctgtttcacctgaaccagcgccgaggatataaacccgtgcgcaccgccacaaagcctgatgaggaagccggcaaggtgaaagaggctgtcgaaaggctggaggcagcaatcgctgcagccggagcacctactctgggagcttggttcgcatggcgaaaaacacgaggagaaactctgcgagcacgactggctgggaagggaaaagaggctgcatacccattctatcccgcacggagaatgctggaggccgaatttgacactctgtgggcagagcaggccaggcaccatccagatctgctgaccgccgaagctcgcgagatcctgcggcacagaatttttcatcagcggcccctgaagccacctccagtgggaagatgcactctgtaccctgacgatgggagagctcctagggcactgccaagcgctcagaggctgcgcctgttccaggagctggccagcctgagagtgatccacctggacctgtccgaacgccctctgaccccagctgagcgagatcggattgtggcatttgtccagggcagaccccctaaagccggaaggaagcctggcaaagtgcagaagagcgtcccattcgaaaagctgagggggctgctggagctgccaccaggcactgggttttctctggagagtgacaaacggcctgaactgctgggcgacgagacaggcgccagaatcgcaccagcattcggacctggatggacagctctgcctctggaggaacaggacgccctggtggaactgctgctgacagaggcagaaccagagagggcaattgcagctctgactgcacgatgggctctggacgaggcaactgcagcaaagctggctggagcaaccctgccagattttcacggacgatatggcaggcgcgcagtggctgaactgctgcctgtcctggaacgcgagacacgaggcgacccagatgggagagtgaggcccatccggctggacgaggcagtgaaactgctgagaggcgggaaggatcactcagacttcagccgggaaggagctctgctggacgcactgccctactatggagccgtgctggagagacatgtcgcttttgggacaggaaaccccgcagatcctgaggaaaagcgggtgggaagagtcgccaatcccactgtgcacatcgctctgaaccagctgcggcatctggtgaatgcaattctggccaggcacggccgccctgaggaaatcgtgattgagctggcacgggacctgaaaaggtctgccgaagatcgacggagagaggacaagcggcaggccgataaccagaaaagaaatgaggaacgcaagcgactgatcctgagtctgggagagcgcccaaccccacgaaacctgctgaagctgcggctgtgggaggaacagggcccagtggaaaataggcgctgcccctactctggggagacaattagtatgagaatgctgctgagcgagcaggtggacatcgatcacattctgccattcagcgtgtccctggacgattccgctgcaaacaaggtggtctgtctgcgggaggccaacagaatcaagcggaatagatctccctgggaggccttcggccatgacagtgagagatgggcagggattctggcacgagcagaagctctgcccaagaacaaaaggtggcgctttgctcctgacgcactggagaaactggaaggagagggaggcctgcgagcacgacacctgaatgatacaaggcatctgagtcgcctggccgtggagtatctgcggtgcgtctgtcctaaggtgcgggtgagcccaggccgactgactgcactgctgcgacggagatggggcatcgacgccattctggcagaagcagatggacctccaccagaagtgcccgcagagacactggacccttccccagctgagaagaaccgagcagaccaccggcaccatgccctggatgctgtggtcatcggctgtattgatcgctcaatggtgcagcgagtccagctggccgctgcaagcgcagaaagagaggccgctgcaagggaggacaatatcaggcgcgtgctggagggattcaaagaggaaccttgggatggctttagagctgaactggagcgacgggcacggaccatcgtggtgagccacagaccagaacatgggattgggggagccctgcataaggagacagcttacgggcctgtggaccctccagaggaaggattcaacctggtggtcaggaaaccaatcgacggcctgtcaaaggatgagattaatagcgtgcgggacccccggctgagaagggcactgatcgatcgcctggccattcgccgacgggatgctaacgaccctgctaccgcactggccaaagcagctgaggatctggcagcacagccagcctcccgcggcatcagaagggtgcgggtcctgaagaaagaatctaaccccattagggtggagcacggcgggaatccaagtggaccccgctcaggaggcccttttcataagctgctgctggcaggagaggtgcaccatgtggacgtcgcactgcgagcagatggccgccgatgggtgggacactgggtcacactgttcgaggcacatgggggacggggagcagacggagctgcagccccacctagactgggcgatggggaaagatttctgatgaggctgcacaagggagactgcctgaaactggagcataagggcagagtgagggtcatgcaggtggtcaaactggaacctagttcaaatagcgtggtcgtggtcgagccacaccaggtgaaaaccgacagatccaaacatgtcaagatctcttgtgatcagctgcgcgctcgaggagcacggagagtgaccgtcgatccactgggacgggtgagagtccacgccccaggagctagggtgggaatcggaggggacgccggacgaaccgctatggaacccgcagaggatattagctaagaattc

SEQ ID NO: 132 - DNA, 3234 bp, Artificial Sequence
  source: /note="Description of Artificial Sequence: Synthetic polynucleotide"
accggtgccaccatgtacccatacgatgttccagattacgcttcgccgaagaaaaagcgcaaggtcgaagcgtccatgggagagaatatgattgacgagagtctgaccttcggcattgacctggggattgggagttgtgggtgggcagtgctgaggcggccaagcgccttcggacggaagggcgtgatcgagggaatgggctcctggtgctttgacgtccccgagacatctaaagaacggactcctaccaaccagatccggagatccaatagactgctgaggcgcgtgatccgacggagaaggaaccggatggccgctattcgccgactgctgcacgcagcaggcctgctgccatcaaccgacagcgatgccctgaagcggcccggacatgatccttgggaactgagggcacgaggcctggacaagccactgaaacccgtggagttcgctgtggtcctgggccacatcgcaaagcggagagggtttaaatccgctgcaaagagaaaagccacaaacattagctccgacgataagaaaatgctgacagccctggaggctactcgagaacggctggggagatacaggaccgtgggagaaatgttcgccagggaccctgattttgcttctaggcgccgaaatcgcgagggcaagtatgataggaccacagctcgcgacgatctggagcacgaagtgcacgccctgttcgcagctcagcggagactgggacagggatttgccagtccagaactggaggaggccttcaccgcttcagcatttcatcagaggcccatgcaggacagcgagcgcctggtgggattctgcccttttgagcgaaccgaaaagcgggcagccaaactgacaccctctttcgagcgctttcgactgctggcccggctgctgaacctgagaatcactaccccagacggagagcggcccctgacagtggatgaaattgctctggtcacccgggacctgggcaagaccgcaaaactgagtatcaagcgggtgagaactctgattggactggaggacaatcagaggttcacaactatccgccccgaggacgaagatcgagacattgtggctcggacaggcggggcaatgacagggactgccaccctgaggaaggcactgggagaggccctgtggactgatatgcaggagcgccctgaacagctggacgctatcgtgcaggtcctgagcttctttgaggccaacgaaacaatcactgagaagctgagggaaattggcctgactctggccgtgctggacgtcctgctgaccgcactggatgccggagtgttcgccaagtttaaaggcgctgcacacatcagcaccaaagccgctaggaatctgctgccacatctggagcagggcaggcgctacgatgaggcctgcacaatggcagggtatgaccacgcagcctcccgcctgtctcaccatggccagatcgtggcaaagacacagttcaacgccctggtcactgagatcggcgaatccattgccaatccaatcgctcggaaggcactgatcgaggggctgaaacagatttgggccatgagaaaccactgggggctgcccggaagtatccatgtggagctggcccgggatgtcggcaactcaattgaaaagcgacgggagattgaaaagcacatcgagaaaaatactgccctgagggctcgcgagagaagggaggtgcatgatctgctggacctggaagatgtcaatggcgacaccctgctgcgataccggctgtggaaggagcagggaggcaaatgcctgtatacagggaaggccatccacattcggcagatcgctgcaactgacaactccgtgcaggtcgatcatattctgccttggagccggttcggcgacgatagttttaacaacaagaccctgtgtctggcctctgctaatcagcagaagaaaaggtcaacaccatacgagtggctgagcggccagactggggatgcatggaacgccttcgtgcagcgcatcgagacaaataaggaactgagagggtttaagaaaaggaactatctgctgaagaatgctaaagaggcagaggaaaaattcagaagcaggaacctgaatgacaccagatacgccgctaggctgttcgcagaggccgtgaagctgctgtatgcctttggggagagacaggaaaaagggggaaaccgccgagtgtttactcggcctggagcactgaccgcagcactgagacaggcttggggagtggagagcctgaagaaacaggatgggaagcgcatcaatgacgatcgacaccatgccctggatgctctgaccgtggctgcagtcgacgaggccgaaattcagaggctgacaaaatcattccacgagtgggaacagcagggcctggggcggcctctgcggagagtggagccaccttgggagagcttccgggcagacgtcgaggctacctaccctgaagtgtttgtcgcacggccagagaggcgccgagcaagaggagaaggccatgccgctaccatccggcaggtgaaggagagagaatgcacaccaattgtgtttgagagaaaggctgtctctagtctgaaagaggcagacctggaacgaatcaaagatggcgagcgcaacgaagcaattgtggaggccatcaggagctggattgccactggacgcccagctgatgcaccaccacgctccccccgaggcgacatcattaccaagatcaggctggccaccaccatcaaggcagccgtgcctgtccgcggagggaccgcaggaaggggagaaatggtgcgcgcagatgtgttcagcaagccaaaccggagagggaaagacgagtggtatctggtgcccgtgtatccacaccagatcatgaacaggaaggcttggcccaaacctccaatgcgctcaattgtggccaataaggatgaggacgaatggaccgaagtgggacctgaacaccagttccggtttagcctgtaccctagatccaatatcgagatcattaggccatctggagaagtgatcgaaggatatttcgtcggcctgcatcgcaacactggcgctctgaccatcagtgcacacaatgatcccaagagtatccattcaggcattgggaccaagacactgctggccatttccaaataccaggtggacagattcggcagaaagtctccagtgcgcaaagaggtccgaacttggcacggggaagcctgtatctctcccaccccccctggataagaattc

SEQ ID NO: 133 - DNA, 3504 bp, Artificial Sequence
  source: /note="Description of Artificial Sequence: Synthetic polynucleotide"
accggtgccaccatgtacccatacgatgttccagattacgcttcgccgaagaaaaagcgcaaggtcgaagcgtccatgagagagaacgggagtgacgaaaggcggaggaatatggacgaaaaaatggattacaggattgggctggacatcggcatcgcatcagtggggtgggccgtcctgcagaacaattcagacgatgagcctgtgaggattgtcgacctgggagtgcgcattttcgataccgcagagatcccaaagacaggcgaaagcctggcaggaccccggagagcagctcgaaccacaaggcgccgactgcggagaaggaaacaccgcctggaccgaatcaagtggctgttcgagaaccaggggctgatcaatattgacgattttctgaagagatacaacatggccggactgccagatgtgtaccagctgcggtatgaggctctggacagaaaactgaccgatgaggaactggcccaggtgctgctgcacatcgctaagcatcggggcttcagaagcaccaggaaagccgagacagcagccaaggaaaacggggcagtgctgaaggccacagacgagaatcagaaacgaatgcaggaaaagggatacaggacagtgggcgagatgatctacctggacgaggccttccggactggctgctcttggagtgagaaagggtacatcctgaccccccgcaacaaggctgaaaattatcagcacacaatgctgcgggcaatgctggtggaggaagtcaaggagattttcagctcccagcgccgactgggcaacgaaaaagccactgaggaactggaggaaaagtacctggagatcatgacctcccagcgctcttttgacctggggcctggaatgcagccagatgggaagccctccccttatgcaatggagggcttctctgacagagtggggaaatgtacttttctgggggatcagggagagctgaggggcgctaaggggacctacacagccgaatatttcgtggctctgcagaaaatcaaccacacaaagctggtcaatcaggacggcgagacaaggaatttcactgaggaagagcggagagccctgactctgctgctgtttacccagaaagaggtgaagtacgctgcagtccgcaagaaactgggcctgcctgaggacatcctgttctacaacctgaactacaagaaggccgctactaaagaagagcagcagaaggagaaccagaataccgaaaaagccaagtttatcgggatgccatactatcacgattacaagaaatgcctggaagagagagtgaagtatctgaccgagaacgaagtcagggacctgtttgatgagatcggaatgattctgacttgttacaaaaatgacgattcccgcaccgaacgactggccaagctgggactggtgcccatcgagatggaaggcctgctggcttatactcctaccaaattccagcatctgtctatgaaggcaatgcggaacatcattccctttctggagaaagggatgacctacgacaaggcttgcgaagaggcaggatatgacttcaaagccgatagcaaggggactaaacagaagctgctgaccggagagaacgtgaatcagacaatcaacgaaattactaatcctgtggtcaaacgctcagtgagccagacagtgaaggtcattaacgccatcattcggacttacggcagtccacaggctatcaatattgagctggcaagagaaatgtcaaagacctttgaagagaggcgcaaaatcaagggggacatggagaaacggcagaagaacaatgaagatgtgaagaaacagattcaggagctgggaaaactgtctcctacaggccaggacatcctgaagtacagactgtggcaggagcagcaggggatttgtatgtatagtggaaaaaccatcccactggaagagctgttcaagcccggctacgacatcgatcacattctgccctattcaattacattcgacgatagctttaggaacaaagtgctggtcacatcccaggagaacagacagaagggcaataggactccttacgagtatatggggaacgacgaacagcgctggaatgagtttgaaaccagggtgaaaactaccatccgcgattacaagaaacagcagaagctgctgaagaaacatttctctgaagaggaaaggagtgagtttaaagaacggaacctgacagacactaagtacatcacaaccgtgatctacaacatgatcagacagaatctggagatggcccccctgaaccgccctgaaaagaaaaagcaggtgcgggctgtcaatggcgcaattaccgcctacctgcgaaaacggtgggggctgccacagaagaatcgggagacagacacacaccatgctatggatgcagtggtcatcgcctgctgtaccgacggcatgatccagaaaattagtagatacacaaaggtgagagagaggtgctattcaaagggaacagagttcgtcgatgcagagactggcgaaatctttagacccgaggactacagcagggccgagtgggatgaaattttcggcgtgcacatcccaaagccctgggagacatttcgcgccgaactggacgtccgaatgggggacgatccaaagggattcctggacactcatagcgatgtggctctggagctggattatcccgagtacatctacgaaaacctgcggcctatcttcgtgagcagaatgccaaatcacaaggtcaccggagcagcccatgctgacacaattcggtccccaagacactttaaagatgagggcatcgtgctgactaagaccgcactgaccgacctgaaactggacaaggatggggagatcgacggatactataacccccagtccgatctgctgctgtacgaagcactgaaaaagcagctgctgctgtatggcaatgatgccaaaaaggccttcgctcaggactttcataaacccaaggccgatggaactgagggccctgtggtcaggaaggtgaagatccagaaaaagcagaccatgggagtgttcgtcgactctggcaacgggattgccgagaatggcgggatggtgcgcatcgatgtgttccgagtcaacggcaagtactattttgtgcccgtctacaccgctgacgtggtcaaaaaggtgctgcctaatagggccagtacagctcacaagccatacggcgagtggaaagtgatggaggacaaggatttcctgtttagtctgtattcacgcgacctgatccatatcaagtctaaaaaggatatccctattaagatggtgaacggaggcatggaggggatcaaggaaacctacgcatactatattggagccgacatcagcgctgcaaatatccagggcattgcccacgattccaggtataaattccgcggactgggcattcagtctctggacgtgctggagaagtgtcagatcgatgtgctgggacatgtcagcgtggtccgatccgaaaagcggatgggctttagctaagaattc

SEQ ID NO: 134 - DNA, 3243 bp, Artificial Sequence; identical to SEQ ID NO: 85
  source: /note="Description of Artificial Sequence: Synthetic polynucleotide"

SEQ ID NO: 135 - DNA, 3243 bp, Artificial Sequence; identical to SEQ ID NO: 85
  source: /note="Description of Artificial Sequence: Synthetic polynucleotide"

SEQ ID NO: 136 - DNA, 3891 bp, Artificial Sequence
  source: /note="Description of Artificial Sequence: Synthetic polynucleotide"
accggtgccaccatgtacccatacgatgttccagattacgcttcgccgaagaaaaagcgcaaggtcgaagcgtccatgaacaatagcatcaaatctaaacctgaagtgaccatcgggctggacctgggagtgggaagcgtggggtgggcaatcgtggataacgaaacaaacatcattcaccatctgggctccaggctgttttctcaggccaagactgctgaggatcggagatctttccgcggggtgaggcgcctgatccgacggagaaaatacaagctgaaacgattcgtcaatctgatttggaagtacaacagctatttcggcttcaagaacaaagaggacatcctgaacaattatcaggagcagcagaagctgcacaataccgtgctgaacctgaaatcagaggcactgaatgccaagatcgatcctaaagcactgagctggattctgcacgactacctgaagaacagaggccatttttatgaggacaatagggatttcaacgtgtacccaacaaaggagctggccaagtacttcgataagtacgggtactacaagggaatcattgacagcaaggaggacaatgataacaaactggaggaagagctgacaaagtacaaattctccaataagcactggctggaagaggtgaagaaagtcctgtctaaccagactggcctgccagaaaagtttaaagaagagtatgagtcactgttcagctacgtgagaaattattcagagggcccagggagcatcaactctgtcagtccctacgggatctaccatctggacgaaaaagagggaaaggtggtccagaagtacaacaacatctgggataagacaatcggaaagtgcaacatcttccctgacgagtatagagctcccaagaacagtcctatcgcaatgattttcaatgaaatcaacgagctgtccacaatcaggtcatacagcatctacctgactggctggttcattaatcaggagttcaagaaagcctacctgaacaagctgctggatctgctgatcaaaaccaacggagagaagccaattgacgcaaggcagttcaagaaactgcgcgaagagacaatcgccgaaagcattggcaaagagacactgaaggatgtggagaatgaagagaaactggaaaaggaggaccacaagtggaaactgaagggactgaagctgaataccaacggcaaaatccagtacaacgatctgagctccctggctaagtttgtgcacaaactgaagcagcatctgaaactggatttcctgctggaggaccagtatgcaacactggacaagatcaatttcctgcagtccctgtttgtgtacctgggcaagcacctgagatattccaatagggtcgattctgccaacctgaaggaattttccgactctaacaaactgttcgagcgcatcctgcagaaacagaaggatgggctgttcaagctgtttgaacagactgacaaagacgatgagaagatcctggcccagacacatagtctgtcaactaaggccatgctgctggctattacccggatgacaaatctggacaacgatgaggacaaccagaaaaacaatgacaagggctggaattttgaggccatcaaaaacttcgatcagaagtttatcgacatcaccaagaaaaacaacaacctgagcctgaaacagaataagcgctacctggacgatcgattcatcaacgatgctattctgtcccctggggtgaagcgaatcctgcgggaggcaaccaaggtctttaatgccattctgaaacagttctctgaagagtacgacgtgacaaaggtggtcatcgaactggctcgcgagctgagcgaagagaaggaactggagaacacaaagaactacaagaaactgatcaagaaaaacggcgacaagattagtgagggcctgaaagcactggggatctcagaagatgagatcaaagacattctgaagagtcccactaaatcatacaagtttctgctgtggctgcagcaggaccacatcgatccttatagcctgaaggagatcgccttcgacgatatttttaccaaaacagaaaagttcgagatcgaccatatcattccctacagcatttccttcgacgattctagttcaaacaagctgctggtgctggctgaaagtaatcaggcaaagtcaaaccagactccttatgagttcatcagctccggaaacgcaggcattaagtgggaagattacgaggcctattgccgcaagttcaaggatggggactctagtctgctggacagcacccagcggtccaagaaattcgccaaaatgatgaaaaccgatacctcaagcaagtacgacatcggatttctggctcgaaatctgaacgatactcggtacgcaaccattgtgttccgggacgccctggaggactatgctaataaccacctggtcgaggacaaacccatgtttaaggtggtctgtatcaatgggtccgtgacctctttcctgcggaagaactttgacgattcctcttacgccaagaaagatagagacaagaatatccaccatgctgtggatgcaagtatcatctcaattttcagcaacgagacaaagactctgttcaaccagctgactcagtttgctgactataaactgttcaagaacaccgatggcagctggaagaaaatcgaccctaagacaggggtggtcactgaagtgaccgacgagaattggaagcagattagggtgcgcaaccaggtgagcgaaatcgccaaagtcattgagaagtacatccaggatagcaacatcgaaagaaaggctaggtattcccgcaaaatcgagaataagactaacatttccctgtttaatgacaccgtgtactctgccaagaaagtcggctatgaggatcagatcaaaagaaagaacctgaaaaccctggacattcacgaatctgctaaagagaataagaacagtaaagtgaagcggcagtttgtctacagaaagctggtgaatgtcagcctgctgaataacgataagctggcagacctgttcgccgaaaaagaggatatcctgatgtatagggccaatccatgggtcatcaacctggctgagcagattttcaatgaatacactgagaacaagaaaatcaagtcccagaacgtgtttgaaaaatatatgctggacctgaccaaagagttccccgagaagttcagcgagtttctggtgaagtccatgctgagaaacaagaccgccatcatctacgacgataagaaaaacattgtccatcgaatcaaacggctgaagatgctgagttcagaactgaaagagaataagctgtctaacgtgatcattaggtctaagaatcagagtgggaccaaactgtcataccaggatacaatcaacagcctggccctgatgattatgcgcagcatcgaccctactgctaagaaacagtatattcgagtgccactgaataccctgaacctgcacctgggagatcatgactttgatctgcacaatatggatgcttacctgaagaaaccaaaattcgtgaagtatctgaaagcaaacgaaatcggcgacgagtacaagccctggagggtcctgacatctggcactctgctgatccataagaaggataagaaactgatgtacatcagctccttccagaatctgaacgacgtgatcgaaattaagaatctgatcgaaaccgagtataaagagaacgacgattctgatagtaagaaaaagaaaaaggcaaaccgctttctgatgaccctgagcacaatcctgaatgactacattctgctggacgccaaggataacttcgacatcctggggctgtctaaaaatcggatcgatgagattctgaacagtaagctgggactggacaagattgtgaaataagaattc

SEQ ID NO: 137 - DNA, 3093 bp, Artificial Sequence
  source: /note="Description of Artificial Sequence: Synthetic polynucleotide"
accggtgccaccatgtacccatacgatgttccagattacgcttcgccgaagaaaaagcgcaaggtcgaagcgtccatgaggattctggggtttgacattggcattaacagcatcgggtgggcttttgtggagaacgacgaactgaaggactgcggagtgcggatcttcacaaaggccgagaacccaaaaaataaggaaagcctggcactgccccggagaaatgcacgcagctccaggcgccgactgaaacggagaaaggcccggctgatcgctattaagagaatcctggccaaagagctgaagctgaactacaaggactatgtcgcagctgatggagagctgccaaaggcctacgaaggatccctggcatctgtgtacgagctgcggtataaggccctgacacagaacctggaaactaaagatctggccagagtgatcctgcacattgctaagcatagggggtacatgaacaagaacgagaagaaatcaaacgacgctaagaaaggaaagatcctgagcgctctgaaaaacaatgcactgaagctggagaactaccagagcgtgggcgaatacttctacaaggagttctttcagaaatacaagaaaaacacaaagaacttcatcaagatccgcaacactaaggataattacaacaattgcgtgctgtctagtgacctggaaaaagagctgaagctgatcctggaaaaacagaaggagttcggctacaactactctgaagatttcatcaacgagattctgaaggtcgccttctttcagcggcccctgaaggacttcagtcacctggtgggggcctgcactttctttgaggaagagaaaagggcctgtaagaacagctactctgcctgggagtttgtggctctgaccaagatcattaacgagatcaagagcctggagaagatcagcggcgaaattgtgccaacccagacaatcaacgaggtcctgaatctgatcctggacaaggggtctatcacctacaagaaattcagaagttgtatcaatctgcatgagagtatcagcttcaagagcctgaagtatgataaagaaaacgccgagaatgctaaactgatcgacttccgcaagctggtggagtttaagaaagccctgggagtccacagcctgtcccggcaggaactggatcagatctccactcatatcaccctgattaaggacaacgtgaagctgaaaaccgtcctggagaaatacaacctgagtaatgaacagatcaacaatctgctggaaattgagttcaacgattatatcaacctgagcttcaaggccctgggaatgattctgccactgatgcgcgagggcaaacgatacgacgaggcctgcgagatcgccaatctgaaacctaagaccgtggacgagaagaaagatttcctgccagcattttgtgattccattttcgcccacgagctgtctaaccccgtggtcaatagggctatcagcgaataccgcaaggtgctgaacgcactgctgaagaaatatggaaaggtccacaaaattcatctggagctggctcgcgacgtgggcctgtccaagaaagcacgagagaagatcgaaaaagagcagaaggaaaaccaggccgtgaatgcatgggccctgaaggaatgcgagaatattggcctgaaggccagcgcaaagaacatcctgaaactgaagctgtggaaagaacagaaggagatctgtatctactccggaaataagatctctattgagcacctgaaagatgaaaaggccctggaggtggaccatatctacccctattctaggagtttcgacgattcttttatcaacaaagtgctggtgttcaccaaggaaaatcaggagaaactgaacaagacacctttcgaggcctttggcaagaatattgaaaaatggagcaagatccagaccctggctcagaacctgccatacaagaaaaagaataagattctggacgagaacttcaaagataagcagcaggaggactttatctctcgaaatctgaacgacacccggtatatcgctacactgattgcaaaatacacaaaggagtatctgaacttcctgctgctgagcgaaaatgagaacgccaatctgaagagtggcgaaaaagggtcaaagatccacgtgcagactattagcgggatgctgacctccgtcctgaggcacacatgggggtttgacaaaaaggatcgcaacaatcatctgcaccatgcactggatgccatcattgtggcctacagtacaaattcaatcattaaggctttcagcgatttccggaaaaaccaggagctgctgaaggccagattctacgctaaagaactgacttccgataactataaacatcaggtcaagttctttgagcctttcaagagttttagagaaaaaatcctgtcaaagatcgacgagattttcgtgtccaaaccacctcgaaagcgagctaggcgcgcactgcacaaggatacctttcattctgagaacaagatcattgacaagtgcagctacaactccaaggaaggcctgcagattgccctgagctgtggaagagtgaggaaaatcggcactaagtatgtcgagaatgataccatcgtgagggtcgacattttcaaaaagcagaacaagttttacgctatcccaatctacgcaatggattttgccctggggatcctgcccaataagatcgtgattactggaaaagataagaacaataaccccaaacagtggcagaccattgacgaatcatacgagttctgctttagcctgtataagaatgacctgatcctgctgcagaaaaagaacatgcaggaacctgagttcgcctactataacgatttttcaatcagcacatcaagcatttgtgtggagaaacacgacaacaagttcgaaaatctgactagcaaccagaagctgctgttttccaatgcaaaagagggctctgtgaaggtcgaaagtctggggatccagaacctgaaagtgttcgagaagtacatcattacccccctgggagataaaattaaggctgactttcagcctcgagaaaacatcagcctgaaaaccagtaaaaagtatggcctgaggtaagaattc

SEQ ID NO: 138 - DNA, 4104 bp, Homo sapiens
  CDS (1)..(4104)
atggacaagaagtacagcatcggcctggacatcggcaccaactctgtgggctgggccgtgatcaccgacgagtacaaggtgcccagcaagaaattcaaggtgctgggcaacaccgaccggcacagcatcaagaagaacctgatcggagccctgctgttcgacagcggcgaaacagccgaggccacccggctgaagagaaccgccagaagaagatacaccagacggaagaaccggatctgctatctgcaagagatcttcagcaacgagatggccaaggtggacgacagcttcttccacagactggaagagtccttcctggtggaagaggataagaagcacgagcggcaccccatcttcggcaacatcgtggacgaggtggcctaccacgagaagtaccccaccatctaccacctgagaaagaaactggtggacagcaccgacaaggccgacctgcggctgatctatctggccctggcccacatgatcaagttccggggccacttcctgatcgagggcgacctgaaccccgacaacagcgacgtggacaagctgttcatccagctggtgcagacctacaaccagctgttcgaggaaaaccccatcaacgccagcggcgtggacgccaaggccatcctgtctgccagactgagcaagagcagacggctggaaaatctgatcgcccagctgcccggcgagaagaagaatggcctgttcggcaacctgattgccctgagcctgggcctgacccccaacttcaagagcaacttcgacctggccgaggatgccaaactgcagctgagcaaggacacctacgacgacgacctggacaacctgctggcccagatcggcgaccagtacgccgacctgtttctggccgccaagaacctgtccgacgccatcctgctgagcgacatcctgagagtgaacaccgagatcaccaaggcccccctgagcgcctctatgatcaagagatacgacgagcaccaccaggacctgaccctgctgaaagctctcgtgcggcagcagctgcctgagaagtacaaagagattttcttcgaccagagcaagaacggctacgccggctacattgacggcggagccagccaggaagagttctacaagttcatcaagcccatcctggaaaagatggacggcaccgaggaactgctcgtgaagctgaacagagaggacctgctgcggaagcagcggaccttcgacaacggcagcatcccccaccagatccacctgggagagctgcacgccattctgcggcggcaggaagatttttacccattcctgaaggacaaccgggaaaagatcgagaagatcctgaccttccgcatcccctactacgtgggccctctggccaggggaaacagcagattcgcctggatgaccagaaagagcgaggaaaccatcaccccctggaacttcgaggaagtggtggacaagggcgcttccgcccagagcttcatcgagcggatgaccaacttcgataagaacctgcccaacgagaaggtgctgcccaagcacagcctgctgtacgagtacttcaccgtgtataacgagctgaccaaagtgaaatacgtgaccgagggaatgagaaagcccgccttcctgagcggcgagcagaaaaaggccatcgtggacctgctgttcaagaccaaccggaaagtgaccgtgaagcagctgaaagaggactacttcaagaaaatcgagtgcttcgactccgtggaaatctccggcgtggaagatcggttcaacgcctccctgggcacataccacgatctgctgaaaattatcaaggacaaggacttcctggacaatgaggaaaacgaggacattctggaagatatcgtgctgaccctgacactgtttgaggacagagagatgatcgaggaacggctgaaaacctatgcccacctgttcgacgacaaagtgatgaagcagctgaagcggcggagatacaccggctggggcaggctgagccggaagctgatcaacggcatccgggacaagcagtccggcaagacaatcctggatttcctgaagtccgacggcttcgccaacagaaacttcatgcagctgatccacgacgacagcctgacctttaaagaggacatccagaaagcccaggtgtccggccagggcgatagcctgcacgagcacattgccaatctggccggcagccccgccattaagaagggcatcctgcagacagtgaaggtggtggacgagctcgtgaaagtgatgggccggcacaagcccgagaacatcgtgatcgccatggccagagagaaccagaccacccagaagggacagaagaacagccgcgagagaatgaagcggatcgaagagggcatcaaagagctgggcagccagatcctgaaagaacaccccgtggaaaacacccagctgcagaacgagaagctgtacctgtactacctgcagaatgggcgggatatgtacgtggaccaggaactggacatcaaccggctgtccgactacgatgtggacgccatcgtgcctcagagctttctgaaggacgactccatcgacgccaaggtgctgaccagaagcgacaaggcccggggcaagagcgacaacgtgccctccgaagaggtcgtgaagaagatgaagaactactggcggcagctgctgaacgccaagctgattacccagagaaagttcgacaatctgaccaaggccgagagaggcggcctgagcgaactggataaggccggcttcatcaagagacagctggtggaaacccggcagatcacaaagcacgtggcacagatcctggactcccggatgaacactaagtacgacgagaatgacaagctgatccgggaagtgaaagtgatcaccctgaagtccaagctggtgtccgatttccggaaggatttccagttttacaaagtgcgcgagatcaacaactaccaccacgcccacgccgcctacctgaacgccgtcgtgggaaccgccctgatcaaaaagtaccctaagctggaaagcgagttcgtgtacggcgactacaaggtgtacgacgtgcggaagatgatcgccaagagcgagcaggaaatcggcaaggctaccgccaagtacttcttctacagcaacatcatgaactttttcaagaccgagattaccctggccaacggcgagatccggaagcggcctctgatcgagacaaacggcgaaaccggggagatcgtgtgggataagggccgggattttgccaccgtgcggaaagtgctgagcatgccccaagtgaatatcgtgaaaaagaccgaggtgcagacaggcggcttcagcaaagagtctatcctgcccaagaggaacagcgataagctgatcgccagaaagaaggactgggaccctaagaagtacggcggcttcgacagccccaccgtggcctattctgtgctggtggtggccaaagtggaaaagggcaagtccaagaaactgaagagtgtgaaagagctgctggggatcaccatcatggaaagaagcagcttcgagaagaatcccatcgactttctggaagccaagggctacaaagaagtgaaaaaggacctgatcatcaagctgcctaagtactccctgttcgagctggaaaacggccggaagagaatgctggcctctgccggcgaactgcagaagggaaacgaactggccctgccctccaaatatgtgaacttcctgtacctggccagccactatgagaagctgaagggctcccccgaggataatgagcagaaacagctgtttgtggaacagcacaagcactacctggacgagatcatcgagcagatcagcgagttctccaagagagtgatcctggccgacgctaatctggacaaagtgctgtccgcctacaacaagcaccgggataagcccatcagagagcaggccgagaatatcatccacctgtttaccctgaccaatctgggagcccctgccgccttcaagtactttgacaccaccatcgaccggaagaggtacaccagcaccaaagaggtgctggacgccaccctgatccaccagagcatcaccggcctgtacgagacacggatcgacctgtctcagctgggaggcgac

SEQ ID NO: 139 - protein, 1368 aa, Homo sapiens
MDKKYSIGLDIGTNSVGWAVITDEYKVPSKKFKVLGNTDRHSIKKNLIGALLFDSGETAEATRLKRTARRRYTRRKNRICYLQEIFSNEMAKVDDSFFHRLEESFLVEEDKKHERHPIFGNIVDEVAYHEKYPTIYHLRKKLVDSTDKADLRLIYLALAHMIKFRGHFLIEGDLNPDNSDVDKLFIQLVQTYNQLFEENPINASGVDAKAILSARLSKSRRLENLIAQLPGEKKNGLFGNLIALSLGLTPNFKSNFDLAEDAKLQLSKDTYDDDLDNLLAQIGDQYADLFLAAKNLSDAILLSDILRVNTEITKAPLSASMIKRYDEHHQDLTLLKALVRQQLPEKYKEIFFDQSKNGYAGYIDGGASQEEFYKFIKPILEKMDGTEELLVKLNREDLLRKQRTFDNGSIPHQIHLGELHAILRRQEDFYPFLKDNREKIEKILTFRIPYYVGPLARGNSRFAWMTRKSEETITPWNFEEVVDKGASAQSFIERMTNFDKNLPNEKVLPKHSLLYEYFTVYNELTKVKYVTEGMRKPAFLSGEQKKAIVDLLFKTNRKVTVKQLKEDYFKKIECFDSVEISGVEDRFNASLGTYHDLLKIIKDKDFLDNEENEDILEDIVLTLTLFEDREMIEERLKTYAHLFDDKVMKQLKRRRYTGWGRLSRKLINGIRDKQSGKTILDFLKSDGFANRNFMQLIHDDSLTFKEDIQKAQVSGQGDSLHEHIANLAGSPAIKKGILQTVKVVDELVKVMGRHKPENIVIAMARENQTTQKGQKNSRERMKRIEEGIKELGSQILKEHPVENTQLQNEKLYLYYLQNGRDMYVDQELDINRLSDYDVDAIVPQSFLKDDSIDAKVLTRSDKARGKSDNVPSEEVVKKMKNYWRQLLNAKLITQRKFDNLTKAERGGLSELDKAGFIKRQLVETRQITKHVAQILDSRMNTKYDENDKLIREVKVITLKSKLVSDFRKDFQFYKVREINNYHHAHAAYLNAVVGTALIKKYPKLESEFVYGDYKVYDVRKMIAKSEQEIGKATAKYFFYSNIMNFFKTEITLANGEIRKRPLIETNGETGEIVWDKGRDFATVRKVLSMPQVNIVKKTEVQTGGFSKESILPKRNSDKLIARKKDWDPKKYGGFDSPTVAYSVLVVAKVEKGKSKKLKSVKELLGITIMERSSFEKNPIDFLEAKGYKEVKKDLIIKLPKYSLFELENGRKRMLASAGELQKGNELALPSKYVNFLYLASHYEKLKGSPEDNEQKQLFVEQHKHYLDEIIEQISEFSKRVILADANLDKVLSAYNKHRDKPIREQAENIIHLFTLTNLGAPAAFKYFDTTIDRKRYTSTKEVLDATLIHQSITGLYETRIDLSQLGGD

SEQ ID NO: 140 - RNA, 155 nt, Suterella wadsworthensis; identical to SEQ ID NO: 102

SEQ ID NO: 141 - RNA, 107 nt, Treponema denticola; identical to SEQ ID NO: 103

SEQ ID NO: 142 - RNA, 99 nt, Filifactor alocis; identical to SEQ ID NO: 104

SEQ ID NO: 143 - RNA, 91 nt, Staphylococcus pseudintermedius; identical to SEQ ID NO: 105

SEQ ID NO: 144 - RNA, 94 nt, Lactobacillus johnsonii; identical to SEQ ID NO: 106

SEQ ID NO: 145 - RNA, 78 nt, Eubacterium ventriosum; identical to SEQ ID NO: 107

SEQ ID NO: 146 - RNA, 84 nt, Streptococcus pasteurianus; identical to SEQ ID NO: 108

SEQ ID NO: 147 - RNA, 85 nt, Lactobacillus farciminis; identical to SEQ ID NO: 109

SEQ ID NO: 148 - RNA, 100 nt, Bacteroides coprophilus; identical to SEQ ID NO: 110

SEQ ID NO: 149 - RNA, 102 nt, Flaviivola taffensis; identical to SEQ ID NO: 111

SEQ ID NO: 150 - RNA, 90 nt, Flavobacterium columnare; identical to SEQ ID NO: 112

SEQ ID NO: 151 - RNA, 78 nt, Sphaerochaeta globus; identical to SEQ ID NO: 113

SEQ ID NO: 152 - RNA, 85 nt, Azospirillum sp.; identical to SEQ ID NO: 114

SEQ ID NO: 153 - RNA, 126 nt, Gluconacetobacter diazotrophicus; identical to SEQ ID NO: 115

SEQ ID NO: 154 - RNA, 82 nt, Roseburia intestinalis; identical to SEQ ID NO: 116

SEQ ID NO: 155 - RNA, 83 nt, Staphylococcus aureus; identical to SEQ ID NO: 117

SEQ ID NO: 156 - RNA, 94 nt, Mycoplasma gallisepticum; identical to SEQ ID NO: 118

SEQ ID NO: 157 - RNA, 117 nt, Campylobacter lari
guuuuagucucugaaaagagacuaaaauaagugguuuuuggucauccacgcaggguuacaaucccuuuaaaaccauuaaaauucaaauaaacuagguuguaucaacuuaguuuuuuu

SEQ ID NO: 158 - RNA, 119 nt, Artificial Sequence
  source: /note="Description of Artificial Sequence: Synthetic polynucleotide"
  modified_base (1)..(20): a, c, u, g, unknown or other
nnnnnnnnnnnnnnnnnnnnacugggguucaggaaacugaaccucaguaagcauuggcucguuuccaauguugauugcuccgccggugcuccuuauuuuuaagggcgccggcuuuuuuu

SEQ ID NO: 159 - protein, 1084 aa, Corynebacterium diphtheriae
MKYHVGIDVGTFSVGLAAIEVDDAGMPIKTLSLVSHIHDSGLDPDEIKSAVTRLASSGIARRTRRLYRRKRRRLQQLDKFIQRQGWPVIELEDYSDPLYPWKVRAELAASYIADEKERGEKLSVALRHIARHRGWRNPYAKVSSLYLPDGPSDAFKAIREEIKRASGQPVPETATVGQMVTLCELGTLKLRGEGGVLSARLQQSDYAREIQEICRMQEIGQELYRKIIDVVFAAESPKGSASSRVGKDPLQPGKNRALKASDAFQRYRIAALIGNLRVRVDGEKRILSVEEKNLVFDHLVNLTPKKEPEWVTIAEILGIDRGQLIGTATMTDDGERAGARPPTHDTNRSIVNSRIAPLVDWWKTASALEQHAMVKALSNAEVDDFDSPEGAKVQAFFADLDDDVHAKLDSLHLPVGRAAYSEDTLVRLTRRMLSDGVDLYTARLQEFGIEPSWTPPTPRIGEPVGNPAVDRVLKTVSRWLESATKTWGAPERVIIEHVREGFVTEKRAREMDGDMRRRAARNAKLFQEMQEKLNVQGKPSRADLWRYQSVQRQNCQCAYCGSPITFSNSEMDHIVPRAGQGSTNTRENLVAVCHRCNQSKGNTPFAIWAKNTSIEGVSVKEAVERTRHWVTDTGMRSTDFKKFTKAVVERFQRATMDEEIDARSMESVAWMANELRSRVAQHFASHGTTVRVYRGSLTAEARRASGISGKLKFFDGVGKSRLDRRHHAIDAAVIAFTSDYVAETLAVRSNLKQSQAHRQEAPQWREFTGKDAEHRAAWRVWCQKMEKLSALLTEDLRDDRVVVMSNVRLRLGNGSAHKETIGKLSKVKLSSQLSVSDIDKASSEALWCALTREPGFDPKEGLPANPERHIRVNGTHVYAGDNIGLFPVSAGSIALRGGYAELGSSFHHARVYKITSGKKPAFAMLRVYTIDLLPYRNQDLFSVELKPQTMSMRQAEKKLRDALATGNAEYLGWLVVDDELVVDTSKIATDQVKAVEAELGTIRRWRVDGFFSPSKLRLRPLQMSKEGIKKESAPELSKIIDRPGWLPAVNKLFSDGNVTVVRRDSLGRVRLESTAHLPVTWKVQ

SEQ ID NO: 160 - DNA, 3336 bp, Artificial Sequence
  source: /note="Description of Artificial Sequence: Synthetic polynucleotide"
accggtgccaccatgtacccatacgatgttccagattacgcttcgccgaagaaaaagcgcaaggtcgaagcgtccatgaagtaccatgtcggaatcgatgtcggaaccttttctgtggggctggctgctattgaagtggatgacgctggaatgcctattaagaccctgagtctggtgtcacacattcatgactcaggactggatcctgacgagatcaagagcgctgtgaccaggctggcaagctccggaatcgcccggagaacaaggcgcctgtaccgacggaagagaaggcgcctgcagcagctggataagttcatccagaggcagggctggccagtgatcgagctggaagattacagcgaccccctgtatccttggaaggtgcgcgccgaactggccgcttcttatattgctgacgagaaggaacggggggagaaactgagtgtggctctgagacacatcgcaaggcatcgcggatggaggaacccttacgccaaggtgtctagtctgtatctgccagatggcccctcagacgccttcaaggctattagggaggaaatcaaacgcgctagcggccagcctgtgccagagactgcaaccgtcgggcagatggtgaccctgtgcgaactgggcacactgaagctgcgaggagagggaggagtgctgagtgcacggctgcagcagtcagattacgcccgcgagatccaggaaatttgtcgaatgcaggagatcggccaggaactgtatcgcaagatcattgacgtggtgttcgcagccgagtccccaaagggctctgcctcaagccgggtggggaaagatcctctgcagccaggaaagaacagagcactgaaagccagcgacgcttttcagcgataccggattgctgcactgatcggcaatctgagagtcagggtggatggggagaagaggattctgagcgtggaggagaagaacctggtgttcgaccacctggtgaatctgactccaaagaaagagcccgaatgggtgaccatcgccgaaattctgggcatcgatcgcgggcagctgatcggaacagctactatgaccgacgatggagagcgagcaggagcccgaccccctacacacgatactaacagaagtattgtgaacagccggatcgcaccactggtcgactggtggaaaacagctagcgcactggagcagcacgccatggtgaaggcactgtccaacgccgaagtcgacgattttgattctcccgagggagcaaaagtgcaggcattctttgccgatctggacgatgacgtccacgccaagctggacagcctgcatctgcctgtgggacgagcagcttactccgaggacactctggtcagactgacccgacggatgctgagtgatggggtggacctgtataccgcccggctgcaggagttcggaattgaacctagctggaccccacccacaccaagaatcggagagcctgtcggcaatccagccgtcgaccgggtgctgaaaacagtgagcagatggctggaatccgcaacaaagacttggggcgccccagagagggtcatcattgagcacgtgcgcgaaggcttcgtcactgagaaacgcgctcgagaaatggatggggacatgagaaggcgcgcagcccggaacgccaagctgtttcaggagatgcaggaaaagctgaatgtgcagggcaaacccagtcgagccgatctgtggagataccagtcagtgcagagacagaactgccagtgtgcctattgcgggtccccaattaccttttctaatagtgaaatggaccacatcgtgcccagagcagggcagggatccaccaacacaagggagaatctggtcgccgtgtgccatcgctgtaaccagtctaagggcaatacacccttcgctatttgggcaaaaaacacttctatcgaaggggtcagtgtgaaggaggccgtggaacggaccagacattgggtcactgataccggcatgagaagcactgacttcaagaagttcaccaaggctgtggtcgagcggtttcagagagcaacaatggatgaggaaatcgacgccagaagcatggaatccgtcgcctggatggctaatgagctgaggagccgcgtggctcagcacttcgcatcccatggaaccacagtcagggtgtaccgaggcagcctgacagcagaggctcgacgggcatctgggatcagtggaaagctgaaattctttgatggcgtggggaagtccaggctggatagaaggcaccatgctattgacgctgcagtgatcgcattcacctctgactatgtggccgaaacactggctgtccgctcaaacctgaaacagagccaggcccaccgacaggaggctcctcagtggagagagttcaccggcaaggatgcagagcatcgagcagcttggagagtgtggtgccagaagatggaaaaactgagcgccctgctgaccgaggacctgcgagatgaccgggtggtcgtgatgtctaacgtgcgactgcggctgggaaatggcagtgcccacaaggaaaccattggcaaactgtcaaaggtgaaactgtcctctcagctgtcagtcagcgatatcgacaaagcaagttcagaggccctgtggtgtgctctgaccagagagcccggattcgatcctaaggaaggcctgcccgctaaccctgagagacacatcagggtgaatgggacacatgtctacgccggggacaatattggactgtttccagtgtcagcaggaagcatcgcactgaggggaggatacgcagagctgggcagctccttccaccatgctcgcgtgtataaaattacttccggcaagaaacccgcatttgccatgctgagggtgtacaccatcgatctgctgccttatcgcaaccaggacctgtttagcgtggaactgaagccacagacaatgtccatgaggcaggctgagaagaaactgcgcgacgctctggcaactgggaatgcagaatatctgggatggctggtcgtggatgacgagctggtcgtggatacatctaagattgccactgaccaggtcaaagcagtggaggccgaactggggactatccgccgatggcgggtggatggattcttttccccctctaaactgagactgaggcctctgcagatgtccaaggaggggatcaagaaagagtccgctcccgaactgtctaaaatcattgacagaccaggatggctgcccgccgtgaacaagctgttctctgatggaaatgtcaccgtcgtgcggagagactctctgggacgcgtgcgactggagagtacagcccacctgcctgtcacttggaaggtgcagtaagaattc

SEQ ID NO: 161 - RNA, 175 nt, Artificial Sequence
  source: /note="Description of Artificial Sequence: Synthetic polynucleotide"
  modified_base (1)..(20): a, c, u, g, unknown or other
nnnnnnnnnnnnnnnnnnnnguuucagugcuauaggaaacuauaggaaaucaccuucgggugagcugaaauccccuaaagcuaagauugaauccggccacuaucuauuaguagauauccggauauucugauauaaaaccucauucuuugauuagaccaaaggaugagguuuuuuu

SEQ ID NO: 162 - protein, 1422 aa, Sutterella wadsworthensis
MTQSERRFSCSIGIDMGAKYTGVFYALFDREELPTNLNSKAMTLVMPETGPRYVQAQRTAVRHRLRGQKRYTLARKLAFLVVDDMIKKQEKRLTDEEWKRGREALSGLLKRRGYSRPNADGEDLTPLENVRADVFAAHPAFSTYFSEVRSLAEQWEEFTANISNVEKFLGDPNIPADKEFIEFAVAEGLIDKTEKKAYQSALSTLRANANVLTGLRQMGHKPRSEYFKAIEADLKKDSRLAKINEAFGGAERLARLLGNLSNLQLRAERWYFNAPDIMKDRGWEPDRFKKTLVRAFKFFHPAKDQNKQHLELIKQIENSEDIIETLCTLDPNRTIPPYEDQNNRRPPLDQTLLLSPEKLTRQYGEIWKTWSARLTSAEPTLAPAAEILERSTDRKSRVAVNGHEPLPTLAYQLSYALQRAFDRSKALDPYALRALAAGSKSNKLTSARTALENCIGGQNVKTFLDCARRYYREADDAKVGLWFDNADGLLERSDLHPPMKKKILPLLVANILQTDETTGQKFLDEIWRKQIKGRETVASRCARIETVRKSFGGGFNIAYNTAQYREVNKLPRNAQDKELLTIRDRVAETADFIAANLGLSDEQKRKFANPFSLAQFYTLIETEVSGFSATTLAVHLENAWRMTIKDAVINGETVRAAQCSRLPAETARPFDGLVRRLVDRQAWEIAKRVSTDIQSKVDFSNGIVDVSIFVEENKFEFSASVADLKKNKRVKDKMLSEAEKLETRWLIKNERIKKASRGTCPYTGDRLAEGGEIDHILPRSLIKDARGIVFNAEPNLIYASSRGNQLKKNQRYSLSDLKANYRNEIFKTSNIAAITAEIEDVVTKLQQTHRLKFFDLLNEHEQDCVRHALFLDDGSEARDAVLELLATQRRTRVNGTQIWMIKNLANKIREELQNWCKTTNNRLHFQAAATNVSDAKNLRLKLAQNQPDFEKPDIQPIASHSIDALCSFAVGSADAERDQNGFDYLDGKTVLGLYPQSCEVIHLQAKPQEEKSHFDSVAIFKEGIYAEQFLPIFTLNEKIWIGYETLNAKGERCGAIEVSGKQPKELLEMLAPFFNKPVGDLSAHATYRILKKPAYEFLAKAALQPLSAEEKRLAALLDALRYCTSRKSLMSLFMAANGKSLKKREDVLKPKLFQLKVELKGEKSFKLNGSLTLPVKQDWLRICDSPELADAFGKPCSADELTSKLARIWKRPVMRDLAHAPVRREFSLPAIDNPSGGFRIRRTNLFGNELYQVHAINAKKYRGFASAGSNVDWSKGILFNELQHENLTECGGRFITSADVTPMSEWRKVVAEDNLSIWIAPGTEGRRYVRVETTFIQASHWFEQSVENWAITSPLSLPASFKVDKPAEFQKAVGTELSELLGQPRSEIFIENVGNAKHIRFWYIVVSSNKKMNESYNNVSKS

SEQ ID NO: 163 - DNA, 4350 bp, Artificial Sequence; identical to SEQ ID NO: 119
  source: /note="Description of Artificial Sequence: Synthetic polynucleotide"

SEQ ID NO: 164 - RNA, 112 nt, Artificial Sequence
  source: /note="Description of Artificial Sequence: Synthetic polynucleotide"
  modified_base (1)..(20): a, c, u, g, unknown or other
nnnnnnnnnnnnnnnnnnnnguuucaguggugaaaacccugaaaucaacaaaauuaaagauugaaucguuuuucuaugcucgucuuaauagcgagcauauaacgauuuuuuu

SEQ ID NO: 165 - protein, 1372 aa, Legionella pneumophila
MESSQILSPIGIDLGGKFTGVCLSHLEAFAELPNHANTKYSVILIDHNNFQLSQAQRRATRHRVRNKKRNQFVKRVALQLFQHILSRDLNAKEETALCHYLNNRGYTYVDTDLDEYIKDETTINLLKELLPSESEHNFIDWFLQKMQSSEFRKILVSKVEEKKDDKELKNAVKNIKNFITGFEKNSVEGHRHRKVYFENIKSDITKDNQLDSIKKKIPSVCLSNLLGHLSNLQWKNLHRYLAKNPKQFDEQTFGNEFLRMLKNFRHLKGSQESLAVRNLIQQLEQSQDYISILEKTPPEITIPPYEARTNTGMEKDQSLLLNPEKLNNLYPNWRNLIPGIIDAHPFLEKDLEHTKLRDRKRIISPSKQDEKRDSYILQRYLDLNKKIDKFKIKKQLSFLGQGKQLPANLIETQKEMETHFNSSLVSVLIQIASAYNKEREDAAQGIWFDNAFSLCELSNINPPRKQKILPLLVGAILSEDFINNKDKWAKFKIFWNTHKIGRTSLKSKCKEIEEARKNSGNAFKIDYEEALNHPEHSNNKALIKIIQTIPDIIQAIQSHLGHNDSQALIYHNPFSLSQLYTILETKRDGFHKNCVAVTCENYWRSQKTEIDPEISYASRLPADSVRPFDGVLARMMQRLAYEIAMAKWEQIKHIPDNSSLLIPIYLEQNRFEFEESFKKIKGSSSDKTLEQAIEKQNIQWEEKFQRIINASMNICPYKGASIGGQGEIDHIYPRSLSKKHFGVIFNSEVNLIYCSSQGNREKKEEHYLLEHLSPLYLKHQFGTDNVSDIKNFISQNVANIKKYISFHLLTPEQQKAARHALFLDYDDEAFKTITKFLMSQQKARVNGTQKFLGKQIMEFLSTLADSKQLQLEFSIKQITAEEVHDHRELLSKQEPKLVKSRQQSFPSHAIDATLTMSIGLKEFPQFSQELDNSWFINHLMPDEVHLNPVRSKEKYNKPNISSTPLFKDSLYAERFIPVWVKGETFAIGFSEKDLFEIKPSNKEKLFTLLKTYSTKNPGESLQELQAKSKAKWLYFPINKTLALEFLHHYFHKEIVTPDDTTVCHFINSLRYYTKKESITVKILKEPMPVLSVKFESSKKNVLGSFKHTIALPATKDWERLFNHPNFLALKANPAPNPKEFNEFIRKYFLSDNNPNSDIPNNGHNIKPQKHKAVRKVFSLPVIPGNAGTMMRIRRKDNKGQPLYQLQTIDDTPSMGIQINEDRLVKQEVLMDAYKTRNLSTIDGINNSEGQAYATFDNWLTLPVSTFKPEIIKLEMKPHSKTRRYIRITQSLADFIKTIDEALMIKPSDSIDDPLNMPNEIVCKNKLFGNELKPRDGKMKIVSTGKIVTYEFESDSTPQWIQTLYVTQLKKQP

SEQ ID NO: 166 - DNA, 4200 bp, Artificial Sequence
  source: /note="Description of Artificial Sequence: Synthetic polynucleotide"
accggtgccaccatgtacccatacgatgttccagattacgcttcgccgaagaaaaagcgcaaggtcgaagcgtccatggagtcctctcagatcctgtcacctatcggcatcgacctgggcggaaagtttactggagtctgcctgtcacacctggaagcatttgctgagctgcctaaccacgcaaatacaaagtactcagtgatcctgattgatcataacaatttccagctgagccaggcacagcggagagccactagacacagggtgcgcaacaagaaaagaaatcagttcgtgaagagggtcgccctgcagctgtttcagcacatcctgtcccgggacctgaacgccaaggaggaaaccgctctgtgccattacctgaacaatagaggctacacctatgtggacacagatctggacgagtatatcaaagatgaaaccacaattaacctgctgaaggagctgctgccaagcgagtccgaacataatttcattgactggtttctgcagaagatgcagagctccgagttccggaagatcctggtgagcaaagtcgaggaaaagaaagacgataaagaactgaagaacgccgtgaagaacatcaagaacttcatcaccggattcgagaaaaatagcgtggaaggccaccgacatcggaaggtctactttgagaacatcaagtccgatattacaaaagacaatcagctggattctatcaagaaaaagattcctagcgtgtgtctgtccaacctgctgggccacctgtccaacctgcagtggaagaatctgcataggtatctggccaaaaatccaaagcagttcgacgagcagaccttcgggaacgaatttctgcggatgctgaagaattttcgacacctgaaaggatctcaggagagtctggctgtgcgcaacctgatccagcagctggaacagtctcaggattacatcagtatcctggagaaaaccccccctgaaatcaccattccaccctatgaggcccggacaaacactggcatggaaaaagaccagagcctgctgctgaaccccgagaagctgaacaatctgtacccaaactggagaaatctgatccccgggatcattgacgcccaccctttcctggagaaggatctggaacatacaaagctgagagacaggaaacgcatcatttctcccagtaaacaggacgagaagcgggatagctacatcctgcagagatatctggacctgaacaaaaagatcgataagttcaagatcaagaagcagctgagctttctgggacagggcaaacagctgcctgctaacctgatcgagacacagaaggagatggaaactcacttcaattctagtctggtgtctgtcctgatccagattgctagtgcatacaacaaggagagggaagatgccgctcaggggatctggttcgacaatgccttttcactgtgcgagctgagcaacatcaatcctccacgcaaacagaagattctgcccctgctggtgggagcaatcctgagcgaggacttcattaacaacaaggataagtgggccaaattcaagatcttttggaacacccacaagattgggcgaacatcactgaaaagcaagtgtaaagagatcgaggaagcccggaagaacagtggaaacgcttttaaaatcgactacgaggaagctctgaatcacccagagcattcaaacaacaaggccctgatcaagatcattcagaccattcccgatatcattcaggccatccagtcacacctgggacataacgacagccaggctctgatctaccacaatcctttctcactgagccagctgtatactatcctggagacaaagagggatggctttcataaaaactgcgtggccgtcacttgtgaaaattactggcggagccagaaaaccgagatcgacccagaaatttcctatgcatctaggctgccagcagacagtgtgcgccccttcgatggcgtcctggcacgaatgatgcagcggctggcctacgagatcgccatggctaagtgggaacagatcaaacacattcctgataactcaagcctgctgatcccaatctacctggagcagaatcggttcgaatttgaggagagcttcaagaagatcaaggggtcctctagtgacaaaaccctggagcaggccatcgaaaagcagaacattcagtgggaggaaaagttccagagaatcattaacgcaagtatgaatatctgcccttacaagggcgcctcaattggcgggcagggggagatcgaccacatctacccaaggtccctgtctaaaaagcatttcggcgtgatctttaactccgaagtcaatctgatctactgttcaagccaggggaatcgcgagaaaaaggaggaacactacctgctggaacatctgtctccactgtatctgaaacaccagttcggcactgacaacgtgtccgatatcaagaattttatttctcagaacgtcgctaatatcaaaaagtacatttccttccacctgctgaccccagagcagcagaaggcagcacggcacgccctgtttctggattatgacgatgaagcattcaaaaccattacaaagtttctgatgtctcagcagaaggccagagtgaacggcacacagaaattcctggggaagcagatcatggagtttctgtccactctggcagattctaaacagctgcagctggagttcagcatcaagcagattaccgccgaggaagtgcacgaccatagagagctgctgtctaagcaggaacccaaactggtcaagagtaggcagcagagtttcccttcacacgctatcgacgcaactctgaccatgtctattgggctgaaggagttcccacagtttagtcaggaactggataactcatggtttatcaatcacctgatgccagacgaggtgcatctgaaccccgtccggagcaaggaaaagtacaacaaacctaacatctcctctactccactgttcaaggattccctgtatgctgagcggttcatccccgtgtgggtcaagggagaaaccttcgcaatcggctttagcgagaaggacctgttcgagatcaagccctccaacaaggagaaactgtttacactgctgaaaacctacagtactaaaaatcctggcgagtcactgcaggaactgcaggctaagagcaaagcaaagtggctgtacttcccaatcaacaaaaccctggccctggagttcctgcaccattattttcacaaggaaatcgtgacacccgacgatactaccgtctgccatttcatcaactcactgagatactacactaaaaaggagagcatcaccgtgaaaattctgaaggaacccatgcctgtgctgtccgtcaagttcgagagttcaaaaaagaacgtgctgggatcttttaaacacacaatcgccctgcctgctactaaggattgggagaggctgttcaaccatccaaattttctggcactgaaggccaacccagctcccaatcctaaagagttcaatgagttcatccgcaagtacttcctgagcgacaacaatcccaactccgatatccctaacaatggccacaatatcaagccccagaaacataaggccgtgcgaaaggtctttagcctgccagtgatccccgggaacgctggaaccatgatgcgcattaggcgcaaagacaataagggacagccactgtatcagctgcagacaatcgacgatactcccagcatgggcatccagattaacgaggatcgcctggtgaaacaggaagtcctgatggacgcctacaagacacgaaatctgagcactatcgatgggattaacaattccgagggacaggcatatgccacattcgacaactggctgaccctgcccgtgagcaccttcaagcctgagatcatcaagctggaaatgaagcctcactctaaaacccgacggtacatcagaattacacagagtctggccgacttcatcaaaactattgatgaggctctgatgatcaagcccagtgactcaattgacgatcctctgaacatgccaaatgagatcgtgtgtaaaaacaagctgttcgggaatgaactgaagcctagggatggaaaaatgaagatcgtgagcactggcaagattgtcacctacgagtttgaaagcgactccaccccccagtggatccagaccctgtatgtgacacagctgaaaaagcagccttaagaattc

SEQ ID NO: 167 - RNA, 127 nt, Artificial Sequence
  source: /note="Description of Artificial Sequence: Synthetic polynucleotide"
  modified_base (1)..(20): a, c, u, g, unknown or other
nnnnnnnnnnnnnnnnnnnnguuugagaguuggaaacaacgaguucaaauaagaauucaucaaaaucgucccuuuugggaccgcucauuguggagcaucaaggcuuaacaugguuaagccuuuuuuu

SEQ ID NO: 168 - protein, 1395 aa, Treponema denticola
MKKEIKDYFLGLDVGTGSVGWAVTDTDYKLLKANRKDLWGMRCFETAETAEVRRLHRGARRRIERRKKRIKLLQELFSQEIAKTDEGFFQRMKESPFYAEDKTILQENTLFNDKDFADKTYHKAYPTINHLIKAWIENKVKPDPRLLYLACHNIIKKRGHFLFEGDFDSENQFDTSIQALFEYLREDMEVDIDADSQKVKEILKDSSLKNSEKQSRLNKILGLKPSDKQKKAITNLISGNKINFADLYDNPDLKDAEKNSISFSKDDFDALSDDLASILGDSFELLLKAKAVYNCSVLSKVIGDEQYLSFAKVKIYEKHKTDLTKLKNVIKKHFPKDYKKVFGYNKNEKNNNNYSGYVGVCKTKSKKLIINNSVNQEDFYKFLKTILSAKSEIKEVNDILTEIETGTFLPKQISKSNAEIPYQLRKMELEKILSNAEKHFSFLKQKDEKGLSHSEKIIMLLTFKIPYYIGPINDNHKKFFPDRCWVVKKEKSPSGKTTPWNFFDHIDKEKTAEAFITSRTNFCTYLVGESVLPKSSLLYSEYTVLNEINNLQIIIDGKNICDIKLKQKIYEDLFKKYKKITQKQISTFIKHEGICNKTDEVIILGIDKECTSSLKSYIELKNIFGKQVDEISTKNMLEEIIRWATIYDEGEGKTILKTKIKAEYGKYCSDEQIKKILNLKFSGWGRLSRKFLETVTSEMPGFSEPVNIITAMRETQNNLMELLSSEFTFTENIKKINSGFEDAEKQFSYDGLVKPLFLSPSVKKMLWQTLKLVKEISHITQAPPKKIFIEMAKGAELEPARTKTRLKILQDLYNNCKNDADAFSSEIKDLSGKIENEDNLRLRSDKLYLYYTQLGKCMYCGKPIEIGHVFDTSNYDIDHIYPQSKIKDDSISNRVLVCSSCNKNKEDKYPLKSEIQSKQRGFWNFLQRNNFISLEKLNRLTRATPISDDETAKFIARQLVETRQATKVAAKVLEKMFPETKIVYSKAETVSMFRNKFDIVKCREINDFHHAHDAYLNIVVGNVYNTKFTNNPWNFIKEKRDNPKIADTYNYYKVFDYDVKRNNITAWEKGKTIITVKDMLKRNTPIYTRQAACKKGELFNQTIMKKGLGQHPLKKEGPFSNISKYGGYNKVSAAYYTLIEYEEKGNKIRSLETIPLYLVKDIQKDQDVLKSYLTDLLGKKEFKILVPKIKINSLLKINGFPCHITGKTNDSFLLRPAVQFCCSNNEVLYFKKIIRFSEIRSQREKIGKTISPYEDLSFRSYIKENLWKKTKNDEIGEKEFYDLLQKKNLEIYDMLLTKHKDTIYKKRPNSATIDILVKGKEKFKSLIIENQFEVILEILKLFSATRNVSDLQHIGGSKYSGVAKIGNKISSLDNCILIYQSITGIFEKRIDLLKV

SEQ ID NO: 169 - DNA, 4269 bp, Artificial Sequence; identical to SEQ ID NO: 120
  source: /note="Description of Artificial Sequence: Synthetic polynucleotide"

SEQ ID NO: 170 - RNA, 119 nt, Artificial Sequence
  source: /note="Description of Artificial Sequence: Synthetic polynucleotide"
  modified_base (1)..(20): a, c, u, g, unknown or other
nnnnnnnnnnnnnnnnnnnnguuugagaguaggaaacuacacgguucaaauaaagaauuuuucuaaucgcccaaugggcccauauugauauggaugaaacucgcuuagcgaguuuuuuu

SEQ ID NO: 171 - protein, 1365 aa, Filifactor alocis
MTKEYYLGLDVGTNSVGWAVTDSQYNLCKFKKKDMWGIRLFESANTAKDRRLQRGNRRRLERKKQRIDLLQEIFSPEICKIDPTFFIRLNESRLHLEDKSNDFKYPLFIEKDYSDIEYYKEFPTIFHLRKHLIESEEKQDIRLIYLALHNIIKTRGHFLIDGDLQSAKQLRPILDTFLLSLQEEQNLSVSLSENQKDEYEEILKNRSIAKSEKVKKLKNLFEISDELEKEEKKAQSAVIENFCKFIVGNKGDVCKFLRVSKEELEIDSFSFSEGKYEDDIVKNLEEKVPEKVYLFEQMKAMYDWNILVDILETEEYISFAKVKQYEKHKTNLRLLRDIILKYCTKDEYNRMFNDEKEAGSYTAYVGKLKKNNKKYWIEKKRNPEEFYKSLGKLLDKIEPLKEDLEVLTMMIEECKNHTLLPIQKNKDNGVIPHQVHEVELKKILENAKKYYSFLTETDKDGYSVVQKIESIFRFRIPYYVGPLSTRHQEKGSNVWMVRKPGREDRIYPWNMEEIIDFEKSNENFITRMTNKCTYLIGEDVLPKHSLLYSKYMVLNELNNVKVRGKKLPTSLKQKVFEDLFENKSKVTGKNLLEYLQIQDKDIQIDDLSGFDKDFKTSLKSYLDFKKQIFGEEIEKESIQNMIEDIIKWITIYGNDKEMLKRVIRANYSNQLTEEQMKKITGFQYSGWGNFSKMFLKGISGSDVSTGETFDIITAMWETDNNLMQILSKKFTFMDNVEDFNSGKVGKIDKITYDSTVKEMFLSPENKRAVWQTIQVAEEIKKVMGCEPKKIFIEMARGGEKVKKRTKSRKAQLLELYAACEEDCRELIKEIEDRDERDFNSMKLFLYYTQFGKCMYSGDDIDINELIRGNSKWDRDHIYPQSKIKDDSIDNLVLVNKTYNAKKSNELLSEDIQKKMHSFWLSLLNKKLITKSKYDRLTRKGDFTDEELSGFIARQLVETRQSTKAIADIFKQIYSSEVVYVKSSLVSDFRKKPLNYLKSRRVNDYHHAKDAYLNIVVGNVYNKKFTSNPIQWMKKNRDTNYSLNKVFEHDVVINGEVIWEKCTYHEDTNTYDGGTLDRIRKIVERDNILYTEYAYCEKGELFNATIQNKNGNSTVSLKKGLDVKKYGGYFSANTSYFSLIEFEDKKGDRARHIIGVPIYIANMLEHSPSAFLEYCEQKGYQNVRILVEKIKKNSLLIINGYPLRIRGENEVDTSFKRAIQLKLDQKNYELVRNIEKFLEKYVEKKGNYPIDENRDHITHEKMNQLYEVLLSKMKKFNKKGMADPSDRIEKSKPKFIKLEDLIDKINVINKMLNLLRCDNDTKADLSLIELPKNAGSFVVKKNTIGKSKIILVNQSVTGLYENRREL

SEQ ID NO: 172 - DNA, 4179 bp, Artificial Sequence; identical to SEQ ID NO: 121
  source: /note="Description of Artificial Sequence: Synthetic polynucleotide"

SEQ ID NO: 173 - RNA, 111 nt, Artificial Sequence
  source: /note="Description of Artificial Sequence: Synthetic polynucleotide"
  modified_base (1)..(20): a, c, u, g, unknown or other
nnnnnnnnnnnnnnnnnnnnguuuuagcacuagaaauaguuaaguuaaaacaagcuuaaagcgucaauguaauauuuuauuaacacccuacugugucagugggguuuuuuu

SEQ ID NO: 174 - protein, 1334 aa, Staphylococcus pseudintermedius
MGRKPYILSLDIGTGSVGYACMDKGFNVLKYHDKDALGVYLFDGALTAQERRQFRTSRRRKNRRIKRLGLLQELLAPLVQNPNFYQFQRQFAWKNDNMDFKNKSLSEVLSFLGYESKKYPTIYHLQEALLLKDEKFDPELIYMALYHLVKYRGHFLFDHLKIENLTNNDNMHDFVELIETYENLNNIKLNLDYEKTKVIYEILKDNEMTKNDRAKRVKNMEKKLEQFSIMLLGLKFNEGKLFNHADNAEELKGANQSHTFADNYEENLTPFLTVEQSEFIERANKIYLSLTLQDILKGKKSMAMSKVAAYDKFRNELKQVKDIVYKADSTRTQFKKIFVSSKKSLKQYDATPNDQTFSSLCLFDQYLIRPKKQYSLLIKELKKIIPQDSELYFEAENDTLLKVLNTTDNASIPMQINLYEAETILRNQQKYHAEITDEMIEKVLSLIQFRIPYYVGPLVNDHTASKFGWMERKSNESIKPWNFDEVVDRSKSATQFIRRMTNKCSYLINEDVLPKNSLLYQEMEVLNELNATQIRLQTDPKNRKYRMMPQIKLFAVEHIFKKYKTVSHSKFLEIMLNSNHRENFMNHGEKLSIFGTQDDKKFASKLSSYQDMTKIFGDIEGKRAQIEEIIQWITIFEDKKILVQKLKECYPELTSKQINQLKKLNYSGWGRLSEKLLTHAYQGHSIIELLRHSDENFMEILTNDVYGFQNFIKEENQVQSNKIQHQDIANLTTSPALKKGIWSTIKLVRELTSIFGEPEKIIMEFATEDQQKGKKQKSRKQLWDDNIKKNKLKSVDEYKYIIDVANKLNNEQLQQEKLWLYLSQNGKCMYSGQSIDLDALLSPNATKHYEVDHIFPRSFIKDDSIDNKVLVIKKMNQTKGDQVPLQFIQQPYERIAYWKSLNKAGLISDSKLHKLMKPEFTAMDKEGFIQRQLVETRQISVHVRDFLKEEYPNTKVIPMKAKMVSEFRKKFDIPKIRQMNDAHHAIDAYLNGVVYHGAQLAYPNVDLFDFNFKWEKVREKWKALGEFNTKQKSRELFFFKKLEKMEVSQGERLISKIKLDMNHFKINYSRKLANIPQQFYNQTAVSPKTAELKYESNKSNEVVYKGLTPYQTYVVAIKSVNKKGKEKMEYQMIDHYVFDFYKFQNGNEKELALYLAQRENKDEVLDAQIVYSLNKGDLLYINNHPCYFVSRKEVINAKQFELTVEQQLSLYNVMNNKETNVEKLLIEYDFIAEKVINEYHHYLNSKLKEKRVRTFFSESNQTHEDFIKALDELFKVVTASATRSDKIGSRKNSMTHRAFLGKGKDVKIAYTSISGLKTTKPKSLFKLAESRNEL

SEQ ID NO: 175 - DNA, 4086 bp, Artificial Sequence; identical to SEQ ID NO: 122
  source: /note="Description of Artificial Sequence: Synthetic polynucleotide"

SEQ ID NO: 176 - RNA, 114 nt, Artificial Sequence
  source: /note="Description of Artificial Sequence: Synthetic polynucleotide"
  modified_base (1)..(20): a, c, u, g, unknown or other
nnnnnnnnnnnnnnnnnnnnguuuuagauggugaaaaccagauuuaaaaucaagcaaugcaucuuuugaugcaaaguuucaauauuugucccacguuaucgagggacuuuuuuu

SEQ ID NO: 177 - protein, 1375 aa, Lactobacillus johnsonii
MTKIKDDYIVGLDIGTDSCGWVAMNSNNDILKLQGKTAIGSRLFEGGKSAAERRLFRTTHRRIKRRRWRLKLLEEFFDPYMAEVDPYFFARLKESGLSPLDKRKTVSSIVFPTSAEDKKFYDDYPTIYHLRYKLMTEDEKFDLREVYLAIHHIIKYRGNFLYNTSVKDFKASKIDVKSSIEKLNELYENLGLDLNVEFNISNTAEIEKVLKDKQIFKRDKVKKIAELFAIKTDNKEQSKRIKDISKQVANAVLGYKTRFDTIALKEISKDELSDWNFKLSDIDADSKFEALMGNLDENEQAILLTIKELFNEVTLNGIVEDGNTLSESMINKYNDHRDDLKLLKEVIENHIDRKKAKELALAYDLYVNNRHGQLLQAKKKLGKIKPRSKEDFYKVVNKNLDDSRASKEIKKKIELDSFMPKQRTNANGVIPYQLQQLELDKIIENQSKYYPFLKEINPVSSHLKEAPYKLDELIRFRVPYYVGPLISPNESTKDIQTKKNQNFAWMIRKEEGRITPWNFDQKVDRIESANKFIKRMTTKDTYLFGEDVLPANSLLYQKFTVLNELNNIRINGKRISVDLKQEIYENLFKKHTTVTVKKLENYLKENHNLVKVEIKGLADEKKFNSGLTTYNRFKNLNIFDNQIDDLKYRNDFEKIIEWSTIFEDKSIYKEKLRSIDWLNEKQINALSNIRLQGWGRLSKKLLAQLHDHNGQTIIEQLWDSQNNFMQIVTQADFKDAIAKANQNLLVATSVEDILNNAYTSPANKKAIRQVIKVVDDIVKAASGKVPKQIAIEFTRDADENPKRSQTRGSKLQKVYKDLSTELASKTIAEELNEAIKDKKLVQDKYYLYFMQLGRDAYTGEPINIDEIQKYDIDHILPQSFIKDDALDNRVLVSRAVNNGKSDNVPVKLFGNEMAANLGMTIRKMWEEWKNIGLISKTKYNNLLTDPDHINKYKSAGFIRRQLVETSQIIKLVSTILQSRYPNTEIITVKAKYNHYLREKFDLYKSREVNDYHHAIDAYLSAICGNLLYQNYPNLRPFFVYGQYKKFSSDPDKEKAIFNKTRKFSFISQLLKNKSENSKEIAKKLKRAYQFKYMLVSRETETRDQEMFKMTVYPRFSHDTVKAPRNLIPKKMGMSPDIYGGYTNNSDAYMVIVRIDKKKGTEYKILGIPTRELVNLKKAEKEDHYKSYLKEILTPRILYNKNGKRDKKITSFEIVKSKIPYKQVIQDGDKKFMLGSSTYVYNAKQLTLSTESMKAITNNFDKDSDENDALIKAYDEILDKVDKYLPLFDINKFREKLHSGREKFIKLSLEDKKDTILKVLEGLHDNAVMTKIPTIGLSTPLGFMQFPNGVILSENAKLIYQSPTGLFKKSVKISDL

SEQ ID NO: 178 - DNA, 4209 bp, Artificial Sequence; identical to SEQ ID NO: 123
  source: /note="Description of Artificial Sequence: Synthetic polynucleotide"

SEQ ID NO: 179 - RNA, 178 nt, Artificial Sequence
  source: /note="Description of Artificial Sequence: Synthetic polynucleotide"
  modified_base (1)..(20): a, c, u, g, unknown or other
nnnnnnnnnnnnnnnnnnnnguuguagcucccauucucgaaagagaaccguugcuacaauaaggccgucugaaaagaugugccgcaacgcucugccccuuaaagcuucugcuuuaaggggcaucguuuauuucgguuaaaaaugccgucugaaaccgguuuuuagguuucagacggca

SEQ ID NO: 180 - protein, 1082 aa, Neisseria cinerea
MAAFKPNPMNYILGLDIGIASVGWAIVEIDEEENPIRLIDLGVRVFERAEVPKTGDSLAAARRLARSVRRLTRRRAHRLLRARRLLKREGVLQAADFDENGLIKSLPNTPWQLRAAALDRKLTPLEWSAVLLHLIKHRGYLSQRKNEGETADKELGALLKGVADNTHALQTGDFRTPAELALNKFEKESGHIRNQRGDYSHTFNRKDLQAELNLLFEKQKEFGNPHVSDGLKEGIETLLMTQRPALSGDAVQKMLGHCTFEPTEPKAAKNTYTAERFVWLTKLNNLRILEQGSERPLTDTERATLMDEPYRKSKLTYAQARKLLDLDDTAFFKGLRYGKDNAEASTLMEMKAYHAISRALEKEGLKDKKSPLNLSPELQDEIGTAFSLFKTDEDITGRLKDRVQPEILEALLKHISFDKFVQISLKALRRIVPLMEQGNRYDEACTEIYGDHYGKKNTEEKIYLPPIPADEIRNPVVLRALSQARKVINGVVRRYGSPARIHIETAREVGKSFKDRKEIEKRQEENRKDREKSAAKFREYFPNFVGEPKSKDILKLRLYEQQHGKCLYSGKEINLGRLNEKGYVEIDHALPFSRTWDDSFNNKVLALGSENQNKGNQTPYEYFNGKDNSREWQEFKARVETSRFPRSKKQRILLQKFDEDGFKERNLNDTRYINRFLCQFVADHMLLTGKGKRRVFASNGQITNLLRGFWGLRKVRAENDRHHALDAVVVACSTIAMQQKITRFVRYKEMNAFDGKTIDKETGEVLHQKAHFPQPWEFFAQEVMIRVFGKPDGKPEFEEADTPEKLRTLLAEKLSSRPEAVHKYVTPLFISRAPNRKMSGQGHMETVKSAKRLDEGISVLRVPLTQLKLKDLEKMVNREREPKLYEALKARLEAHKDDPAKAFAEPFYKYDKAGNRTQQVKAVRVEQVQKTGVWVHNHNGIADNATIVRVDVFEKGGKYYLVPIYSWQVAKGILPDRAVVQGKDEEDWTVMDDSFEFKFVLYANDLIKLTAKKNEFLGYFVSLNRATGAIDIRTHDTDSTKGKNGIFQSVGVKTALSFQKYQIDELGKEIRPCRLKKRPPVR

SEQ ID NO: 181 - DNA, 3330 bp, Artificial Sequence
  source: /note="Description of Artificial Sequence: Synthetic polynucleotide"
accggtgccaccatgtacccatacgatgttccagattacgcttcgccgaagaaaaagcgcaaggtcgaagcgtccatggctgccttcaaacctaatcctatgaactacatcctgggcctggacattggaatcgcttctgtcgggtgggctatcgtggaaatcgacgaggaagagaaccctatcagactgattgatctgggagtcagagtgtttgaaagggcagaggtgccaaagaccggcgactccctggccgctgcacggagactggctcggtctgtcaggcgcctgacacgacggagagcacacaggctgctgcgagctaggcgcctgctgaagagagagggcgtgctgcaggccgctgacttcgatgaaaacggcctgatcaagagcctgcccaatactccttggcagctgagagcagccgctctggacaggaagctgaccccactggagtggtctgccgtgctgctgcacctgatcaagcatcgcggctacctgagtcagcgaaaaaatgaaggggagacagcagataaggagctgggagcactgctgaaaggagtggccgacaacactcatgctctgcagaccggcgattttaggacacccgctgagctggcactgaataagttcgaaaaagagagtggacacattcgaaaccagcggggcgactattcacataccttcaaccgcaaggatctgcaggccgagctgaatctgctgtttgaaaagcagaaagagttcgggaatccccacgtgtccgacgggctgaaagaaggaatcgagacactgctgatgactcagaggcctgcactgtctggcgatgccgtgcagaagatgctggggcattgcacctttgaaccaacagagcccaaggcagccaaaaacacctacacagccgagaggttcgtgtggctgacaaagctgaacaatctgcgcatcctggaacagggcagtgagcggcccctgactgacaccgaaagagccacactgatggatgagccttacaggaagtctaaactgacttatgcccaggctcgcaagctgctggacctggacgatactgccttctttaagggcctgaggtacgggaaagataatgcagaagccagcaccctgatggagatgaaggcctatcacgctatctcccgcgccctggaaaaagagggcctgaaggacaagaaatctcccctgaacctgagtcctgaactgcaggatgagattgggaccgcttttagcctgttcaagactgacgaggatatcaccggacgcctgaaagaccgagtgcagcccgaaattctggaggcactgctgaagcacatcagttttgataaattcgtgcagatttcactgaaggccctgcgacggatcgtccctctgatggagcagggcaatcggtacgacgaggcctgcaccgagatctacggagatcattatggcaagaaaaacacagaagagaaaatctatctgccccctattcctgccgacgagatccggaatccagtggtcctgagagctctgtcacaggcaagaaaagtgatcaacggagtggtcagaaggtacggcagccctgctaggatccacattgaaaccgcacgcgaagtgggaaagtcctttaaagaccgcaaggaaatcgagaagcgacaggaagagaatagaaaagatagggaaaagtctgctgcaaaattcagggagtactttccaaacttcgtgggcgaacccaagagtaaagacatcctgaagctgcgcctgtacgagcagcagcacgggaagtgtctgtatagcggaaaagaaattaacctgggccggctgaatgaaaagggctatgtggagatcgatcatgcactgcccttttccagaacatgggacgattctttcaacaataaggtcctggctctggggagcgagaaccagaacaagggaaatcagactccttacgaatatttcaacgggaaggacaatagccgagaatggcaggagtttaaagcccgcgtggagacaagccggttcccacgaagcaagaaacagcggattctgctgcagaagtttgacgaagatggattcaaagagagaaacctgaatgacacccggtacatcaacagatttctgtgccagttcgtggctgatcacatgctgctgaccggaaagggcaaacgccgagtctttgcaagcaacggccagatcacaaatctgctgaggggcttctgggggctgcggaaggtgagagccgagaatgaccgccaccatgcactggatgccgtggtcgtggcttgttccactattgcaatgcagcagaagatcaccaggtttgtgcgctataaagagatgaacgccttcgacggaaagacaattgataaagaaactggcgaggtgctgcaccagaaggcacattttcctcagccatgggagttcttcgcccaggaagtgatgatccgggtctttgggaagcctgacggaaaaccagagttcgaagaggccgataccccagaaaagctgcggacactgctggctgaaaaactgagctccagacccgaggcagtgcacaagtacgtcacccccctgttcattagcagggcccctaatcgcaaaatgtccgggcagggacatatggagactgtgaaatcagctaagcggctggacgaaggcatcagcgtgctgagagtcccactgacccagctgaagctgaaagatctggagaagatggtgaaccgggaaagagagcccaagctgtatgaagctctgaaagcaagactggaggcccacaaggacgatccagctaaagcatttgccgagcccttctacaaatatgacaaggccggcaatcggacacagcaggtgaaggctgtcagagtggagcaggtccagaaaactggggtctgggtgcacaaccataatggaattgccgacaacgctacaatcgtccgggtggatgtgttcgagaaaggcgggaagtactatctggtgcctatctactcctggcaggtcgccaagggaatcctgccagatagagctgtcgtgcagggcaaagacgaagaggattggactgtgatggacgattctttcgagtttaagttcgtcctgtacgcaaacgacctgatcaagctgacagccaagaaaaatgaatttctggggtatttcgtgtcactgaacagggcaactggagccatcgatattcgcacacatgacactgatagcaccaagggaaaaaacggcatctttcagtctgtgggcgtcaagaccgccctgagtttccagaaatatcagattgacgaactggggaaggagatccgaccctgtcggctgaagaaacgaccacccgtgcggtaagaattc

SEQ ID NO: 182 - RNA, 145 nt, Artificial Sequence
  source: /note="Description of Artificial Sequence: Synthetic polynucleotide"
  modified_base (1)..(20): a, c, u, g, unknown or other
nnnnnnnnnnnnnnnnnnnngcugcggauugcgggaaaucgcuuuucgcaagcaaauugaccccuugugcgggcucggcaucccaaggucagcugccgguuauuaucgaaaaggcccaccgcaagcagcgcgugggccuuuuuuu

SEQ ID NO: 183 - protein, 1037 aa, Parvibaculum lavamentivorans
MERIFGFDIGTTSIGFSVIDYSSTQSAGNIQRLGVRIFPEARDPDGTPLNQQRRQKRMMRRQLRRRRIRRKALNETLHEAGFLPAYGSADWPVVMADEPYELRRRGLEEGLSAYEFGRAIYHLAQHRHFKGRELEESDTPDPDVDDEKEAANERAATLKALKNEQTTLGAWLARRPPSDRKRGIHAHRNVVAEEFERLWEVQSKFHPALKSEEMRARISDTIFAQRPVFWRKNTLGECRFMPGEPLCPKGSWLSQQRRMLEKLNNLAIAGGNARPLDAEERDAILSKLQQQASMSWPGVRSALKALYKQRGEPGAEKSLKFNLELGGESKLLGNALEAKLADMFGPDWPAHPRKQEIRHAVHERLWAADYGETPDKKRVIILSEKDRKAHREAAANSFVADFGITGEQAAQLQALKLPTGWEPYSIPALNLFLAELEKGERFGALVNGPDWEGWRRTNFPHRNQPTGEILDKLPSPASKEERERISQLRNPTVVRTQNELRKVVNNLIGLYGKPDRIRIEVGRDVGKSKREREEIQSGIRRNEKQRKKATEDLIKNGIANPSRDDVEKWILWKEGQERCPYTGDQIGFNALFREGRYEVEHIWPRSRSFDNSPRNKTLCRKDVNIEKGNRMPFEAFGHDEDRWSAIQIRLQGMVSAKGGTGMSPGKVKRFLAKTMPEDFAARQLNDTRYAAKQILAQLKRLWPDMGPEAPVKVEAVTGQVTAQLRKLWTLNNILADDGEKTRADHRHHAIDALTVACTHPGMTNKLSRYWQLRDDPRAEKPALTPPWDTIRADAEKAVSEIVVSHRVRKKVSGPLHKETTYGDTGTDIKTKSGTYRQFVTRKKIESLSKGELDEIRDPRIKEIVAAHVAGRGGDPKKAFPPYPCVSPGGPEIRKVRLTSKQQLNLMAQTGNGYADLGSNHHIAIYRLPDGKADFEIVSLFDASRRLAQRNPIVQRTRADGASFVMSLAAGEAIMIPEGSKKGIWIVQGVWASGQVVLERDTDADHSTTTRPMPNPILKDDAKKVSIDPIGRVRPSND

SEQ ID NO: 184 - DNA, 3195 bp, Artificial Sequence
  source: /note="Description of Artificial Sequence: Synthetic polynucleotide"
accggtgccaccatgtacccatacgatgttccagattacgcttcgccgaagaaaaagcgcaaggtcgaagcgtccatggagaggattttcggctttgacatcggcacaacaagtatcggattcagcgtgattgattacagtagcacccagtccgcaggcaacatccagaggctgggcgtgcgcattttccctgaggcaagggacccagatgggacccccctgaaccagcagcggagacagaaacgcatgatgaggcgccagctgcgacggagaaggattcgccgaaaggcactgaatgagacactgcacgaagccggctttctgccagcttacgggtctgcagattggcccgtggtcatggccgacgagccttatgaactgcggagaaggggactggaggaaggcctgagtgcttacgagttcggacgggcaatctatcatctggcccagcaccggcattttaaaggcagagaactggaggaatccgatacacccgaccctgatgtggacgatgagaaggaagccgctaacgagagagcagccactctgaaggccctgaaaaatgaacagaccacactgggagcatggctggcccgccgacccccttctgaccgcaagcgaggaatccacgcccataggaacgtggtcgctgaggagttcgagcgcctgtgggaagtgcagtccaagtttcaccccgctctgaaatctgaggaaatgcgggcaagaatcagtgatacaattttcgcccagaggcctgtgttttggcgcaagaacactctgggagagtgcagattcatgcctggcgaaccactgtgtcccaaggggtcctggctgtctcagcagcggagaatgctggagaaactgaacaatctggctatcgcaggcgggaatgctaggccactggatgcagaggaacgcgacgccattctgagtaagctgcagcagcaggccagcatgtcctggccaggcgtgcggtcagctctgaaggcactgtacaaacagagaggcgagcccggggctgaaaagagcctgaaattcaacctggagctgggaggcgaatccaagctgctgggaaatgccctggaggctaaactggcagatatgtttggccctgactggccagctcacccccgaaagcaggagatccggcacgcagtgcatgaacggctgtgggctgcagattacggcgagacacccgacaagaaaagagtcatcattctgtccgagaaggatcgaaaagctcatcgggaagccgctgcaaactctttcgtggcagactttggaattactggcgagcaggcagctcagctgcaggccctgaagctgccaaccggctgggaaccttatagcatcccagcactgaacctgttcctggccgagctggaaaagggggagaggtttggagccctggtgaatggacctgattgggaaggctggaggcgcacaaacttcccccaccgcaatcagcctactggggagatcctggacaagctgccaagtcccgcctcaaaagaggaaagggaacgcattagccagctgcgcaacccaaccgtggtccgaacacagaatgagctgagaaaggtggtcaacaatctgatcgggctgtatggaaaacccgatcgaatccggattgaagtgggccgggacgtcgggaagtccaaaagagaaagggaggaaatccagtctggcattcgacggaacgagaagcagagaaagaaagccactgaagatctgatcaaaaacggaattgctaatcctagccgggacgatgtggagaagtggatcctgtggaaagagggccaggaaagatgcccatacaccggcgaccagattggcttcaatgccctgtttagagaaggcagatatgaggtggaacacatctggcctcgctctcgaagttttgataacagcccaaggaataagacactgtgtcgcaaagacgtgaacatcgagaagggaaataggatgcctttcgaggcatttggccatgacgaagatcggtggagcgccatccagattagactgcagggcatggtgtcagccaaagggggaactgggatgagccccggaaaggtcaaacgcttcctggctaagaccatgcctgaggattttgcagcccggcagctgaacgacacaagatacgctgcaaagcagatcctggcccagctgaaaaggctgtggccagacatgggacctgaggctccagtgaaggtcgaagcagtgactggacaggtcaccgcccagctgcgcaaactgtggactctgaacaatattctggctgacgatggggagaaaaccagagcagatcacaggcaccatgccatcgacgctctgacagtggcctgcactcatcctggaatgaccaacaagctgagcaggtattggcagctgcgcgacgatccacgagcagagaagccagctctgactccaccctgggataccatccgcgccgacgctgagaaagccgtgtctgaaattgtggtcagtcaccgggtgagaaagaaagtcagcggcccactgcataaggagactacctacggcgatacagggactgacattaagaccaaatccggcacatatagacagttcgtgaccaggaagaaaatcgagtcactgagcaagggggagctggatgaaattcgcgacccccgaatcaaagaaattgtggcagctcacgtcgcaggacgaggaggcgaccccaagaaggccttccctccatacccctgtgtgtctcccggaggccctgagatccggaaggtcagactgaccagtaaacagcagctgaacctgatggcccagacagggaatggatacgctgacctgggctccaaccaccatatcgcaatctaccggctgcccgatgggaaggccgacttcgagattgtgtcactgtttgatgctagcagaaggctggcacagagaaatccaatcgtgcagaggacacgagcagacggagccagcttcgtcatgtccctggcagccggagaggccatcatgattcccgaaggctcaaagaaagggatctggattgtgcagggagtctgggcaagcggacaggtggtcctggagagggacaccgatgctgaccactctacaactacccgccctatgccaaaccccatcctgaaggacgatgccaagaaagtgagtatcgatcctattggccgagtccggccatcaaatgactaagaattc

SEQ ID NO: 185 - RNA, 103 nt, Artificial Sequence
  source: /note="Description of Artificial Sequence: Synthetic polynucleotide"
  modified_base (1)..(20): a, c, u, g, unknown or other
nnnnnnnnnnnnnnnnnnnnguuuuaguacucuggaaacagaaucuacuaaaacaaggcaaaaugccguguuuaucucgucaacuuguuggcgagauuuuuuu

SEQ ID NO: 186 - protein, 1053 aa, Staphylococcus aureus
MKRNYILGLDIGITSVGYGIIDYETRDVIDAGVRLFKEANVENNEGRRSKRGARRLKRRRRHRIQRVKKLLFDYNLLTDHSELSGINPYEARVKGLSQKLSEEEFSAALLHLAKRRGVHNVNEVEEDTGNELSTKEQISRNSKALEEKYVAELQLERLKKDGEVRGSINRFKTSDYVKEAKQLLKVQKAYHQLDQSFIDTYIDLLETRRTYYEGPGEGSPFGWKDIKEWYEMLMGHCTYFPEELRSVKYAYNADLYNALNDLNNLVITRDENEKLEYYEKFQIIENVFKQKKKPTLKQIAKEILVNEEDIKGYRVTSTGKPEFTNLKVYHDIKDITARKEIIENAELLDQIAKILTIYQSSEDIQEELTNLNSELTQEEIEQISNLKGYTGTHNLSLKAINLILDELWHTNDNQIAIFNRLKLVPKKVDLSQQKEIPTTLVDDFILSPVVKRSFIQSIKVINAIIKKYGLPNDIIIELAREKNSKDAQKMINEMQKRNRQTNERIEEIIRTTGKENAKYLIEKIKLHDMQEGKCLYSLEAIPLEDLLNNPFNYEVDHIIPRSVSFDNSFNNKVLVKQEENSKKGNRTPFQYLSSSDSKISYETFKKHILNLAKGKGRISKTKKEYLLEERDINRFSVQKDFINRNLVDTRYATRGLMNLLRSYFRVNNLDVKVKSINGGFTSFLRRKWKFKKERNKGYKHHAEDALIIANADFIFKEWKKLDKAKKVMENQMFEEKQAESMPEIETEQEYKEIFITPHQIKHIKDFKDYKYSHRVDKKPNRELINDTLYSTRKDDKGNTLIVNNLNGLYDKDNDKLKKLINKSPEKLLMYHHDPQTYQKLKLIMEQYGDEKNPLYKYYEETGNYLTKYSKKDNGPVIKKIKYYGNKLNAHLDITDDYPNSRNKVVKLSLKPYRFDVYLDNGVYKFVTVKNLDVIKKENYYEVNSKCYEEAKKLKKISNQAEFIASFYNNDLIKINGELYRVIGVNNDLLNRIEVNMIDITYREYLENMNDKRPPRIIKTIASKTQSIKKYSTDILGNLYEVKSKKHPQIIKKG

SEQ ID NO: 187 - DNA, 3243 bp, Artificial Sequence; identical to SEQ ID NO: 85
  source: /note="Description of Artificial Sequence: Synthetic polynucleotide"

SEQ ID NO: 188 - RNA, 114 nt, Artificial Sequence
  source: /note="Description of Artificial Sequence: Synthetic polynucleotide"
  modified_base (1)..(20): a, c, u, g, unknown or other
nnnnnnnnnnnnnnnnnnnnguuuuagcacuguacaagaaauugucgugcuaaaauaaggcgcuguuaaugcagcugccgcauccgccagagcauuuaugcucuggcuuuuuuu

SEQ ID NO: 189 - protein, 1269 aa, Mycoplasma gallisepticum
MNNSIKSKPEVTIGLDLGVGSVGWAIVDNETNIIHHLGSRLFSQAKTAEDRRSFRGVRRLIRRRKYKLKRFVNLIWKYNSYFGFKNKEDILNNYQEQQKLHNTVLNLKSEALNAKIDPKALSWILHDYLKNRGHFYEDNRDFNVYPTKELAKYFDKYGYYKGIIDSKEDNDNKLEEELTKYKFSNKHWLEEVKKVLSNQTGLPEKFKEEYESLFSYVRNYSEGPGSINSVSPYGIYHLDEKEGKVVQKYNNIWDKTIGKCNIFPDEYRAPKNSPIAMIFNEINELSTIRSYSIYLTGWFINQEFKKAYLNKLLDLLIKTNGEKPIDARQFKKLREETIAESIGKETLKDVENEEKLEKEDHKWKLKGLKLNTNGKIQYNDLSSLAKFVHKLKQHLKLDFLLEDQYATLDKINFLQSLFVYLGKHLRYSNRVDSANLKEFSDSNKLFERILQKQKDGLFKLFEQTDKDDEKILAQTHSLSTKAMLLAITRMTNLDNDEDNQKNNDKGWNFEAIKNFDQKFIDITKKNNNLSLKQNKRYLDDRFINDAILSPGVKRILREATKVFNAILKQFSEEYDVTKVVIELARELSEEKELENTKNYKKLIKKNGDKISEGLKALGISEDEIKDILKSPTKSYKFLLWLQQDHIDPYSLKEIAFDDIFTKTEKFEIDHIIPYSISFDDSSSNKLLVLAESNQAKSNQTPYEFISSGNAGIKWEDYEAYCRKFKDGDSSLLDSTQRSKKFAKMMKTDTSSKYDIGFLARNLNDTRYATIVFRDALEDYANNHLVEDKPMFKVVCINGSVTSFLRKNFDDSSYAKKDRDKNIHHAVDASIISIFSNETKTLFNQLTQFADYKLFKNTDGSWKKIDPKTGVVTEVTDENWKQIRVRNQVSEIAKVIEKYIQDSNIERKARYSRKIENKTNISLFNDTVYSAKKVGYEDQIKRKNLKTLDIHESAKENKNSKVKRQFVYRKLVNVSLLNNDKLADLFAEKEDILMYRANPWVINLAEQIFNEYTENKKIKSQNVFEKYMLDLTKEFPEKFSEFLVKSMLRNKTAIIYDDKKNIVHRIKRLKMLSSELKENKLSNVIIRSKNQSGTKLSYQDTINSLALMIMRSIDPTAKKQYIRVPLNTLNLHLGDHDFDLHNMDAYLKKPKFVKYLKANEIGDEYKPWRVLTSGTLLIHKKDKKLMYISSFQNLNDVIEIKNLIETEYKENDDSDSKKKKKANRFLMTLSTILNDYILLDAKDNFDILGLSKNRIDEILNSKLGLDKIVK

SEQ ID NO: 190 - DNA, 3891 bp, Artificial Sequence; identical to SEQ ID NO: 136
  source: /note="Description of Artificial Sequence: Synthetic polynucleotide"

SEQ ID NO: 191 - RNA, 137 nt, Artificial Sequence
  source: /note="Description of Artificial Sequence: Synthetic polynucleotide"
  modified_base (1)..(20): a, c, u, g, unknown or other
nnnnnnnnnnnnnnnnnnnnguuuuagucucugaaaagagacuaaaauaagugguuuuuggucauccacgcaggguuacaaucccuuuaaaaccauuaaaauucaaauaaacuagguuguaucaacuuaguuuuuuu

SEQ ID NO: 192 - protein, 1003 aa, Campylobacter lari
MRILGFDIGINSIGWAFVENDELKDCGVRIFTKAENPKNKESLALPRRNARSSRRRLKRRKARLIAIKRILAKELKLNYKDYVAADGELPKAYEGSLASVYELRYKALTQNLETKDLARVILHIAKHRGYMNKNEKKSNDAKKGKILSALKNNALKLENYQSVGEYFYKEFFQKYKKNTKNFIKIRNTKDNYNNCVLSSDLEKELKLILEKQKEFGYNYSEDFINEILKVAFFQRPLKDFSHLVGACTFFEEEKRACKNSYSAWEFVALTKIINEIKSLEKISGEIVPTQTINEVLNLILDKGSITYKKFRSCINLHESISFKSLKYDKENAENAKLIDFRKLVEFKKALGVHSLSRQELDQISTHITLIKDNVKLKTVLEKYNLSNEQINNLLEIEFNDYINLSFKALGMILPLMREGKRYDEACEIANLKPKTVDEKKDFLPAFCDSIFAHELSNPVVNRAISEYRKVLNALLKKYGKVHKIHLELARDVGLSKKAREKIEKEQKENQAVNAWALKECENIGLKASAKNILKLKLWKEQKEICIYSGNKISIEHLKDEKALEVDHIYPYSRSFDDSFINKVLVFTKENQEKLNKTPFEAFGKNIEKWSKIQTLAQNLPYKKKNKILDENFKDKQQEDFISRNLNDTRYIATLIAKYTKEYLNFLLLSENENANLKSGEKGSKIHVQTISGMLTSVLRHTWGFDKKDRNNHLHHALDAIIVAYSTNSIIKAFSDFRKNQELLKARFYAKELTSDNYKHQVKFFEPFKSFREKILSKIDEIFVSKPPRKRARRALHKDTFHSENKIIDKCSYNSKEGLQIALSCGRVRKIGTKYVENDTIVRVDIFKKQNKFYAIPIYAMDFALGILPNKIVITGKDKNNNPKQWQTIDESYEFCFSLYKNDLILLQKKNMQEPEFAYYNDFSISTSSICVEKHDNKFENLTSNQKLLFSNAKEGSVKVESLGIQNLKVFEKYIITPLGDKIKADFQPRENISLKTSKKYGLR

SEQ ID NO: 193 - DNA, 3093 bp, Artificial Sequence; identical to SEQ ID NO: 137
  source: /note="Description of Artificial Sequence: Synthetic polynucleotide"

SEQ ID NO: 194 - RNA, 103 nt, Artificial Sequence
  source: /note="Description of Artificial Sequence: Synthetic polynucleotide"
  modified_base (1)..(20): a, c, u, g, unknown or other
nnnnnnnnnnnnnnnnnnnnguuuuagagcuagaaauagcaaguuaaaauaaggcuaguccguuaucaacuugaaaaaguggcaccgagucggugcuuuuuuu

SEQ ID NO: 195 - protein, 1368 aa, Streptococcus pyogenes [sequence omitted]

SEQ ID NO: 196 - DNA, 4218 bp, Artificial Sequence
  source: /note="Description of Artificial Sequence: Synthetic polynucleotide"
accggtgccaccatgtacccatacgatgttccagattacgcttcgccgaagaaaaagcgcaaggtcgaagcgtccgacaagaagtacagcatcggcctggacatcggcaccaactctgtgggctgggccgtgatcaccgacgagtacaaggtgcccagcaagaaattcaaggtgctgggcaacaccgaccggcacagcatcaagaagaacctgatcggagccctgctgttcgacagcggcgaaacagccgaggccacccggctgaagagaaccgccagaagaagatacaccagacggaagaaccggatctgctatctgcaagagatcttcagcaacgagatggccaaggtggacgacagcttcttccacagactggaagagtccttcctggtggaagaggataagaagcacgagcggcaccccatcttcggcaacatcgtggacgaggtggcctaccacgagaagtaccccaccatctaccacctgagaaagaaactggtggacagcaccgacaaggccgacctgcggctgatctatctggccctggcccacatgatcaagttccggggccacttcctgatcgagggcgacctgaaccccgacaacagcgacgtggacaagctgttcatccagctggtgcagacctacaaccagctgttcgaggaaaaccccatcaacgccagcggcgtggacgccaaggccatcctgtctgccagactgagcaagagcagacggctggaaaatctgatcgcccagctgcccggcgagaagaagaatggcctgttcggcaacctgattgccctgagcctgggcctgacccccaacttcaagagcaacttcgacctggccgaggatgccaaactgcagctgagcaaggacacctacgacgacgacctggacaacctgctggcccagatcggcgaccagtacgccgacctgtttctggccgccaagaacctgtccgacgccatcctgctgagcgacatcctgagagtgaacaccgagatcaccaaggcccccctgagcgcctctatgatcaagagatacgacgagcaccaccaggacctgaccctgctgaaagctctcgtgcggcagcagctgcctgagaagtacaaagagattttcttcgaccagagcaagaacggctacgccggctacattgacggcggagccagccaggaagagttctacaagttcatcaagcccatcctggaaaagatggacggcaccgaggaactgctcgtgaagctgaacagagaggacctgctgcggaagcagcggaccttcgacaacggcagcatcccccaccagatccacctgggagagctgcacgccattctgcggcggcaggaagatttttacccattcctgaaggacaaccgggaaaagatcgagaagatcctgaccttccgcatcccctactacgtgggccctctggccaggggaaacagcagattcgcctggatgaccagaaagagcgaggaaaccatcaccccctggaacttcgaggaagtggtggacaagggcgcttccgcccagagcttcatcgagcggatgaccaacttcgataagaacctgcccaacgagaaggtgctgcccaagcacagcctgctgtacgagtacttcaccgtgtataacgagctgaccaaagtgaaatacgtgaccgagggaatgagaaagcccgccttcctgagcggcgagcagaaaaaggccatcgtggacctgctgttcaagaccaaccggaaagtgaccgtgaagcagctgaaagaggactacttcaagaaaatcgagtgcttcgactccgtggaaatctccggcgtggaagatcggttcaacgcctccctgggcacataccacgatctgctgaaaattatcaaggacaaggacttcctggacaatgaggaaaacgaggacattctggaagatatcgtgctgaccctgacactgtttgaggacagagagatgatcgaggaacggctgaaaacctatgcccacctgttcgacgacaaagtgatgaagcagctgaagcggcggagatacaccggctggggcaggctgagccggaagctgatcaacggcatccgggacaagcagtccggcaagacaatcctggatttcctgaagtccgacggcttcgccaacagaaacttcatgcagctgatccacgacgacagcctgacctttaaagaggacatccagaaagcccaggtgtccggccagggcgatagcctgcacgagcacattgccaatctggccggcagccccgccattaagaagggcatcctgcagacagtgaaggtggtggacgagctcgtgaaagtgatgggccggcacaagcccgagaacatcgtgatcgaaatggccagagagaaccagaccacccagaagggacagaagaacagccgcgagagaatgaagcggatcgaagagggcatcaaagagctgggcagccagatcctgaaagaacaccccgtggaaaacacccagctgcagaacgagaagctgtacctgtactacctgcagaatgggcgggatatgtacgtggaccaggaactggacatcaaccggctgtccgactacgatgtggaccatatcgtgcctcagagctttctgaaggacgactccatcgacaacaaggtgctgaccagaagcgacaagaaccggggcaagagcgacaacgtgccctccgaagaggtcgtgaagaagatgaagaactactggcggcagctgctgaacgccaagctgattacccagagaaagttcgacaatctgaccaaggccgagagaggcggcctgagcgaactggataaggccggcttcatcaagagacagctggtggaaacccggcagatcacaaagcacgtggcacagatcctggactcccggatgaacactaagtacgacgagaatgacaagctgatccgggaagtgaaagtgatcaccctgaagtccaagctggtgtccgatttccggaaggatttccagttttacaaagtgcgcgagatcaacaactaccaccacgcccacgacgcctacctgaacgccgtcgtgggaaccgccctgatcaaaaagtaccctaagctggaaagcgagttcgtgtacggcgactacaaggtgtacgacgtgcggaagatgatcgccaagagcgagcaggaaatcggcaaggctaccgccaagtacttcttctacagcaacatcatgaactttttcaagaccgagattaccctggccaacggcgagatccggaagcggcctctgatcgagacaaacggcgaaaccggggagatcgtgtgggataagggccgggattttgccaccgtgcggaaagtgctgagcatgccccaagtgaatatcgtgaaaaagaccgaggtgcagacaggcggcttcagcaaagagtctatcctgcccaagaggaacagcgataagctgatcgccagaaagaaggactgggaccctaagaagtacggcggcttcgacagccccaccgtggcctattctgtgctggtggtggccaaagtggaaaagggcaagtccaagaaactgaagagtgtgaaagagctgctggggatcaccatcatggaaagaagcagcttcgagaagaatcccatcgactttctggaagccaagggctacaaagaagtgaaaaaggacctgatcatcaagctgcctaagtactccctgttcgagctggaaaacggccggaagagaatgctggcctctgccggcgaactgcagaagggaaacgaactggccctgccctccaaatatgtgaacttcctgtacctggccagccactatgagaagctgaagggctcccccgaggataatgagcagaaacagctgtttgtggaacagcacaagcactacctggacgagatcatcgagcagatcagcgagttctccaagagagtgatcctggccgacgctaatctggacaaagtgctgtccgcctacaacaagcaccgggataagcccatcagagagcaggccgagaatatcatccacctgtttaccctgaccaatctgggagcccctgccgccttcaagtactttgacaccaccatcgaccggaagaggtacaccagcaccaaagaggtgctggacgccaccctgatccaccagagcatcaccggcctgtacgagacacggatcgacctgtctcagctgggaggcgacagccccaagaagaagagaaaggtggaggccagctaagaattc

SEQ ID NO: 197 - RNA, 116 nt, Artificial Sequence
  source: /note="Description of Artificial Sequence: Synthetic polynucleotide"
  modified_base (1)..(20): a, c, u, g, unknown or other
nnnnnnnnnnnnnnnnnnnnguuuuuguacucucaagauuuagaaacuugcagaagcuacaaagauaaggcuucaugccgaaaucaacacccugucauuuuauggcaggguguuuu

SEQ ID NO: 198 - protein, 1120 aa, Streptococcus thermophilus
MSDLVLGLDIGIGSVGVGILNKVTGEIIHKNSRIFPAAQAENNLVRRTNRQGRRLARRKKHRRVRLNRLFEESGLITDFTKISINLNPYQLRVKGLTDELSNEELFIALKNMVKHRGISYLDDASDDGNSSVGDYAQIVKENSKQLETKTPGQIQLERYQTYGQLRGDFTVEKDGKKHRLINVFPTSAYRSEALRILQTQQEFNPQITDEFINRYLEILTGKRKYYHGPGNEKSRTDYGRYRTSGETLDNIFGILIGKCTFYPDEFRAAKASYTAQEFNLLNDLNNLTVPTETKKLSKEQKNQIINYVKNEKAMGPAKLFKYIAKLLSCDVADIKGYRIDKSGKAEIHTFEAYRKMKTLETLDIEQMDRETLDKLAYVLTLNTEREGIQEALEHEFADGSFSQKQVDELVQFRKANSSIFGKGWHNFSVKLMMELIPELYETSEEQMTILTRLGKQKTTSSSNKTKYIDEKLLTEEIYNPVVAKSVRQAIKIVNAAIKEYGDFDNIVIEMARETNEDDEKKAIQKIQKANKDEKDAAMLKAANQYNGKAELPHSVFHGHKQLATKIRLWHQQGERCLYTGKTISIHDLINNSNQFEVDHILPLSITFDDSLANKVLVYATANQEKGQRTPYQALDSMDDAWSFRELKAFVRESKTLSNKKKEYLLTEEDISKFDVRKKFIERNLVDTRYASRVVLNALQEHFRAHKIDTKVSVVRGQFTSQLRRHWGIEKTRDTYHHHAVDALIIAASSQLNLWKKQKNTLVSYSEDQLLDIETGELISDDEYKESVFKAPYQHFVDTLKSKEFEDSILFSYQVDSKFNRKISDATIYATRQAKVGKDKADETYVLGKIKDIYTQDGYDAFMKIYKKDKSKFLMYRHDPQTFEKVIEPILENYPNKQINEKGKEVPCNPFLKYKEEHGYIRKYSKKGNGPEIKSLKYYDSKLGNHIDITPKDSNNKVVLQSVSPWRADVYFNKTTGKYEILGLKYADLQFEKGTGTYKISQEKYNDIKKKEGVDSDSEFKFTLYKNDLLLVKDTETKEQQLFRFLSRTMPKQKHYVELKPYDKQKFEGGEALIKVLGNVANSGQCKKGLGKSNISIYKVRTDVLGNQHIIKNEGDKPKLM

SEQ ID NO: 199 - DNA, 3477 bp, Artificial Sequence
  source: /note="Description of Artificial Sequence: Synthetic polynucleotide"
accggtgccaccatgtacccatacgatgttccagattacgcttcgccgaagaaaaagcgcaaggtcgaagcgtcctccgacctggtacttggactggatattggtatcggttcggtgggagtcggaatcctcaacaaggtcacgggggagatcattcacaagaactcgcggatcttccccgcagctcaggctgagaacaacttggtgcggagaacgaataggcagggcaggcgactggcgaggaggaagaaacacaggagagtccgattgaaccggctgttcgaggagtccggtttgatcaccgactttacgaaaatctcgattaaccttaatccctatcagcttcgggtgaaaggcctgacagacgaactttcgaatgaggaacttttcatcgcgctgaaaaacatggtcaagcacagagggatttcctacctcgatgacgcctcggatgacggaaattcctcagtaggagattatgcacagatcgtgaaagagaactcaaagcaactggaaacaaagacaccggggcagatccaacttgaaagataccagacatacggacagctcagaggagattttacggtggagaaggacggtaaaaagcacagactcattaacgtatttcccacgtcggcgtacagatccgaagcgctccgcatccttcagactcaacaggagttcaacccgcaaattactgatgagttcatcaaccgctatttggaaatcttgaccggaaagcgcaagtattatcatgggccgggtaatgagaaatccagaacagattacggccgatacagaacttcgggggaaaccttggataacatctttggtattttgattggaaagtgcaccttttacccggacgagtttcgagcggccaaggcgtcatacacagcacaagagtttaatctcttgaatgatttgaacaacttgacggtccccacggagacaaagaagctctccaaagagcaaaagaaccaaatcatcaactacgtcaagaacgagaaggctatggggccagcgaagctgttcaagtatatcgctaaacttctcagctgtgatgtggcggacatcaaagggtaccgaatcgacaagtcgggaaaagcggaaattcacacgtttgaagcatatcgaaagatgaaaacgttggaaacactggacattgagcagatggaccgggaaacgctcgacaaactggcatacgtgctcacgttgaatactgaacgagagggaatccaagaggcccttgaacatgagttcgccgatggatcgttcagccagaagcaggtcgacgaacttgtgcaattccgcaaggcgaatagctccatcttcgggaagggatggcacaacttttcggtcaaactcatgatggagttgatcccagaactttatgagacttcggaggagcaaatgacgatcttgacgcgcttggggaaacagaaaacgacaagctcatcgaacaaaactaagtacattgatgagaaattgctgacggaagaaatctataatccggtagtagcgaaatcggtaagacaagcgatcaaaatcgtgaacgcggcgatcaaggaatatggtgactttgataacatcgtaattgaaatggctagagagacgaacgaagatgacgagaaaaaggcaatccagaagatccagaaggccaacaaggatgaaaaagatgcagcgatgcttaaagcggccaaccaatacaatggaaaggcggagctgccccattcagtgtttcacggtcataaacagttggcgaccaagatccgactctggcatcagcagggtgagcggtgtctctacaccggaaagactatctccatccatgacttgattaacaattcgaaccagtttgaagtggatcatattctgcccctgtcaatcacctttgacgactcgcttgcgaacaaggtgctcgtgtacgcaacggcaaatcaggagaaaggccagcggactccgtatcaggcgctcgactcaatggacgatgcgtggtcattccgggagctgaaggcgttcgtacgcgagagcaagacactgagcaacaaaaagaaagagtatctgctgacagaggaggacatctcgaaattcgatgtcaggaagaagttcatcgagcggaatcttgtcgacactcgctacgcttccagagtagtactgaacgcgctccaggaacactttagagcgcacaaaattgacacgaaggtgtcagtggtgagagggcagttcacatcccaactccgccgacattggggcatcgaaaagacgcgggacacatatcaccatcatgcggtggacgcgctgattattgccgcttcgtcccagttgaatctctggaaaaagcagaagaacacgctggtgtcgtattcggaggatcagcttttggacatcgaaaccggggagctgatttccgacgatgaatacaaagaatcggtgtttaaggcaccatatcagcatttcgtggacacgctgaagagcaaagagtttgaggacagcatcctcttttcgtaccaagtggactcgaagtttaatcgcaagatttcagacgccacaatctacgcgacgaggcaggcgaaggtgggcaaagataaagcagatgaaacctacgtccttggtaaaatcaaggacatctacactcaggacgggtacgatgcgttcatgaaaatctacaagaaggataagtcgaagtttctcatgtaccgccacgatccacagactttcgaaaaagtcattgagcctattttggagaactaccctaacaagcaaatcaacgagaaagggaaagaagtcccgtgcaacccctttctgaagtacaaggaagagcacggttatatccgcaaatactcgaagaaaggaaatgggcctgagattaagtcgcttaagtattacgactcaaagttgggtaaccacatcgacattaccccgaaagactccaacaacaaagtcgtgttgcagtccgtctcgccctggcgagcagatgtgtattttaataagacgaccggcaaatatgagatccttggactcaaatacgcagaccttcaattcgaaaaggggacgggcacttataagatttcacaagagaagtacaacgacatcaagaaaaaggaaggggtcgattcagattcggagttcaaattcaccctctacaaaaacgacctcctgcttgtgaaggacacagaaacgaaggagcagcagctctttcggttcctctcacgcacgatgcccaaacaaaaacattacgtcgaacttaaaccttacgataagcaaaagtttgaagggggagaggcactgatcaaagtattgggtaacgtagccaatagcggacagtgtaagaaagggctgggaaagtccaatatctcgatctataaagtacgaacagatgtattgggaaaccagcatatcatcaaaaatgagggggataaacccaaactcgatttcagccccaagaagaagagaaaggtggaggccagctaagaattc

SEQ ID NO: 200 - DNA, 27 bp, Artificial Sequence
  source: /note="Description of Artificial Sequence: Synthetic oligonucleotide"
gcccgggtggaactggtagccatgaat

SEQ ID NO: 201 - DNA, 26 bp, Artificial Sequence
  source: /note="Description of Artificial Sequence: Synthetic oligonucleotide"
gttgaagatgaagcccagagcggagt

SEQ ID NO: 202 - DNA, 27 bp, Artificial Sequence
  source: /note="Description of Artificial Sequence: Synthetic oligonucleotide"
gcttccgacgaggtggccatcaaggat

SEQ ID NO: 203 - DNA, 27 bp, Artificial Sequence
  source: /note="Description of Artificial Sequence: Synthetic oligonucleotide"
gcaccatctctccgtggtaccccgggt

SEQ ID NO: 204 - DNA, 26 bp, Artificial Sequence
  source: /note="Description of Artificial Sequence: Synthetic oligonucleotide"
ggtggaactggtagccatgaatgaga

SEQ ID NO: 205 - DNA, 27 bp, Artificial Sequence
  source: /note="Description of Artificial Sequence: Synthetic oligonucleotide"
gccatgaatgagaccgacccaaagagc

SEQ ID NO: 206 - DNA, 27 bp, Artificial Sequence
  source: /note="Description of Artificial Sequence: Synthetic oligonucleotide"
gcatcctcgtgggcacttccgacgagg

SEQ ID NO: 207 - DNA, 27 bp, Artificial Sequence
  source: /note="Description of Artificial Sequence: Synthetic oligonucleotide"
gcagagcggagtgctgttctcccaagt

SEQ ID NO: 208 - DNA, 26 bp, Artificial Sequence
  source: /note="Description of Artificial Sequence: Synthetic oligonucleotide"
ggtcggtctcattcatggctaccagt

SEQ ID NO: 209 - DNA, 26 bp, Artificial Sequence
  source: /note="Description of Artificial Sequence: Synthetic oligonucleotide"
gcaataaaaggtgctattgctatagt

SEQ ID NO: 210 - DNA, 26 bp, Artificial Sequence
  source: /note="Description of Artificial Sequence: Synthetic oligonucleotide"
gtactcaaccaagtcattctgagaat

SEQ ID NO: 211 - DNA, 26 bp, Artificial Sequence
  source: /note="Description of Artificial Sequence: Synthetic oligonucleotide"
  modified_base (1)..(7): a, c, t, g, unknown or other
nnnnnnngtactcaaccaagtcattc

SEQ ID NO: 212 - protein, 1121 aa, Streptococcus thermophilus
MSDLVLGLDIGIGSVGVGILNKVTGEIIHKNSRIFPAAQAENNLVRRTNRQGRRLARRKKHRRVRLNRLFEESGLITDFTKISINLNPYQLRVKGLTDELSNEELFIALKNMVKHRGISYLDDASDDGNSSVGDYAQIVKENSKQLETKTPGQIQLERYQTYGQLRGDFTVEKDGKKHRLINVFPTSAYRSEALRILQTQQEFNPQITDEFINRYLEILTGKRKYYHGPGNEKSRTDYGRYRTSGETLDNIFGILIGKCTFYPDEFRAAKASYTAQEFNLLNDLNNLTVPTETKKLSKEQKNQIINYVKNEKAMGPAKLFKYIAKLLSCDVADIKGYRIDKSGKAEIHTFEAYRKMKTLETLDIEQMDRETLDKLAYVLTLNTEREGIQEALEHEFADGSFSQKQVDELVQFRKANSSIFGKGWHNFSVKLMMELIPELYETSEEQMTILTRLGKQKTTSSSNKTKYIDEKLLTEEIYNPVVAKSVRQAIKIVNAAIKEYGDFDNIVIEMARETNEDDEKKAIQKIQKANKDEKDAAMLKAANQYNGKAELPHSVFHGHKQLATKIRLWHQQGERCLYTGKTISIHDLINNSNQFEVDHILPLSITFDDSLANKVLVYATANQEKGQRTPYQALDSMDDAWSFRELKAFVRESKTLSNKKKEYLLTEEDISKFDVRKKFIERNLVDTRYASRVVLNALQEHFRAHKIDTKVSVVRGQFTSQLRRHWGIEKTRDTYHHHAVDALIIAASSQLNLWKKQKNTLVSYSEDQLLDIETGELISDDEYKESVFKAPYQHFVDTLKSKEFEDSILFSYQVDSKFNRKISDATIYATRQAKVGKDKADETYVLGKIKDIYTQDGYDAFMKIYKKDKSKFLMYRHDPQTFEKVIEPILENYPNKQINEKGKEVPCNPFLKYKEEHGYIRKYSKKGNGPEIKSLKYYDSKLGNHIDITPKDSNNKVVLQSVSPWRADVYFNKTTGKYEILGLKYADLQFEKGTGTYKISQEKYNDIKKKEGVDSDSEFKFTLYKNDLLLVKDTETKEQQLFRFLSRTMPKQKHYVELKPYDKQKFEGGEALIKVLGNVANSGQCKKGLGKSNISIYKVRTDVLGNQHIIKNEGDKPKLDF

SEQ ID NO: 213 - DNA, 20 bp, Corynebacter diphtheriae
aaaagggaataagggcgaca

SEQ ID NO: 214 - DNA, 27 bp, Sutterella wadsworthensis
  modified_base (1)..(1): a, c, t, g, unknown or other
  modified_base (4)..(7): a, c, t, g, unknown or other
nggnnnncattctgagaatagtgtatg

SEQ ID NO: 215 - DNA, 20 bp, Sutterella wadsworthensis
gcgaccgagttgctcttgcc

SEQ ID NO: 216 - DNA, 27 bp, Legionella pneumophila
  modified_base (1)..(1): a, c, t, g, unknown or other
  modified_base (4)..(7): a, c, t, g, unknown or other
nggnnnncattctgagaatagtgtatg

SEQ ID NO: 217 - DNA, 20 bp, Legionella pneumophila
gcgaccgagttgctcttgcc

SEQ ID NO: 218 - DNA, 27 bp, Filifactor alocis
  modified_base (1)..(3): a, c, t, g, unknown or other
nnnaagcttgagtactcaccagtcaca

SEQ ID NO: 219 - DNA, 20 bp, Filifactor alocis
ctcttcctttttcaatatta

SEQ ID NO: 220 - DNA, 27 bp, Lactobacillus johnsonii
  modified_base (1)..(2): a, c, t, g, unknown or other
  modified_base (6)..(7): a, c, t, g, unknown or other
nnaaanntaaatgcttcaataatattg

SEQ ID NO: 221 - DNA, 20 bp, Lactobacillus johnsonii
aaagggaataagggcgacac

SEQ ID NO: 222 - DNA, 27 bp, Parvibaculum lavamentivorans
  modified_base (1)..(3): a, c, t, g, unknown or other
  modified_base (7)..(7): a, c, t, g, unknown or other
nnncatnaaaggaagagtatgagtatt

SEQ ID NO: 223 - DNA, 20 bp, Staphylococcus aureus
ctattctcagaatgacttgg

SEQ ID NO: 224 - DNA, 27 bp, Mycoplasma gallisepticum
  modified_base (1)..(2): a, c, t, g, unknown or other
  modified_base (5)..(5): a, c, t, g, unknown or other
nnganggagtcacagaaaagcatctta

SEQ ID NO: 225 - DNA, 20 bp, Mycoplasma gallisepticum
gtttctgggtgagcaaaaac

SEQ ID NO: 226 - DNA, 27 bp, Campylobacter lari
  modified_base (1)..(2): a, c, t, g, unknown or other
  modified_base (6)..(6): a, c, t, g, unknown or other
nngggnagaaggcaaaatgccgcaaaa

SEQ ID NO: 227 - DNA, 20 bp, Campylobacter lari
ggtattatcccgtattgacg

SEQ ID NO: 228 - DNA, 20 bp, Unknown
  source: /note="Description of Unknown: SpCas9 oligonucleotide"
gggactcaaccaagtcattc